European Patent Specification EP 4 062 917 B1, published December 3, 2025. Title: CANCER TREATMENTS USING COMBINATIONS OF PI3K/AKT PATHWAY AND ERK INHIBITORS. Applicant: BIOMED VALLEY DISCOVERIES, INC. The sequence listing filed with the application follows.

SEQUENCE LISTING (93 sequences)

SEQ ID NO: 1 - DNA, 5436 bp, Homo sapiens
ggccgcggcggcggaggcagcagcggcggcggcagtggcggcggcgaaggtggcggcggctcggccagtactcccggcccccgccatttcggactgggagcgagcgcggcgcaggcactgaaggcggcggcggggccagaggctcagcggctcccaggtgcgggagagaggcctgctgaaaatgactgaatataaacttgtggtagttggagctggtggcgtaggcaagagtgccttgacgatacagctaattcagaatcattttgtggacgaatatgatccaacaatagaggattcctacaggaagcaagtagtaattgatggagaaacctgtctcttggatattctcgacacagcaggtcaagaggagtacagtgcaatgagggaccagtacatgaggactggggagggctttctttgtgtatttgccataaataatactaaatcatttgaagatattcaccattatagagaacaaattaaaagagttaaggactctgaagatgtacctatggtcctagtaggaaataaatgtgatttgccttctagaacagtagacacaaaacaggctcaggacttagcaagaagttatggaattccttttattgaaacatcagcaaagacaagacagagagtggaggatgctttttatacattggtgagggagatccgacaatacagattgaaaaaaatcagcaaagaagaaaagactcctggctgtgtgaaaattaaaaaatgcattataatgtaatctgggtgttgatgatgccttctatacattagttcgagaaattcgaaaacataaagaaaagatgagcaaagatggtaaaaagaagaaaaagaagtcaaagacaaagtgtgtaattatgtaaatacaatttgtacttttttcttaaggcatactagtacaagtggtaatttttgtacattacactaaattattagcatttgttttagcattacctaatttttttcctgctccatgcagactgttagcttttaccttaaatgcttattttaaaatgacagtggaagtttttttttcctctaagtgccagtattcccagagttttggtttttgaactagcaatgcctgtgaaaaagaaactgaatacctaagatttctgtcttggggtttttggtgcatgcagttgattacttcttatttttcttaccaattgtgaatgttggtgtgaaacaaattaatgaagcttttgaatcatccctattctgtgttttatctagtcacataaatggattaattactaatttcagttgagaccttctaattggtttttactgaaacattgagggaacacaaatttatgggcttcctgatgatgattcttctaggcatcatgtcctatagtttgtcatccctgatgaatgtaaagttacactgttcacaaaggttttgtctcctttccactgctattagtcatggtcactctccccaaaatattatattttttctataaaaagaaaaaaatggaaaaaaattacaaggcaatggaaactattataaggccatttccttttcacattagataaattactataaagactcctaatagcttttcctgttaaggcagacccagtatgaaatggggattattatagcaaccattttggggctatatttacatgctactaaatttttataataattgaaaagattttaacaagtataaaaaattctcataggaattaaatgtagtctccctgtgtcagactgctctttcatagtataactttaaatcttttcttcaacttgagtctttgaagatagttttaattctgcttgtgacattaaaagattatttgggccagttatagcttattaggtgttgaagagaccaaggttgcaaggccaggccctgtgtgaacctttgagctttcatagagagtttcacagcatggactgtgtccccacggtcatccagtgttgtcatgcattggttagtcaaaatggggagggactagggcagtttggatagctcaacaagatacaatctcactctgtggtggtcctgctgacaaatcaagagcattgcttttgtttcttaagaaaacaaactcttttttaaaaattacttttaaatattaactcaaaagttgagattttggggtggtggtgtgccaagacattaattttttttttaaacaatgaagtgaaaaagttttacaatctctaggtttggctagttctcttaacactggttaaattaacattgcataaacacttttcaagtctgatccatatttaataatgctttaaaataaaaataaaaacaatccttttgataaatttaaaatgttacttattttaaaataaatgaagtgagatggcatggtgaggtgaaagtatcactggactaggaagaaggtgacttaggttctagataggtgtcttttaggactctgattttgaggacatcacttactatccatttcttcatgttaaaagaagtcatctcaaactcttagttttttttttttacaactatgtaatttatattccatttacataaggatacacttatttgtcaagctcagcacaatctgtaaatttttaacctatgttacaccatcttcagtgccagtcttgggcaaaattgtgcaagaggtgaagtttatatttgaatatccattctcgttttaggactcttcttccatattagtgtcatcttgcctccctaccttccacatgccccatgacttgatgcagttttaatacttgtaattcccctaaccataagatttactgctgctgtggatatctccatgaagttttcccactgagtcacatcagaaatgccctacatcttatttcctcagggctcaagagaatctgacagataccataaagggatttgacctaatcactaattttcaggtggtggctgatgctttgaacatctctttgctgcccaatccattagcgacagtaggatttttcaaacctggtatgaatagacagaaccctatccagtggaaggagaatttaataaagatagtgctgaaagaattccttaggtaatctataactaggactactcctggtaacagtaatacattccattgttttagtaaccagaaatcttcatgcaatgaaaaatactttaattcatgaagcttactttttttttttggtgtcagagtctcgctcttgtcacccaggctggaatgcagtggcgccatctcagctcactgcaacctccatctcccaggttcaagcgattctcgtgcctcggcctcctgagtagctgggattacaggcgtgtgccactacactcaactaatttttgtatttttaggagagacggggtttcaccctgttggccaggctggtctcgaactcctgacctcaagtgattcacccaccttggcctcataaacctgttttgcagaactcatttattcagcaaatatttattgagtgcctaccagatgccagtcaccgcacaaggcactgggtatatggtatccccaaacaagagacataatcccggtccttaggtagtgctagtgtggtctgtaatatcttactaaggcctttggtatacgacccagagataacacgatgcgtattttagttttgcaaagaaggggtttggtctctgtgccagctctataattgttttgctacgattccactgaaactcttcgatcaagctactttatgtaaatcacttcattgttttaaaggaataaacttgattatattgtttttttatttggcataactgtgattcttttaggacaattactgtacacattaaggtgtatgtcagatattcatattgacccaaatgtgtaatattccagttttctctgcataagtaattaaaatatacttaaaaattaatagttttatctgggtacaaataaacaggtgcctgaactagttcacagacaaggaaacttctatgtaaaaatcactatgatttctgaattgctatgtgaaactacagatctttggaacactgtttaggtagggtgttaagacttacacagtacctcgtttctacacagagaaagaaatggccatacttcaggaactgcagtgcttatgaggggatatttaggcctcttgaatttttgatgtagatgggcatttttttaaggtagtggttaattacctttatgtgaactttgaatggtttaacaaaagatttgtttttgtagagattttaaagggggagaattctagaaataaatgttacctaattattacagccttaaagacaaaaatccttgttgaagtttttttaaaaaaagctaaattacatagacttaggcattaacatgtttgtggaagaatatagcagacgtatattgtatcatttgagtgaatgttcccaagtaggcattctaggctctatttaactgagtcacactgcataggaatttagaacctaacttttataggttatcaaaactgttgtcaccattgcacaattttgtcctaatatatacatagaaactttgtggggcatgttaagttacagtttgcacaagttcatctcatttgtattccattgattttttttttcttctaaacattttttcttcaaacagtatataactttttttaggggatttttttttagacagcaaaaactatctgaagatttccatttgtcaaaaagtaatgatttcttgataattgtgtagtaatgttttttagaacccagcagttaccttaaagctgaatttatatttagtaacttctgtgttaatactggatagcatgaattctgcattgagaaactgaatagctgtcataaaatgaaactttctttctaaagaaagatactcacatgagttcttgaagaatagtcataactagattaagatctgtgttttagtttaatagtttgaagtgcctgtttgggataatgataggtaatttagatgaatttaggggaaaaaaaagttatctgcagatatgttgagggcccatctctccccccacacccccacagagctaactgggttacagtgttttatccgaaagtttccaattccactgtcttgtgttttcatgttgaaaatacttttgcatttttcctttgagtgccaatttcttactagtactatttcttaatgtaacatgtttacctggaatgtattttaactatttttgtatagtgtaaactgaaacatgcacattttgtacattgtgctttcttttgtgggacatatgcagtgtgatccagttgttttccatcatttggttgcgctgacctaggaatgttggtcatatcaaacattaaaaatgaccactcttttaattgaaattaacttttaaatgtttataggagtatgtgctgtgaagtgatctaaaatttgtaatatttttgtcatgaactgtactactcctaattattgtaatgtaataaaaatagttacagtgacaaaaaaaaaaaaaaa

SEQ ID NO: 2 - protein, 189 aa, Homo sapiens [sequence omitted]

SEQ ID NO: 3 - DNA, 5312 bp, Homo sapiens
ggccgcggcggcggaggcagcagcggcggcggcagtggcggcggcgaaggtggcggcggctcggccagtactcccggcccccgccatttcggactgggagcgagcgcggcgcaggcactgaaggcggcggcggggccagaggctcagcggctcccaggtgcgggagagaggcctgctgaaaatgactgaatataaacttgtggtagttggagctggtggcgtaggcaagagtgccttgacgatacagctaattcagaatcattttgtggacgaatatgatccaacaatagaggattcctacaggaagcaagtagtaattgatggagaaacctgtctcttggatattctcgacacagcaggtcaagaggagtacagtgcaatgagggaccagtacatgaggactggggagggctttctttgtgtatttgccataaataatactaaatcatttgaagatattcaccattatagagaacaaattaaaagagttaaggactctgaagatgtacctatggtcctagtaggaaataaatgtgatttgccttctagaacagtagacacaaaacaggctcaggacttagcaagaagttatggaattccttttattgaaacatcagcaaagacaagacagggtgttgatgatgccttctatacattagttcgagaaattcgaaaacataaagaaaagatgagcaaagatggtaaaaagaagaaaaagaagtcaaagacaaagtgtgtaattatgtaaatacaatttgtacttttttcttaaggcatactagtacaagtggtaatttttgtacattacactaaattattagcatttgttttagcattacctaatttttttcctgctccatgcagactgttagcttttaccttaaatgcttattttaaaatgacagtggaagtttttttttcctctaagtgccagtattcccagagttttggtttttgaactagcaatgcctgtgaaaaagaaactgaatacctaagatttctgtcttggggtttttggtgcatgcagttgattacttcttatttttcttaccaattgtgaatgttggtgtgaaacaaattaatgaagcttttgaatcatccctattctgtgttttatctagtcacataaatggattaattactaatttcagttgagaccttctaattggtttttactgaaacattgagggaacacaaatttatgggcttcctgatgatgattcttctaggcatcatgtcctatagtttgtcatccctgatgaatgtaaagttacactgttcacaaaggttttgtctcctttccactgctattagtcatggtcactctccccaaaatattatattttttctataaaaagaaaaaaatggaaaaaaattacaaggcaatggaaactattataaggccatttccttttcacattagataaattactataaagactcctaatagcttttcctgttaaggcagacccagtatgaaatggggattattatagcaaccattttggggctatatttacatgctactaaatttttataataattgaaaagattttaacaagtataaaaaattctcataggaattaaatgtagtctccctgtgtcagactgctctttcatagtataactttaaatcttttcttcaacttgagtctttgaagatagttttaattctgcttgtgacattaaaagattatttgggccagttatagcttattaggtgttgaagagaccaaggttgcaaggccaggccctgtgtgaacctttgagctttcatagagagtttcacagcatggactgtgtccccacggtcatccagtgttgtcatgcattggttagtcaaaatggggagggactagggcagtttggatagctcaacaagatacaatctcactctgtggtggtcctgctgacaaatcaagagcattgcttttgtttcttaagaaaacaaactcttttttaaaaattacttttaaatattaactcaaaagttgagattttggggtggtggtgtgccaagacattaattttttttttaaacaatgaagtgaaaaagttttacaatctctaggtttggctagttctcttaacactggttaaattaacattgcataaacacttttcaagtctgatccatatttaataatgctttaaaataaaaataaaaacaatccttttgataaatttaaaatgttacttattttaaaataaatgaagtgagatggcatggtgaggtgaaagtatcactggactaggaagaaggtgacttaggttctagataggtgtcttttaggactctgattttgaggacatcacttactatccatttcttcatgttaaaagaagtcatctcaaactcttagttttttttttttacaactatgtaatttatattccatttacataaggatacacttatttgtcaagctcagcacaatctgtaaatttttaacctatgttacaccatcttcagtgccagtcttgggcaaaattgtgcaagaggtgaagtttatatttgaatatccattctcgttttaggactcttcttccatattagtgtcatcttgcctccctaccttccacatgccccatgacttgatgcagttttaatacttgtaattcccctaaccataagatttactgctgctgtggatatctccatgaagttttcccactgagtcacatcagaaatgccctacatcttatttcctcagggctcaagagaatctgacagataccataaagggatttgacctaatcactaattttcaggtggtggctgatgctttgaacatctctttgctgcccaatccattagcgacagtaggatttttcaaacctggtatgaatagacagaaccctatccagtggaaggagaatttaataaagatagtgctgaaagaattccttaggtaatctataactaggactactcctggtaacagtaatacattccattgttttagtaaccagaaatcttcatgcaatgaaaaatactttaattcatgaagcttactttttttttttggtgtcagagtctcgctcttgtcacccaggctggaatgcagtggcgccatctcagctcactgcaacctccatctcccaggttcaagcgattctcgtgcctcggcctcctgagtagctgggattacaggcgtgtgccactacactcaactaatttttgtatttttaggagagacggggtttcaccctgttggccaggctggtctcgaactcctgacctcaagtgattcacccaccttggcctcataaacctgttttgcagaactcatttattcagcaaatatttattgagtgcctaccagatgccagtcaccgcacaaggcactgggtatatggtatccccaaacaagagacataatcccggtccttaggtagtgctagtgtggtctgtaatatcttactaaggcctttggtatacgacccagagataacacgatgcgtattttagttttgcaaagaaggggtttggtctctgtgccagctctataattgttttgctacgattccactgaaactcttcgatcaagctactttatgtaaatcacttcattgttttaaaggaataaacttgattatattgtttttttatttggcataactgtgattcttttaggacaattactgtacacattaaggtgtatgtcagatattcatattgacccaaatgtgtaatattccagttttctctgcataagtaattaaaatatacttaaaaattaatagttttatctgggtacaaataaacaggtgcctgaactagttcacagacaaggaaacttctatgtaaaaatcactatgatttctgaattgctatgtgaaactacagatctttggaacactgtttaggtagggtgttaagacttacacagtacctcgtttctacacagagaaagaaatggccatacttcaggaactgcagtgcttatgaggggatatttaggcctcttgaatttttgatgtagatgggcatttttttaaggtagtggttaattacctttatgtgaactttgaatggtttaacaaaagatttgtttttgtagagattttaaagggggagaattctagaaataaatgttacctaattattacagccttaaagacaaaaatccttgttgaagtttttttaaaaaaagctaaattacatagacttaggcattaacatgtttgtggaagaatatagcagacgtatattgtatcatttgagtgaatgttcccaagtaggcattctaggctctatttaactgagtcacactgcataggaatttagaacctaacttttataggttatcaaaactgttgtcaccattgcacaattttgtcctaatatatacatagaaactttgtggggcatgttaagttacagtttgcacaagttcatctcatttgtattccattgattttttttttcttctaaacattttttcttcaaacagtatataactttttttaggggatttttttttagacagcaaaaactatctgaagatttccatttgtcaaaaagtaatgatttcttgataattgtgtagtaatgttttttagaacccagcagttaccttaaagctgaatttatatttagtaacttctgtgttaatactggatagcatgaattctgcattgagaaactgaatagctgtcataaaatgaaactttctttctaaagaaagatactcacatgagttcttgaagaatagtcataactagattaagatctgtgttttagtttaatagtttgaagtgcctgtttgggataatgataggtaatttagatgaatttaggggaaaaaaaagttatctgcagatatgttgagggcccatctctccccccacacccccacagagctaactgggttacagtgttttatccgaaagtttccaattccactgtcttgtgttttcatgttgaaaatacttttgcatttttcctttgagtgccaatttcttactagtactatttcttaatgtaacatgtttacctggaatgtattttaactatttttgtatagtgtaaactgaaacatgcacattttgtacattgtgctttcttttgtgggacatatgcagtgtgatccagttgttttccatcatttggttgcgctgacctaggaatgttggtcatatcaaacattaaaaatgaccactcttttaattgaaattaacttttaaatgtttataggagtatgtgctgtgaagtgatctaaaatttgtaatatttttgtcatgaactgtactactcctaattattgtaatgtaataaaaatagttacagtgacaaaaaaaaaaaaaaa

SEQ ID NO: 4 - protein, 188 aa, Homo sapiens [sequence omitted]

SEQ ID NO: 5 - DNA, 661 bp, Rattus norvegicus
atgactgagtataaacttgtggtagttggagctggtggcgtaggcaagagtgccttgacgatacagctaattcagaatcactttgtggatgaatatgatcctacgatagaggactcctacaggaaacaagtagtaattgatggagaaacctgtctcttggatattctcgacacagcaggtcaagaggagtacagtgcaatgagggaccagtacatgagaactggggagggctttctttgtgtatttgccataaataatactaaatcatttgaagatattcaccattatagagaacaaattaaaagagtaaaggactctgaagatgtgcctatggtcctagtagggaataagtgtgacttgccttctagaacagtagacacgaaacaggctcaggagttagcaaggagttatgggattccattcattgagacctcagcgaagacaagacagggtgttgacgatgccttctatacattagtccgagaaattcgaaaacataaagaaaagatgagcaaagatgggaaaaagaagaagaagaagtcaaggacaaggtgtatagtcatgtgaatagtttgtactctttcttaaggcacacttaagtaaagtgtgatttttgtacattacactaaattattagcatttgttttagcattacctaatc

SEQ ID NO: 6 - protein, 188 aa, Rattus norvegicus
MTEYKLVVVGAGGVGKSALTIQLIQNHFVDEYDPTIEDSYRKQVVIDGETCLLDILDTAGQEEYSAMRDQYMRTGEGFLCVFAINNTKSFEDIHHYREQIKRVKDSEDVPMVLVGNKCDLPSRTVDTKQAQELARSYGIPFIETSAKTRQGVDDAFYTLVREIRKHKEKMSKDGKKKKKKSRTRCIVM

SEQ ID NO: 7 - DNA, 4670 bp, Mus musculus
aggcggcggccgcggcggctgaggcggcagcgctgtggcggcggctgagacggcaggggaaggcggcggcggctcggcccggagtcccgctcccgcgccatttcggacccggagcgagcgcggcgcgggcctgaaggcggcggcgggagcctgaggcgcggcggctccgcggcgcggagagaggcctgctgaaaatgactgagtataaacttgtggtggttggagctggtggcgtaggcaagagcgccttgacgatacagctaattcagaatcactttgtggatgagtatgaccctacgatagaggactcctacaggaaacaagtagtaattgatggagaaacctgtctcttggatattctcgacacagcaggtcaagaggagtacagtgcaatgagggaccagtacatgagaactggggagggctttctttgtgtatttgccataaataatactaaatcatttgaagatattcaccattatagagaacaaattaaaagagtaaaggactctgaagatgtgcctatggtcctggtagggaataagtgtgatttgccttctagaacagtagacacgaaacaggctcaggagttagcaaggagttacgggattccgttcattgagacctcagcaaagacaagacagggtgttgacgatgccttctatacattagtccgagaaattcgaaaacataaagaaaagatgagcaaagatgggaagaagaagaagaagaagtcaaggacaaggtgtacagttatgtgaatactttgtactctttcttaaggcacacttaagtaaaagtgtgatttttgtacattacactaaattattagcatttgttttagcattacctaatctttttttttcttctgttcgtgcaaactgtcagcttttatctcaaatgcttattttaaaagaacagtggaaaccttcttttttctaagtgccagtattccctgggttttggacttaaactagcaatgcctgtggaagagactaaagacctgagactctgtcttgggatttggtgcatgcagttgattccttgctagttctcttaccaactgtgaacactgatgggaagcaggataatgaagcttccggaccatccctgctctgtgtccatctactcatccaatggagtcattagcagtcaatcgccgcttcactggacactgaggggtcacagacttaggctccctttgagtcgcgtccagcgtgtcctagactttatcatctttcagaggcgtaggcagactgttcacaaaggctttctgtagctttccactgcaattaatcttggtcactccctcaaatagtatattttttctagaaaaggggaaaaatggaaaaaaaaaggcaatggaaaatgttgaaatccattcagtttccatgttagctaaattactgtaagattcctataatagcttttcctggtaaggcagacccagtatgaaatagtaataaccatttgggctatatttacatgctactaaatttttgtaataattcaaacaactttagcatatataaaaagttctcataagaattaagtacaattcccctttgtcagattgttcttatcctaactttcaagtcttttttgaatttctgttgttgaaagtagttttaatggttgtgaagctgaagatgatctgagacagttatagcttggcaggtgttgaggagaccagagttgcagggttgggccttacgtgaacctgtgacgaacgctactgggttttgcagcactgctgcattcaatgttggcgacgcattgtttggtcaacataggggataaggagactttgatggcttagtataatgcattctcaccatgtaacagtcctactgacaaatcaagaaatttgtttataataataaaaaatttttaaaaatttcgatgttcgcttcaaggttgagattttggggtaggaggctacaacaagagtaaatcttaaagcaaggttttaagaaggtttgaaaatgcaggtttgactagtctctcaactctagctaaacaaacattcccaagtacttcccaaatctgataggtatttaaaattatctaatgctttaagaatagttaacaggaaaaaaatctcctcagtgcacttaaagcaacccttcacatcatttgaaatgagatggaaatatcactggactatgaggactggatgtctgtctgattttaagcaaatcactgtctgcttggttttgaatcatctcaaagacattaacctcccagccgtgtaacatagtttacatgttgacacacctagttatcaagctcagcacaatctgtaactgttttacatggattaacatcttcactgccagtcttgggcaaattgtgcaagaggtaaaatttatatttcagtatccattctcccatttcaggactcccctccaacattatgctggctttcagcctgtctctcacctgcccatcacttagtgtagttttaataatttcccccacttcaaactttgtttccactatggacaacttcatgaactttgcccactaaggtaggtacatcaaagctgccctatggctttcttccccgggactgaaaataacagacaccatagtgggatttaaactaatagatggttttcagggccactacaacaattcaatctcaatcctttggacttcattcctgctgcccaggccactggtgcctcagtaggaattttcaaaattagtgtgaacagacagagcacagtccagtggaaggtgagcttaatcttcatctagccatcatcatggtaagtgatagattctattgttttaataaatacagtctaacaatgaaaaacacttcgaagtttcaatcataaagctgtctttttaaaaattttatttactcaacatttattcagtgcttgtcatattctgggaattacactaggcactcagggtgcggtgtcctcaatccttggccagtggtatgtagcatgatctgtaataccactaaataaggcatatagcatatgacttagacataatgaaatacatgatttgagttttgcagagaggagtttgggtttgtacattcccttcccccccagtttagcaagaattgtttgctgtgaatccaatgcaacttttaaatcaaactactttatataattatttcatttttctaaaggaacagaagtaccctaaactatttttttgaaatgttctaaactgtacatattcatagaacattctttgggtgaattttaagtcttaaaatgcaattagtaatacttctcatttctattcagaggaacaggtgtacttcaaaagctgcagtgtataatcagatatttttaatggacaatgtgttaaagaagtggtaattaccactatgtaaatttgaattgtgttacactttggttaacaaaaggggaaagaatcctagaaacaaatatgttatctagttactgcagccttaaagtccttgttgaagttaaaaagcaatgctaagttacagtcataggcattaacatgtttatgggaaggatatagtaggcaaatacaatttgagtaaatattttcagtagggaattttaggctctactgactgagtcacactgcataggaatttagatcttaacttttataggttatcgacctttgccaccattgcacaattttgtcctaacataaatacaagttctgtgaggcatgtcaaaagttacagtttgcataaattcatctcattttgtattccactgattttacattttcctcaaacatacatacatacatacatacaacacacacacactcacacatgaagggttttttttttgtaggcaataaaaatttaactaatttccatttgttaaaaagtagtgatttattgagaattatgcagtcattttttaaacccaaaagttatttaaaggtgaatttatactcaataacttctgtgtaatactgggtagcatgaattctgcattgaaaaattgaacagataataccaatagctgtaaattctgtcaaaacatgaaaattatttctaaagaagtacattagttttcaaagaacagttattagaatcagatctgtggtttagttcaataatttgaagtgcctgtttgggatggtggtaggcattttagatgaatttgggaaaaataaagttctgcagaaatgccagtttcagaccccgctaacccgctgagtgggctgtgtgctgtgttagctccagtgccccaatcccgtttcatgtcttcatgttgaaacacttctgcatttttatttgagtgccaatttcttactagtgctatttcttagtgtaacatgtttacctgggatgtattttaactatttttgtatagtgtaaactgaaacatgcacattttgtacattgtgctttccttctttccattccttttctttctgttttgtttgtttgtttgtttgtttgtttgttatgggacatatgcagtgtgatccagttgttttccatcctttggttgcgctgacctagggaatgttggtcatatcaaacattaaatttaaaagtgaccactcttaattaaaattaacttttaaatgtttataggagtacgtgctgtgaagtgatctgaaatttgtaatatttttgtcatgaaccgtactgctcctaatcattgtaatgtaataaaaatagttatggtgactatgaa

SEQ ID NO: 8 - protein, 188 aa, Mus musculus
MTEYKLVVVGAGGVGKSALTIQLIQNHFVDEYDPTIEDSYRKQVVIDGETCLLDILDTAGQEEYSAMRDQYMRTGEGFLCVFAINNTKSFEDIHHYREQIKRVKDSEDVPMVLVGNKCDLPSRTVDTKQAQELARSYGIPFIETSAKTRQGVDDAFYTLVREIRKHKEKMSKDGKKKKKKSRTRCTVM

SEQ ID NO: 9 - DNA, 2068 bp, Oryctolagus cuniculus
acacacgcgcccacccagccacccggccaccagccgccatgggcaaggacaggcagccccgcgggcagcagaggcagggggacgccgccgggcccgacgacccggggccgaagaaaggcgccgggacccgcgagcagcgcggggaggaggaggcccagacgtgctgcggctgccgcttcccgctgctgctcgcgctgctgcagctggccctgggcgtcgccgtgaccgtggtgggcttcctcatggcgagcgtcagctcctccctgctagtcagagccactccatattgggctgggatcattgtctgcgtggtggcctatcttggcttgtttatgctttgtgtctcgtaccaagttgatgaacggacgtgtatccagttttctatgaaactgctgtacttcgtgctgagcgccctggggctggtggtgtgcgtgctggccgtggccttcgccgcccaccactactcgctgctcacgcacctgacctgtgagaacgcccccgactcctgccagtgcaagctgccgtcctcggagccgctgagccggaccttcgtgtaccgggatgtgactgactgtaccagcatcacgggcaccttccaggtgttcctgctcgtccagatggttctgaacttggtctgtggccttgtgtgcttggtggcctgctttgtgatgtggaaacacaggtatcaggtcttttatgtgggggtcaggatgtgccccctgtcggcttccgaaggccagcagcagaaggtgtaggaatcttgctcagaattgggagagaaaatggcacactggctagctgaggttaaaaagaaaaattatttttaaggagaaagagagaaaacttttgccaatatttactgctctaaatgaatattttttatatttttcaagaaacaaaagagcatttcttcaggtttctattgtatttttaaacattcgtataggttcaacaagatacacattgatttgcgggatattcaaagtcaaaagcacaccaaactgggaagcaatggcacagaactgtcctcacagtctggggtttactcttcatgctcactttcgccaccactgacgtacggctttctggttaatacggtctaaggtttgtagtggctgccccaggtccttcccgcctcctaccacaatcccccactgcgtcttagagaaaggcaaggtgtggagaagtcactgggcaaccaggtggaatctcttcatttcccctactgcggatgttgtcaaggcccaaaacatgagcgaacttcaaaaacctcatgggaagtggagttcgaagtttattttgctgccaaaaaattaagatccacacatatatagggatcttcagaaagttcacagaaaatgcataatatgggaaaaaaaaagattcacggatttcagaattttgtttggaccaaactaaagttatcttttaatgccatttctgaagtgccctcatagcttggaaagccaagcagaaaagaggctttgcaaaaatacaagtaattataaacacctgggccagggcggctgtctcagctgccttcgcttggctctgtacgtagatcactcgcgcggggcttggcagggctctctgcttctcaataattgaaatatggtggtagttgtattcttaatgatgtagaaggtttaaaaataattacattacgcttccattctatcatctacaacaaatcattcaacctaatttctagctaattgttaattataattatgctcagaagtctatttaatgagctctggctgtacttaggcagctctgccagtgtaaagagaaattattctcgtaagagaagaggcctaaagattctttcttctgaaagtcaagcgttataagggaaaacttttttttaattaatagctcaggataaaaacaccaatttaaacaaaaacaagagcatttataataggaagtacttgtacaaatagcacgtttgtggcacattgcagagtgtctctctttgcagctaaatagctttgaagaaggctggcgagtgcagatgtattctgtgcacaaaactgtatttggctcataaccctattattgattc

SEQ ID NO: 10 - protein, 238 aa, Oryctolagus cuniculus
MGKDRQPRGQQRQGDAAGPDDPGPKKGAGTREQRGEEEAQTCCGCRFPLLLALLQLALGVAVTVVGFLMASVSSSLLVRATPYWAGIIVCVVAYLGLFMLCVSYQVDERTCIQFSMKLLYFVLSALGLVVCVLAVAFAAHHYSLLTHLTCENAPDSCQCKLPSSEPLSRTFVYRDVTDCTSITGTFQVFLLVQMVLNLVCGLVCLVACFVMWKHRYQVFYVGVRMCPLSASEGQQQKV

SEQ ID NO: 11 - DNA, 1039 bp, Cavia porcellus
ggtggcttctcggccagacctcccggcccccgccatttcggaccgggagccagcgcgacgcgggcactgagggcggcggcgggggccacaggctcggcggctcccaggtgcgggagagaggcctgctgaaaatgactgaatataaacttgtggtagttggagctggtggcgtaggcaagagtgccttgacgatacagctaattcagaatcactttgtggatgaatatgatcctacaatagaggattcctacaggaaacaagtagtaattgatggagaaacctgtctcttggatattctcgacacagcaggtcaagaggagtacagtgcaatgagggaccagtacatgaggactggggagggctttctttgtgtatttgccataaataatactaaatcttttgaagatattcaccattatagagaacaaattaaaagagttaaagactctgaagatgtacctatggtcctagtaggaaataaatgtgatttgccttctagaacagtagacacaaaacaagctcaggacttagcaagaagttatggaattccttttattgaaacatcagcaaagacaagacagagagtggaggatgctttttatacattggtgagagagattcgacaatacagattgaaaaaaatcagcaaagaagaaaagactcctggctgtgtgaaaattaaaaaatgcattataatgggtgttgatgatgccttctatacgttagttcgagaaattcgaaaacataaagaaaagatgagcaaagatggtaaaaagaagaaaaagaagtcgaagacaaagtgtataattatgtaaatacaatttgtacttttttcttaaggcatacttaagtaaaagtggtaatttttgtacattacactaaattattagcttttgttttagcattacttaattcttttcctatttcatgcaaactgttagcttttatcttaaatgctcattttaaaatgacagtggaaaccttttatttcctcttaagtgccagtattccctgcattttggtttttgaactagcaatg

SEQ ID NO: 12 - protein, 227 aa, Cavia porcellus
MTEYKLVVVGAGGVGKSALTIQLIQNHFVDEYDPTIEDSYRKQVVIDGETCLLDILDTAGQEEYSAMRDQYMRTGEGFLCVFAINNTKSFEDIHHYREQIKRVKDSEDVPMVLVGNKCDLPSRTVDTKQAQDLARSYGIPFIETSAKTRQRVEDAFYTLVREIRQYRLKKISKEEKTPGCVKIKKCIIMGVDDAFYTLVREIRKHKEKMSKDGKKKKKKSKTKCIIM

SEQ ID NO: 13 - DNA, 835 bp, Cavia porcellus
acaggctcggcggctcccaggtgcgggagagaggcctgctgaaaatgactgaatataaacttgtggtagttggagctggtggcgtaggcaagagtgccttgacgatacagctaattcagaatcactttgtggatgaatatgatcctacaatagaggattcctacaggaaacaagtagtaattgatggagaaacctgtctcttggatattctcgacacagcaggtcaagaggagtacagtgcaatgagggaccagtacatgaggactggggagggctttctttgtgtatttgccataaataatactaaatcttttgaagatattcaccattatagagaacaaattaaaagagttaaagactctgaagatgtacctatggtcctagtaggaaataaatgtgatttgccttctagaacagtagacacaaaacaagctcaggacttagcaagaagttatggaattccttttattgaaacatcagcaaagacaagacagggtgttgatgatgccttctatacgttagttcgagaaattcgaaaacataaagaaaagatgagcaaagatggtaaaaagaagaaaaagaagtcgaagacaaagtgtataattatgtaaatacaatttgtacttttttcttaaggcatacttaagtaaaagtggtaatttttgtacattacactaaattattagcttttgttttagcattacttaattcttttcctatttcatgcaaactgttagcttttatcttaaatgctcattttaaaatgacagtggaaaccttttatttcctcttaagtgccagtattccctgcattttggtttttgaactagcaatg

SEQ ID NO: 14 - protein, 188 aa, Cavia porcellus
MTEYKLVVVGAGGVGKSALTIQLIQNHFVDEYDPTIEDSYRKQVVIDGETCLLDILDTAGQEEYSAMRDQYMRTGEGFLCVFAINNTKSFEDIHHYREQIKRVKDSEDVPMVLVGNKCDLPSRTVDTKQAQDLARSYGIPFIETSAKTRQGVDDAFYTLVREIRKHKEKMSKDGKKKKKKSKTKCIIM

SEQ ID NO: 15 - DNA, 4993 bp, Canis lupus familiaris
gctgaaaatgactgaatataaacttgtggtagttggagctggtggcgtaggcaagagtgccttgacgatacagctaattcagaatcactttgtggatgaatatgatcctacaatagaggattcctacaggaaacaagtagtaattgatggagaaacctgtctcttggatattctcgacacagcaggtcaagaggagtacagtgcaatgagggaccagtacatgaggactggggagggctttctttgtgtatttgccataaataatactaaatcatttgaagatattcaccattatagagaacaaattaaaagagttaaagactctgaagatgtacctatggtcctagtaggaaataaatgtgatttgccttctagaacagtagacacaaaacaggctcaggacttagcaagaagttatggaattccttttattgaaacatcagcaaagacaagacagagagtggaggatgctttttatacattggtgagagagatccgacaatacagattgaaaaaaatcaacaaagaagaaaagactcctggctgtgtgaaaattaaaaaatgcattgtaatgggtgttgacgatgccttctatacattagttcgagaaattcgaaaacataaagaaaagatgagcaaagatggtaaaaagaagaaaaagaagtcaaagacaaagtgtataattatgtaaatacaatttgtacttttttcttaaggcatacttaagtaaaagtggtaatttttgtacattacactaaattattagcatttgttttagcattacctaattttctgctccatccaaactgttagcttttatcttgaatgcttattttaaaatgacagtggaaactttttcctctaagtgccagtattccctgagttttggttttgaactagcaatgcctgtgaaaaagaaactgaatacctgagatttctgtcttggggtttttggtgcatgcagttgattacttcctatttttcttaccaattgtgaactttggtgtgaaacaaattaatgaagctttcgaatcatccctattctgtgttttacctagtcacatacatggattaattactaattataacttcagttgatatttcatgattggttttactgaaacattgagggaacatgaatttatgggctgcttcttataggtataatgtcctatagtttcagtcacccttaatgaatgtaaagctacactgttcacaaaggttttctccatcttttcactgctatttgtcatagccacgctcccaaaaatattatattttttctataaaaaagggaaaaaatagaaaaaaatacaaggcaatggaaaatattaaaaggcatttactttccatattagataaattcctataatactctgaatagcttttcctgttaaggcagacccagtatgtaatgaggattatagcaaccattttggggctatatttacatgctactaaatttttgtattaattgaaaaagttttaacatgtataaaaaattcccataggaattaaatatagtctccctgtgtcagattgctctttcttagcataactttaaatcttttcttgatcttcaatcttagaaaatagttttaattcttgtagtgatgttaaagattatttgggccagttagtttttaatagatgttaaagagaccacagttccaaggccaggccttgtgtgaacctttaagcttcattaagagtttcatagtacagactgcatccctgtggtctcccagggtcatcatgcattgattgggtggtcaaaagtggggacaaagagtgtttagataagatgcatcctcactgtatggtggtcctgctgacagatcaggaccatcacttttgttttttaaaaaaccaacagagctttttaaaaacattatttaaaatgagatttttgggggcagggggtggcaagacttgaattttttttaaacaatgaagtaaaaaggtttcaaaatctctagtgttggctagttctcaacattggctaaagtaacatttcataaacactttacaagtattggtccatatttaagaatatctaatgcttaaataatagattaataacaattctttcagtgcatttaaaatgtatttttaaatatctgaagtgagatggtgtgttgaggtgaaaatatcactggactaggaggaaggtgacttagattctagttacgtgtcttttacaacttcagttttgggcaaatcactcactatccatttcttcatgttaagtcatctcaaaggctatatctagcatcaactatgtgatttacattcagtttacataaggatatacctatttgtcaatctcagcacaatctgtaactttttacctatgttctcttcagcgccagtcttaggcaaagttgtgcaagaggtgaggtttatttttgagaatctgatctccggtagcaggtactcctctcccatgttagtgtcatcttgcctgcctaccttctacatgccccatgacttgatgctttctaattccccgaacctcaagatgtagtgctgctttggatatctccatgaggtaataagtcacattagtcaggctcaacataatctgacagatactgtagtgggatttgatctaatagctaattttcaggtggtaactgtatcaatttaattttgatcttttgaacatcatctctgctacctggtccattagtgactaagtaggaaaagtaggaattttcatatctgtgatgtgtagacagaccctatccagtagaagaatttaataaatttaattaataaatactgaaagatttccttagataatccaaaactaggactagccctggtaacggtgatacattccattattttaataagtaaaatcttcttacaatgaaaaatactttaaaatttaattcataaagcttactttttagcagaattcatttattcaacaaatacttgagtgcctgctagatgccaggttctacacaaggcaccggggatattatggtattcccaacaagggacataatccctatccttaagtagtactgttattttagagtggtctgtagtatattagtgaggcatttggcacatgacccagagataatataatgcatattttagttttgcacagaagggatatggtctctaaggttttttccagctctaaaataattgttcgctctgattccaataaactgtttaatcaagctactttatataaatcactttacttcattattttaaagaagtaaacttgactatattgttttttatttgggataattatgtgattctgttgggatacttatatagtacacattaaattgtatgtcagatgataacattaaaattcccaagtgtaatattctacttggtctctgtgtatcataattaaaatagatttaaatattgagttcaaaaatagttttatttatctgggtgtgaataaacagatgcctgaactaattcacagaaaaggaaacttctgtgtaaaaagtcagtccaatttctgaaatgctatgctaaactacaggtttatggaacattagatagggtgttaagactttatatagtacttcctcttgtttctatacaagagaaagaaatggccatacttcaggaattgcagtgcataactgagggatttttaggactcttgaatttttgatgtagccgggcaactttttttaggcagtggtaattatcctttattatgtgaattttgaatggtttgacaaaacgtttgtttttgtagagattttaaaaggggagcgctaatcctagaaataaatattatgtaattattacggccttaaagataaaaatccttgttgaaagttgaaaaaaattgctaaattacatagtcttagacattaacatgtttgtggaagaatgtagcagaggtatgtagtataatttgagtgaatattcccaattaggaattctaggctctagtttaactgagtcacactgcataggaatttagaacctaacttctaggttatcaaaatctttgccaccattgcacaattttgtcctaatatatagagaaactttgtgaggcatgttcagttgcggtttgcacaagttcatctcatttgtattccagtgattttttttcttctaaccatttttttaaacaacatgtacacattgttttttttggtaggcaatgaaaactgtcatttccattgtcaaacagtaattcctcgataactgtattaatggtttttaaaaaaccatcagttactttaaaactgaatttatatttaataacttctgtattagtattgggtagcatgaaatctctattgagaaattgaacagcatacaactagtagctgtaaattccttcagaaagtgaaaattatttcttcctaaagatatcttgacatcagtgcttgaagaatagtcataactagattaataattgttttagttaaacagttttaagtgcctgtttcagatgatgataggcaatttagatgaatttaggaaaaatcaaagtttttacttgcagaaatgtccattatagggggcccccctcctcatagagctgaatgggttatgtaatgttttatccaaaagtttccaattccactgtcttgtgttttcatgttgaaaatacttttgcatttttcctttgagtgccaatttcttactagtactatttcttaatgtaacatgtttacctggaatgtattttaactatttttgtatagtgtaaactgaaacatgcacattttgtacattgtgcttttttttgtgggacatatgcagtgtgatccagttgttttccatcatttggttgcgctgacctaggaatgttggtcatatcaaacattaaatttaaaaatgaccactcttttaattaaaattaacttttaaatgtttataggagtatgtgctgtgaagtgatctgaaatttgtaatatttttgtcatgaactgtactgctcctaattattgtaatgtaataaaaatagttatggtgactatga

SEQ ID NO: 16 - protein, 227 aa, Canis lupus familiaris
MTEYKLVVVGAGGVGKSALTIQLIQNHFVDEYDPTIEDSYRKQVVIDGETCLLDILDTAGQEEYSAMRDQYMRTGEGFLCVFAINNTKSFEDIHHYREQIKRVKDSEDVPMVLVGNKCDLPSRTVDTKQAQDLARSYGIPFIETSAKTRQRVEDAFYTLVREIRQYRLKKINKEEKTPGCVKIKKCIVMGVDDAFYTLVREIRKHKEKMSKDGKKKKKKSKTKCIIM

SEQ ID NO: 17 - DNA, 4876 bp, Canis lupus familiaris
gctgaaaatgactgaatataaacttgtggtagttggagctggtggcgtaggcaagagtgccttgacgatacagctaattcagaatcactttgtggatgaatatgatcctacaatagaggattcctacaggaaacaagtagtaattgatggagaaacctgtctcttggatattctcgacacagcaggtcaagaggagtacagtgcaatgagggaccagtacatgaggactggggagggctttctttgtgtatttgccataaataatactaaatcatttgaagatattcaccattatagagaacaaattaaaagagttaaagactctgaagatgtacctatggtcctagtaggaaataaatgtgatttgccttctagaacagtagacacaaaacaggctcaggacttagcaagaagttatggaattccttttattgaaacatcagcaaagacaagacagggtgttgacgatgccttctatacattagttcgagaaattcgaaaacataaagaaaagatgagcaaagatggtaaaaagaagaaaaagaagtcaaagacaaagtgtataattatgtaaatacaatttgtacttttttcttaaggcatacttaagtaaaagtggtaatttttgtacattacactaaattattagcatttgttttagcattacctaattttctgctccatccaaactgttagcttttatcttgaatgcttattttaaaatgacagtggaaactttttcctctaagtgccagtattccctgagttttggttttgaactagcaatgcctgtgaaaaagaaactgaatacctgagatttctgtcttggggtttttggtgcatgcagttgattacttcctatttttcttaccaattgtgaactttggtgtgaaacaaattaatgaagctttcgaatcatccctattctgtgttttacctagtcacatacatggattaattactaattataacttcagttgatatttcatgattggttttactgaaacattgagggaacatgaatttatgggctgcttcttataggtataatgtcctatagtttcagtcacccttaatgaatgtaaagctacactgttcacaaaggttttctccatcttttcactgctatttgtcatagccacgctcccaaaaatattatattttttctataaaaaagggaaaaaatagaaaaaaatacaaggcaatggaaaatattaaaaggcatttactttccatattagataaattcctataatactctgaatagcttttcctgttaaggcagacccagtatgtaatgaggattatagcaaccattttggggctatatttacatgctactaaatttttgtattaattgaaaaagttttaacatgtataaaaaattcccataggaattaaatatagtctccctgtgtcagattgctctttcttagcataactttaaatcttttcttgatcttcaatcttagaaaatagttttaattcttgtagtgatgttaaagattatttgggccagttagtttttaatagatgttaaagagaccacagttccaaggccaggccttgtgtgaacctttaagcttcattaagagtttcatagtacagactgcatccctgtggtctcccagggtcatcatgcattgattgggtggtcaaaagtggggacaaagagtgtttagataagatgcatcctcactgtatggtggtcctgctgacagatcaggaccatcacttttgttttttaaaaaaccaacagagctttttaaaaacattatttaaaatgagatttttgggggcagggggtggcaagacttgaattttttttaaacaatgaagtaaaaaggtttcaaaatctctagtgttggctagttctcaacattggctaaagtaacatttcataaacactttacaagtattggtccatatttaagaatatctaatgcttaaataatagattaataacaattctttcagtgcatttaaaatgtatttttaaatatctgaagtgagatggtgtgttgaggtgaaaatatcactggactaggaggaaggtgacttagattctagttacgtgtcttttacaacttcagttttgggcaaatcactcactatccatttcttcatgttaagtcatctcaaaggctatatctagcatcaactatgtgatttacattcagtttacataaggatatacctatttgtcaatctcagcacaatctgtaactttttacctatgttctcttcagcgccagtcttaggcaaagttgtgcaagaggtgaggtttatttttgagaatctgatctccggtagcaggtactcctctcccatgttagtgtcatcttgcctgcctaccttctacatgccccatgacttgatgctttctaattccccgaacctcaagatgtagtgctgctttggatatctccatgaggtaataagtcacattagtcaggctcaacataatctgacagatactgtagtgggatttgatctaatagctaattttcaggtggtaactgtatcaatttaattttgatcttttgaacatcatctctgctacctggtccattagtgactaagtaggaaaagtaggaattttcatatctgtgatgtgtagacagaccctatccagtagaagaatttaataaatttaattaataaatactgaaagatttccttagataatccaaaactaggactagccctggtaacggtgatacattccattattttaataagtaaaatcttcttacaatgaaaaatactttaaaatttaattcataaagcttactttttagcagaattcatttattcaacaaatacttgagtgcctgctagatgccaggttctacacaaggcaccggggatattatggtattcccaacaagggacataatccctatccttaagtagtactgttattttagagtggtctgtagtatattagtgaggcatttggcacatgacccagagataatataatgcatattttagttttgcacagaagggatatggtctctaaggttttttccagctctaaaataattgttcgctctgattccaataaactgtttaatcaagctactttatataaatcactttacttcattattttaaagaagtaaacttgactatattgttttttatttgggataattatgtgattctgttgggatacttatatagtacacattaaattgtatgtcagatgataacattaaaattcccaagtgtaatattctacttggtctctgtgtatcataattaaaatagatttaaatattgagttcaaaaatagttttatttatctgggtgtgaataaacagatgcctgaactaattcacagaaaaggaaacttctgtgtaaaaagtcagtccaatttctgaaatgctatgctaaactacaggtttatggaacattagatagggtgttaagactttatatagtacttcctcttgtttctatacaagagaaagaaatggccatacttcaggaattgcagtgcataactgagggatttttaggactcttgaatttttgatgtagccgggcaactttttttaggcagtggtaattatcctttattatgtgaattttgaatggtttgacaaaacgtttgtttttgtagagattttaaaaggggagcgctaatcctagaaataaatattatgtaattattacggccttaaagataaaaatccttgttgaaagttgaaaaaaattgctaaattacatagtcttagacattaacatgtttgtggaagaatgtagcagaggtatgtagtataatttgagtgaatattcccaattaggaattctaggctctagtttaactgagtcacactgcataggaatttagaacctaacttctaggttatcaaaatctttgccaccattgcacaattttgtcctaatatatagagaaactttgtgaggcatgttcagttgcggtttgcacaagttcatctcatttgtattccagtgattttttttcttctaaccatttttttaaacaacatgtacacattgttttttttggtaggcaatgaaaactgtcatttccattgtcaaacagtaattcctcgataactgtattaatggtttttaaaaaaccatcagttactttaaaactgaatttatatttaataacttctgtattagtattgggtagcatgaaatctctattgagaaattgaacagcatacaactagtagctgtaaattccttcagaaagtgaaaattatttcttcctaaagatatcttgacatcagtgcttgaagaatagtcataactagattaataattgttttagttaaacagttttaagtgcctgtttcagatgatgataggcaatttagatgaatttaggaaaaatcaaagtttttacttgcagaaatgtccattatagggggcccccctcctcatagagctgaatgggttatgtaatgttttatccaaaagtttccaattccactgtcttgtgttttcatgttgaaaatacttttgcatttttcctttgagtgccaatttcttactagtactatttcttaatgtaacatgtttacctggaatgtattttaactatttttgtatagtgtaaactgaaacatgcacattttgtacattgtgcttttttttgtgggacatatgcagtgtgatccagttgttttccatcatttggttgcgctgacctaggaatgttggtcatatcaaacattaaatttaaaaatgaccactcttttaattaaaattaacttttaaatgtttataggagtatgtgctgtgaagtgatctgaaatttgtaatatttttgtcatgaactgtactgctcctaattattgtaatgtaataaaaatagttatggtgactatga

SEQ ID NO: 18 - protein, 188 aa, Canis lupus familiaris; identical to SEQ ID NO: 14

SEQ ID NO: 19 - DNA, 1394 bp, Felis catus
gctgaaaatgactgaatataaacttgtggtagttggagctggtggcgtaggcaagagtgccttgacgatacagctaattcagaatcactttgtggatgaatatgatcctacaatagaggattcctacaggaaacaagtagtaattgatggagaaacctgtctcttggatattctcgacacagcaggtcaagaggagtacagtgcaatgagggaccagtacatgaggactggggagggctttctttgcgtatttgccataaataatactaaatcatttgaagatattcaccactatagagaacaaataaaaagagttaaagactctgaagatgtacctatggtcctagtaggaaataaatgtgatttgccttctagaacagtagatacaaaacaggctcaggacttagcaagaagttatggaattccttttattgaaacatcagcaaagacaagacagggtgttgacgatgccttctatacattagttcgagaaattcgaaaacataaagaaaagatgagcaaagatggtaaaaagaagaaaaagaagtcaaagacaaagtgtataattatgtaaatacaatttgtacttttttcttaaggcatacttaagtaaaagtggtaatttttgtacattacactaaattattagcatttgttttagcattacctaattttctgctccatccaaactgttagcttttatcttgaatgcttattttaaatgacagtggaaactttttttcctctaagtgccagtattccctgagttttggtttttgaactagcaatgcctgtgaaaaagaaactgaatacctgagatttctgtcttggggtttttggtgcatgcagttgattacttcctatttttcttaccaattgtgaactttggtgtgaaacaaattaatgaaactttcgaatcatccctattctgtgtttcatgtagtcacatacatggattaattactaattataacttcagttgagatttcatgattcgttttactgaaacattgagggaacatgaatttatgggcttcttgtagattcatcttgtaggtattaatgtcctatagtttcagtcacccttaatgaatgtaaagttacactgttcataaaagtttctccatcttttcactgctgtttgtcatcgtcacgctcccccaaaatattatattttttctataaaaagggaaaaaaggaaaaaaatacaaggcaatggaaaatattaaaaggcatttactttctgtattagataaattcctataatactctgaatagcttttcctgttaaggcagacccagtatgtgatgaggattatagcaaccattttggggctatatttacatgctactaaatttttgtaataattgaaaaaattttaacatgtataaaa

SEQ ID NO: 20 - protein, 188 aa, Felis catus; identical to SEQ ID NO: 14

SEQ ID NO: 21 - DNA, 1512 bp, Felis catus
tgctgaaaatgactgaatataaacttgtggtagttggagctggtggcgtaggcaagagtgccttgacgatacagctaattcagaatcactttgtggatgaatatgatcctacaatagaggattcctacaggaaacaagtagtaattgatggagaaacctgtctcttggatattctcgacacagcaggtcaagaggagtacagtgcaatgagggaccagtacatgaggactggggagggctttctttgcgtatttgccataaataatactaaatcatttgaagatattcaccactatagagaacaaataaaaagagttaaagactctgaagatgtacctatggtcctagtaggaaataaatgtgatttgccttctagaacagtagatacaaaacaggctcaggacttagcaagaagttatggaattccttttattgaaacatcagcaaagacaagacagagagtggaggatgctttttatacattggtgagagagatccgacagtacagattgaaaaaaatcaacaaagaagaaaagactcctggctgtgtgaaaattaaaaaatgcattgtaatgggtgttgacgatgccttctatacattagttcgagaaattcgaaaacataaagaaaagatgagcaaagatggtaaaaagaagaaaaagaagtcaaagacaaagtgtataattatgtaaatacaatttgtacttttttcttaaggcatacttaagtaaaagtggtaatttttgtacattacactaaattattagcatttgttttagcattacctaattttctgctccatccaaactgttagcttttatcttgaatgcttattttaaatgacagtggaaactttttttcctctaagtgccagtattccctgagttttggtttttgaactagcaatgcctgtgaaaaagaaactgaatacctgagatttctgtcttggggtttttggtgcatgcagttgattacttcctatttttcttaccaattgtgaactttggtgtgaaacaaattaatgaaactttcgaatcatccctattctgtgtttcatgtagtcacatacatggattaattactaattataacttcagttgagatttcatgattcgttttactgaaacattgagggaacatgaatttatgggcttcttgtagattcatcttgtaggtattaatgtcctatagtttcagtcacccttaatgaatgtaaagttacactgttcataaaagtttctccatcttttcactgctgtttgtcatcgtcacgctcccccaaaatattatattttttctataaaaagggaaaaaaggaaaaaaatacaaggcaatggaaaatattaaaaggcatttactttctgtattagataaattcctataatactctgaatagcttttcctgttaaggcagacccagtatgtgatgaggattatagcaaccattttggggctatatttacatgctactaaatttttgtaataattgaaaaaattttaacatgtataaaa

SEQ ID NO: 22 - protein, 227 aa, Felis catus; identical to SEQ ID NO: 16

SEQ ID NO: 23 - DNA, 2144 bp, Bos taurus
ggcggtggcggcggcggcggcggtggcggtggcggttcggccagtactcccggcccccgccatttctgactgggagcgagcgcggcgcaggcactgaaggcagcggcgggggccagaggctcggcggctcccaggtgagggagagaggcctgctgaaaatgactgaatataaacttgtggtagttggagctggtggcgtaggcaagagtgccttgacgatacagctaattcagaatcactttgtggatgaatatgatcctacgatagaggattcctacaggaaacaagtagtaattgatggagaaacctgtctcttggatattctcgacacagcaggtcaagaggagtacagtgcaatgagggaccagtacatgaggactggggagggctttctttgtgtatttgccataaataatactaaatcatttgaagatattcaccattatagagaacaaataaaaagagttaaagactctgaagatgtacctatggttctagtaggaaataaatgtgatttgccttctagaacagtagacacaaaacaggctcaggacttagcaagaagttatggaattccttttattgaaacatcagcaaagacaagacagggtgttgacgatgccttctatacattagttcgagaaattcgaaaacataaagaaaagatgagcaaagatggtaaaaagaagaaaaagaagtcaaagacaaagtgtataattatgtaaatacaatttgtacttttttcttaaggcatacttaagtaaaagtggtaatttttgtatattacactaaattattagcatttgttttagcattatctaattttctttctgctccatccatactgttagcttttatcttgaatgcttattttaaaatgacagtggaaacttttttcctctaagtgccagtattccctgcgttttggtttttgaactagcaatgcctgtgaaaaagaaactgaacacccaagatttttgtcttggggtttttggtgcatgcagttgattacttcctatttttcttatcaattgtgaactttagtgtgaaacaaattaatgaggctttcaaatcatccctattgtattgttttatctagtcacacacatggattaattactaattataacttcagttgagatttcatgattggttttactgaaacatcgagggaacatgaatttatgggcttcctatagtttcatcttgtaggtatcattgtcctatagtttcagttacccttaatgaatgtcaggttacactgttcacaaaggttttcttctttccactgctatttgtcaaatggtcacgttccctaaaatactatattttttctataaaaaaaagaaaaaaatggaaaaaaatacaaggcaatggaaaatattaaaaggccacttactttccacattaggtaaattcctataatgctctgaatagctttttatgttaaggcagacccagtaggtaatgaggattagaacaagcattttgggactatatttacatgctttaaatttttgtaataacaaaaaaattttaacatgtataaagaattctcataggaattaaatacagtctccctgtgtcagattgctctttcttagcataaatctttttcttgaacttcaatctttaaaagtagttttaattctactgatagtgatgtaaaagattatttgggccagttagcttggtaggtgttacagagaccagggtggcatagccgggccttgtgtgaacctttaagctacatggagagtttcacagtgtggactgcatccctgtggtcttccattgttgccatgccttggttggtcaaaaacaaggacttgcagagagattgaatagctcagcaaggtacattctcattatgtcgtagtcctactcaggaacatcacttttttaaaataaaaaaccccaaaaaacagaacttaaaaaaaaaaacaacattattttaaatgagattttcggtggggtggaaagattttaattttttttaaacgatgaaatgaaaaaatgtcaaaatcttgagtattggctagttctctttaacactggctaaagtaacatttttgtaaacacttcagtacagtctggtccattattaagaatatctaatgcttatacaataaagtaatgctaac

SEQ ID NO: 24 - protein, 188 aa, Bos taurus; identical to SEQ ID NO: 14

SEQ ID NO: 25 - DNA, 1010 bp, Bos taurus
ggcggtggcggcggcggcggcggtggcggtggcggttcggccagtactcccggcccccgccatttctgactgggagcgagcgcggcgcaggcactgaaggcagcggcgggggccagaggctcggcggctcccaggtgagggagagaggcctgctgaaaatgactgaatataaacttgtggtagttggagctggtggcgtaggcaagagtgccttgacgatacagctaattcagaatcactttgtggatgaatatgatcctacgatagaggattcctacaggaaacaagtagtaattgatggagaaacctgtctcttggatattctcgacacagcaggtcaagaggagtacagtgcaatgagggaccagtacatgaggactggggagggctttctttgtgtatttgccataaataatactaaatcatttgaagatattcaccattatagagaacaaataaaaagagttaaagactctgaagatgtacctatggttctagtaggaaataaatgtgatttgccttctagaacagtagacacaaaacaggctcaggacttagcaagaagttatggaattccttttattgaaacatcagcaaagacaagacagagagtggaggatgctttttatacattggtgagagagatccgacaatacagattgaaaaaaatcagcaaagaagaaaagactcctggctgtgtgaaaattaaaaaatgcattgtaatgggtgttgacgatgccttctatacattagttcgagaaattcgaaaacataaagaaaagatgagcaaagatggtaaaaagaagaaaaagaagtcaaagacaaagtgtataattatgtaaatacaatttgtacttttttcttaaggcatacttaagtaaaagtggtaatttttgtatattacactaaattattagcatttgttttagcattatctaattttctttctgctccatccatactgttagcttttatcttgaatgcttattttaaaatgacagtggaaactt

SEQ ID NO: 26 - protein, 227 aa, Bos taurus
MTEYKLVVVGAGGVGKSALTIQLIQNHFVDEYDPTIEDSYRKQVVIDGETCLLDILDTAGQEEYSAMRDQYMRTGEGFLCVFAINNTKSFEDIHHYREQIKRVKDSEDVPMVLVGNKCDLPSRTVDTKQAQDLARSYGIPFIETSAKTRQRVEDAFYTLVREIRQYRLKKISKEEKTPGCVKIKKCIVMGVDDAFYTLVREIRKHKEKMSKDGKKKKKKSKTKCIIM

SEQ ID NO: 27 - DNA, 797 bp, Bos taurus
gcggtggcggcggcggcggcggtggcggtggcggttcggccagtactcccggcccccgccatttctgactgggagcgagcgcggcgcaggcactgaaggcagcggcgggggccagaggctcggcggctcccaggtgagggagagaggcctgctgaaaatgactgaatataaacttgtggtagttggagctggtggcgtaggcaagagtgccttgacgatacagctaattcagaatcactttgtggatgaatatgatcctacgatagaggattcctacaggaaacaagtagtaattgatggagaaacctgtctcttggatattctcgacacagcaggtcaagaggagtacagtgcaatgagggaccagtacatgaggactggggagggctttctttgtgtatttgccataaataatactaaatcatttgaagatattcaccattatagagaacaaataaaaagagttaaagactctgaagatgtacctatggttctagtaggaaataaatgtgatttgccttctagaacagtagacacaaaacaggctcaggacttagcaagaagttatggaattccttttattgaaacatcagcaaagacaagacagagagtggaggatgctttttatacattggtgagagagatccgacaatacagattgaaaaaaatcagcaaagaagaaaagactcctggctgtgtgaaaattaaaaaatgcattgtaatgtaatctgggtgttgacgatgccttctatacattagttcgagaaattcgaaaacataaagaaaagatgagcaaa

SEQ ID NO: 28 - protein, 189 aa, Bos taurus
MTEYKLVVVGAGGVGKSALTIQLIQNHFVDEYDPTIEDSYRKQVVIDGETCLLDILDTAGQEEYSAMRDQYMRTGEGFLCVFAINNTKSFEDIHHYREQIKRVKDSEDVPMVLVGNKCDLPSRTVDTKQAQDLARSYGIPFIETSAKTRQRVEDAFYTLVREIRQYRLKKISKEEKTPGCVKIKKCIVM

SEQ ID NO: 29 - DNA, 1112 bp, Gallus gallus
caggtctgctaaaaaatgacagagtataagcttgttgtcgttggagctggtggtgtgggcaagagcgccttgacaatacagctcattcagaaccactttgtggatgagtatgaccctaccatagaggattcctacagaaagcaagtagtaattgatggggaaacctgtctcttggatattcttgatacagcaggtcaagaagaatatagtgcaatgagggaccaatatatgagaacaggagaaggctttctgtgtgtttttgctataaacaatacaaaatcttttgaagatattcaccattatagggaacaaataaagagagttaaagactctgaagatgtcccaatggtgctagtaggaaacaaatgtgatttgccttccagaacagtagatacaaaacaagctcaggatttagcaagaagttatggaattccttttattgaaacatcagcaaagacaagacagggtgttgatgatgccttctatacattagttcgagaaatcagaaaacacaaagagaagatgagcaaagatggtaaaaagaagaaaaagaagacaaagacaaagtgtataattatgtaaatacaatgtatccttattcttaagacgtactgaagtaatttttgtacattacactaaattattagcatttgtttttagcattactttactttctgcttcatgatcctgttagctttacctgaatgcttgttttaaatgacagtggaaacttcattcctcttaaagtgccagtattctttgagtgttggttcttgaactagcaatgcctgtgaagaaaaataaaaacaaatgaaaaaaaaaaaaacacacaaaaacctgagaactgtcttaggactctttggtgcatgcacagttgctaacttcctatttttcttactgattgtgaacttctgttccgtgcgtaaacaaaacaatgaaacgatctacacgttctaacatcccccttcatttgtactctcttattttttacatctggttgggaaaacggaccagttagtgacaaagactttattttcagacttccttctaatttcgactgactgcaatatagagagaccagaagcctttatagtcttcctgtagattttgct

SEQ ID NO: 30 - protein, 188 aa, Gallus gallus
MTEYKLVVVGAGGVGKSALTIQLIQNHFVDEYDPTIEDSYRKQVVIDGETCLLDILDTAGQEEYSAMRDQYMRTGEGFLCVFAINNTKSFEDIHHYREQIKRVKDSEDVPMVLVGNKCDLPSRTVDTKQAQDLARSYGIPFIETSAKTRQGVDDAFYTLVREIRKHKEKMSKDGKKKKKKTKTKCIIM

SEQ ID NO: 31 - DNA, 3724 bp, Homo sapiens
tctccctcggcgccgccgccgccgcccgcggggctgggacccgatgcggttagagccgcggagcctggaagagccccgagcgtttctgctttgggacaaccatacatctaattccttaaagtagttttatatgtaaaacttgcaaagaatcagaacaatgcctccacgaccatcatcaggtgaactgtggggcatccacttgatgcccccaagaatcctagtagaatgtttactaccaaatggaatgatagtgactttagaatgcctccgtgaggctacattaataaccataaagcatgaactatttaaagaagcaagaaaataccccctccatcaacttcttcaagatgaatcttcttacattttcgtaagtgttactcaagaagcagaaagggaagaattttttgatgaaacaagacgactttgtgaccttcggctttttcaaccctttttaaaagtaattgaaccagtaggcaaccgtgaagaaaagatcctcaatcgagaaattggttttgctatcggcatgccagtgtgtgaatttgatatggttaaagatccagaagtacaggacttccgaagaaatattctgaacgtttgtaaagaagctgtggatcttagggacctcaattcacctcatagtagagcaatgtatgtctatcctccaaatgtagaatcttcaccagaattgccaaagcacatatataataaattagataaagggcaaataatagtggtgatctgggtaatagtttctccaaataatgacaagcagaagtatactctgaaaatcaaccatgactgtgtaccagaacaagtaattgctgaagcaatcaggaaaaaaactcgaagtatgttgctatcctctgaacaactaaaactctgtgttttagaatatcagggcaagtatattttaaaagtgtgtggatgtgatgaatacttcctagaaaaatatcctctgagtcagtataagtatataagaagctgtataatgcttgggaggatgcccaatttgatgttgatggctaaagaaagcctttattctcaactgccaatggactgttttacaatgccatcttattccagacgcatttccacagctacaccatatatgaatggagaaacatctacaaaatccctttgggttataaatagtgcactcagaataaaaattctttgtgcaacctacgtgaatgtaaatattcgagacattgataagatctatgttcgaacaggtatctaccatggaggagaacccttatgtgacaatgtgaacactcaaagagtaccttgttccaatcccaggtggaatgaatggctgaattatgatatatacattcctgatcttcctcgtgctgctcgactttgcctttccatttgctctgttaaaggccgaaagggtgctaaagaggaacactgtccattggcatggggaaatataaacttgtttgattacacagacactctagtatctggaaaaatggctttgaatctttggccagtacctcatggattagaagatttgctgaaccctattggtgttactggatcaaatccaaataaagaaactccatgcttagagttggagtttgactggttcagcagtgtggtaaagttcccagatatgtcagtgattgaagagcatgccaattggtctgtatcccgagaagcaggatttagctattcccacgcaggactgagtaacagactagctagagacaatgaattaagggaaaatgacaaagaacagctcaaagcaatttctacacgagatcctctctctgaaatcactgagcaggagaaagattttctatggagtcacagacactattgtgtaactatccccgaaattctacccaaattgcttctgtctgttaaatggaattctagagatgaagtagcccagatgtattgcttggtaaaagattggcctccaatcaaacctgaacaggctatggaacttctggactgtaattacccagatcctatggttcgaggttttgctgttcggtgcttggaaaaatatttaacagatgacaaactttctcagtatttaattcagctagtacaggtcctaaaatatgaacaatatttggataacttgcttgtgagatttttactgaagaaagcattgactaatcaaaggattgggcactttttcttttggcatttaaaatctgagatgcacaataaaacagttagccagaggtttggcctgcttttggagtcctattgtcgtgcatgtgggatgtatttgaagcacctgaataggcaagtcgaggcaatggaaaagctcattaacttaactgacattctcaaacaggagaagaaggatgaaacacaaaaggtacagatgaagtttttagttgagcaaatgaggcgaccagatttcatggatgctctacagggctttctgtctcctctaaaccctgctcatcaactaggaaacctcaggcttgaagagtgtcgaattatgtcctctgcaaaaaggccactgtggttgaattgggagaacccagacatcatgtcagagttactgtttcagaacaatgagatcatctttaaaaatggggatgatttacggcaagatatgctaacacttcaaattattcgtattatggaaaatatctggcaaaatcaaggtcttgatcttcgaatgttaccttatggttgtctgtcaatcggtgactgtgtgggacttattgaggtggtgcgaaattctcacactattatgcaaattcagtgcaaaggcggcttgaaaggtgcactgcagttcaacagccacacactacatcagtggctcaaagacaagaacaaaggagaaatatatgatgcagccattgacctgtttacacgttcatgtgctggatactgtgtagctaccttcattttgggaattggagatcgtcacaatagtaacatcatggtgaaagacgatggacaactgtttcatatagattttggacactttttggatcacaagaagaaaaaatttggttataaacgagaacgtgtgccatttgttttgacacaggatttcttaatagtgattagtaaaggagcccaagaatgcacaaagacaagagaatttgagaggtttcaggagatgtgttacaaggcttatctagctattcgacagcatgccaatctcttcataaatcttttctcaatgatgcttggctctggaatgccagaactacaatcttttgatgacattgcatacattcgaaagaccctagccttagataaaactgagcaagaggctttggagtatttcatgaaacaaatgaatgatgcacatcatggtggctggacaacaaaaatggattggatcttccacacaattaaacagcatgcattgaactgaaaagataactgagaaaatgaaagctcactctggattccacactgcactgttaataactctcagcaggcaaagaccgattgcataggaattgcacaatccatgaacagcattagaatttacagcaagaacagaaataaaatactatataatttaaataatgtaaacgcaaacagggtttgatagcacttaaactagttcatttcaaaattaagctttagaataatgcgcaatttcatgttatgccttaagtccaaaaaggtaaactttgaagattgtttgtatctttttttaaaaaacaaaacaaaacaaaaatccccaaaatatatagaaatgatggagaaggaaaaaaaaaaaaaaaaa

SEQ ID NO: 32 - protein, 1068 aa, Homo sapiens
MPPRPSSGELWGIHLMPPRILVECLLPNGMIVTLECLREATLITIKHELFKEARKYPLHQLLQDESSYIFVSVTQEAEREEFFDETRRLCDLRLFQPFLKVIEPVGNREEKILNREIGFAIGMPVCEFDMVKDPEVQDFRRNILNVCKEAVDLRDLNSPHSRAMYVYPPNVESSPELPKHIYNKLDKGQIIVVIWVIVSPNNDKQKYTLKINHDCVPEQVIAEAIRKKTRSMLLSSEQLKLCVLEYQGKYILKVCGCDEYFLEKYPLSQYKYIRSCIMLGRMPNLMLMAKESLYSQLPMDCFTMPSYSRRISTATPYMNGETSTKSLWVINSALRIKILCATYVNVNIRDIDKIYVRTGIYHGGEPLCDNVNTQRVPCSNPRWNEWLNYDIYIPDLPRAARLCLSICSVKGRKGAKEEHCPLAWGNINLFDYTDTLVSGKMALNLWPVPHGLEDLLNPIGVTGSNPNKETPCLELEFDWFSSVVKFPDMSVIEEHANWSVSREAGFSYSHAGLSNRLARDNELRENDKEQLKAISTRDPLSEITEQEKDFLWSHRHYCVTIPEILPKLLLSVKWNSRDEVAQMYCLVKDWPPIKPEQAMELLDCNYPDPMVRGFAVRCLEKYLTDDKLSQYLIQLVQVLKYEQYLDNLLVRFLLKKALTNQRIGHFFFWHLKSEMHNKTVSQRFGLLLESYCRACGMYLKHLNRQVEAMEKLINLTDILKQEKKDETQKVQMKFLVEQMRRPDFMDALQGFLSPLNPAHQLGNLRLEECRIMSSAKRPLWLNWENPDIMSELLFQNNEIIFKNGDDLRQDMLTLQIIRIMENIWQNQGLDLRMLPYGCLSIGDCVGLIEVVRNSHTIMQIQCKGGLKGALQFNSHTLHQWLKDKNKGEIYDAAIDLFTRSCAGYCVATFILGIGDRHNSNIMVKDDGQLFHIDFGHFLDHKKKKFGYKRERVPFVLTQDFLIVISKGAQECTKTREFERFQEMCYKAYLAIRQHANLFINLFSMMLGSGMPELQSFDDIAYIRKTLALDKTEQEALEYFMKQMNDAHHGGWTTKMDWIFHTIKQHALN

SEQ ID NO: 33 - DNA, 6435 bp, Rattus norvegicus
atgcctccacgaccatcttcgggtgaactgtggggcatccacttgatgcccccacgaatcctagtggaatgtttactcccaaatggaatgatagtgactttagaatgcctccgtgaggccacactagtcaccatcaagcatgaactgttcaaagaggccaggaaataccctctccatcagcttctgcaagatgaatcatcttacattttcgtaagtgttacccaagaagcagaaagggaagaatttttcgatgaaacaagacggctttgtgaccttcggctttttcaaccctttttaaaagtaattgagccagtaggcaaccgtgaagaaaagatcctcaaccgagaaattggttttgttattggcatgccagtgtgtgaatttgatatggttaaagatccagaagtccaagacttccgaaggaacattctgaatgtttgcaaagaagccgtggacctgcgggatctcaactcgcctcatagcagagcaatgtatgtctaccctccaaatgtcgagtcttccccagaactgccaaagcacatctacaacaagttagataaaggacaaatcatagtggtgatttgggtgatagtctctccaaacaacgacaagcagaagtacactctgaagatcaaccatgactgcgtgccagagcaagtcattgctgaggccatcaggaagaagacccggagcatgttgctgtcctcggagcagctgaaactctgtgtcttagaataccagggcaagtacattctcaaagtgtgtggctgtgatgagtacttcctagagaagtaccctctgagtcagtacaagtacataagaagctgtataatgctggggaggatgcccaacttgatgctgatggccaaggagagcctgtactctcagctgccgatcgatagcttcacaatgccatcctactccaggcgcatttccacagcgacaccctatatgaacggggagactgctacgaaatccctctgggttataaatagcgcgctcagaataaaaattctgtgtgcaacctatgtaaatgtaaatattcgagacattgataagatctatgttcgaacaggtatctaccatggaggagaacccttatgtgacaatgtgaatactcaaagagtcccttgttccaatcctaggtggaatgaatggctgaattatgatatatacattcctgatcttcctcgtgctgcccgcctttgcctttcaatctgctctgttaaaggccgaaagggtgctaaggaggagcactgtccgttggcctggggaaacataaacttgtttgattatacagacaccctagtgtccgggaaaatggctttgaatctctggcctgtaccacatgggttggaagatctgctgaaccctattggtgttactgggtcaaatccaaataaagaaactccatgcttagagttggagtttgattggttcagcagtgtggtgaagtttccagatatgtctgtgatcgaagagcatgccaattggtctgtgtcccgagaagccggattcagttactctcatacaggactgagtaacagactagccagagacaatgagttaagagaaaatgacaaggaacagctccgagcactttgtacccgggacccactgtctgaaatcactgaacaagagaaagacttcctatggagccacagacactactgtgtaactattcctgaaatcctacccaaattgcttctgtctgtcaagtggaattccagagatgaagtggcccagatgtactgcttagtaaaagattggcctccaatcaaaccagagcaagccatggagctcctggactgtaactacccagaccccatggttcggagctttgctgtccggtgcttggaaaaatacttaacagatgacaaactttctcagtacctcatccagcttgtacaggtcttaaaatatgaacagtatttggataacctgcttgtgagatttttactcaagaaagcactgacaaatcaaaggattggccattttttcttttggcatttaaaatctgagatgcacaataagactgtcagtcagaggttcggcctgctgttggagtcctactgccgtgcctgtgggatgtatctgaagcacctgaacagacaggtagaggccatggagaagctcatcaatctaactgacatcctcaagcaggagaagaaggatgagacacagaaggtacagatgaagttcttggttgaacagatgagacagccagatttcatggatgctttgcagggttttctgtcccctctaaatcctgctcatcaactaggaaacctcaggcttgaagagtgtcgaattatgtcctctgcaaaaaggccactgtggttgaattgggagaacccagacatcatgtcagagctactgtttcagaacaatgagatcatctttaaaaatggcgatgacttacggcaagacatgttaacccttcagatcatccgaatcatggagaacatctggcaaaaccaaggccttgaccttcgcatgctaccttatggctgtctatccattggggactgtgtgggtctcatcgaggtggtgagaaactctcacaccatcatgcagattcagtgcaaaggaggcctgaaaggggcactgcagttcaacagccacacgctgcatcagtggctcaaggacaagaacaagggcgagatatatgacgcagccattgacctgttcactcggtcctgcgctgggtactgcgtggcaacctttatcttgggaattggagaccggcacaacagcaacatcatggtgaaagatgacggacagctgtttcatatagattttgggcactttttggatcacaagaagaaaaaatttggctataaacgggaacgtgtgccgtttgttttgacgcaggatttcttaatagtgattagtaaaggagcacaagagtacacaaagaccagagagtttgagaggtttcaggagatgtgttacaaggcgtacctagcaattcggcagcatgccaatctcttcatcaaccttttctccatgatgcttggctccggaatgccagaactgcagtctttcgatgatattgcatatattcgaaagactctagccttagacaaaactgagcaagaggctctggagtatttcacaaagcaaatgaatgacgcacatcatggtggctggacaacaaaaatggactggatcttccacaccatcaagcagcatgcattgaactgagatggcagctggggactgcgagctggtgcctagcttctccactgcatggcagtgagtggcagcaggcacacggtggcatgggatggcacagtcaggaacaacatcaggactcgagcaagaacataaacaacgtgctctataattgaaacactgtacacgcaaacagggtttgatagcactaaactagttcatttcaaaattcagctttagaataatgagcaatttcatgttatgccttaagtccaaaaaaaggtaaactttgaagattgtttgtatcttttttaaaaaaacaaaacaaaacaaaaatccccaaaatacatacaaatgatggagacgaaaagagaatgctgttgtttgtctgccagtgttctgtccaagatgtggacacccaagctgactgctgtaggcccgagtaagctgaagcttatattaagttacatgaaattgaagaagaatgaaaattctgattttcccaatgctgttcagacttatgattggaagtgggtattttgactccctgcttaatgaggaacaacttttggggtgaagggatttgctttttgctttgaacaaacaacccttcgatggacttggggtctcacctacggttttgaaagcagtcacgaatgatacctgcagacagctgtgtttttgttgggttttgtttttttgttgtttttctctctggacagtatttacaaggatctgacttatttcctagggaaattctgggctcgcgtcaagtacagcagtaaccacagaggagaggcagcagggagctcctgttcctgacttgtacagtattcactttaagctgattgtttctccttttgcaattgaactgaatacttttttttcatgcatgttttccagaaaatagaagtgagtattaatgttattaaaaagattatttttttttattaaaggctatttatattatagaaactatcattaatatatattctttatttacataatctgtcccatagtcatgcattgttttgcaccccaaattttttattgttggtaacagcatggttaggttttctcggtctatagatgaggctcaggcactattccatttacccagatacccctgtatgactccttaaggaacagattgacctgcacatgctctccttcctctgctgtccgttttttacacgctgccctcattgcacacccatctgtagttgagatggcacaatcctatgagatcagttactgaaatgaatgcaaagcagactatcatcctgactcctaagtccctctgctgaggtcagtcatgaatgactttttacattatatatgagagactggaaaccatgaattttttaccttcataagctgtgtatccatatccaatgataaaagtaggacattaacccatttttactatcatgtcccatttccaagtggtgaggtctcactccgacttcatgatcccgttcagtcacggagtgcgttggtgagcattctgaggagcgtccatcctagatgtagggctgctgttagtggtcactctagacttctactccgtgtttgaatgattcatgtcctagaaaatagctttagcagatactcagatgccacaccaaaaagaaaaaaaaaaaaagaaaaaaaaagaaaaagaaaaaaaagtgcaataatttactgacagttcctagcttaggcgttattggagagcatcttcatgaagagcgcacgctgtacactctagaaaacacaatccttttaataaagcgctcaccgtgaggtcagacacatatatagaagttttgaatagtaaacaggggactctaataaaaatactcttaatatctgcctattttagaacccttaaagggcataattattgaagatttaggtacttcactaaagcatgtatatattattgccaacaagaaaaacctgaagattaggggaacttagttctgtaaactgtcttggaatagttaagcagaatttaaactctgttttatgcagaaaaccagatagattcttttgcagatatagaaaacttcctaacttatttaaacttggcatttaacactttgtgttacttagatatgcagttgctaggtactaacatcccattcttctctatatcagggattattacagtcaaactcagtgacatggtacaaatctacaactttgatggtggaaactgaggaattacagagaactgttttcccgagtgccaaaaaaaaaaaaaaaaaaaaaaaaaaaaagccgcgagcctccttgcacaaaattgataggtgtgtgtgtgtgtgtgtgtgtgtgtgtgtgtgtgtgtgtgtgtttaacattagttcattagttgccgcagtatcacctcccagggtctctgcacaattaaaacacagccacatagcttattttgtcacttactaccacactgattttatttgaaagaaagtctatattctataaagggtattagtaaagaaaggagaactggtgtattcaaaaaggcaaaagccaaacttgaatgaagctggggtgatcaatatctgtttccagagagcaataatgtgccactcactcccaggtgcttcagtaccagaaagtcctgcagacctggtctgtaggtgaccgaccttgtcattaaatattgtataaatgacttgggctccatagttacactaagtcatgtggggatgcttcatcagtgatttttttctggaaggaaagaaaacaaatctaaagaaagaaactaaatacactgtagcaagaagtaactcttaaatcatgctttaactttttaccatattctcagctataaaacaaaacaactttagtgtgaagattttagactgctgttcatttgaaatctgttgtttttactggggagtttgatttgtttgtttgtttgctttttgtttgtttttaaagatgtttctaattagattttctaaaaaaagaagaatggaatctggttgctattttaaggtagaacctgagacttttgtggttcttcatgtcctctgtaaaacgtggtgtcaagagtcatcaactctgaggttgtcccttctgttatgctttatattactgcccatcaggacatgggaacctggtgaatatatgatgacctgtaaaatattttaaatgtgtaactttttcaactgtgaaactgactattggttttttgatgaaaacagctgctcataaagtattttgtgtaaagtgtagttcttattaatcagaaaaaaaaaaaaaaaa

SEQ ID NO: 34 - protein, 1068 aa, Rattus norvegicus
MPPRPSSGELWGIHLMPPRILVECLLPNGMIVTLECLREATLVTIKHELFKEARKYPLHQLLQDESSYIFVSVTQEAEREEFFDETRRLCDLRLFQPFLKVIEPVGNREEKILNREIGFVIGMPVCEFDMVKDPEVQDFRRNILNVCKEAVDLRDLNSPHSRAMYVYPPNVESSPELPKHIYNKLDKGQIIVVIWVIVSPNNDKQKYTLKINHDCVPEQVIAEAIRKKTRSMLLSSEQLKLCVLEYQGKYILKVCGCDEYFLEKYPLSQYKYIRSCIMLGRMPNLMLMAKESLYSQLPIDSFTMPSYSRRISTATPYMNGETATKSLWVINSALRIKILCATYVNVNIRDIDKIYVRTGIYHGGEPLCDNVNTQRVPCSNPRWNEWLNYDIYIPDLPRAARLCLSICSVKGRKGAKEEHCPLAWGNINLFDYTDTLVSGKMALNLWPVPHGLEDLLNPIGVTGSNPNKETPCLELEFDWFSSVVKFPDMSVIEEHANWSVSREAGFSYSHTGLSNRLARDNELRENDKEQLRALCTRDPLSEITEQEKDFLWSHRHYCVTIPEILPKLLLSVKWNSRDEVAQMYCLVKDWPPIKPEQAMELLDCNYPDPMVRSFAVRCLEKYLTDDKLSQYLIQLVQVLKYEQYLDNLLVRFLLKKALTNQRIGHFFFWHLKSEMHNKTVSQRFGLLLESYCRACGMYLKHLNRQVEAMEKLINLTDILKQEKKDETQKVQMKFLVEQMRQPDFMDALQGFLSPLNPAHQLGNLRLEECRIMSSAKRPLWLNWENPDIMSELLFQNNEIIFKNGDDLRQDMLTLQIIRIMENIWQNQGLDLRMLPYGCLSIGDCVGLIEVVRNSHTIMQIQCKGGLKGALQFNSHTLHQWLKDKNKGEIYDAAIDLFTRSCAGYCVATFILGIGDRHNSNIMVKDDGQLFHIDFGHFLDHKKKKFGYKRERVPFVLTQDFLIVISKGAQEYTKTREFERFQEMCYKAYLAIRQHANLFINLFSMMLGSGMPELQSFDDIAYIRKTLALDKTEQEALEYFTKQMNDAHHGGWTTKMDWIFHTIKQHALN

SEQ ID NO: 35 - DNA, 8917 bp, Mus musculus
tgattctgactccataaggcggttttctatgtaaagtttgcagagggtcagagcaatgcctccacgaccatcttcgggtgaactgtggggcatccacttgatgcccccacgaatcctagtggaatgtttactccccaatggaatgatagtgactttagaatgcctccgtgaggccacactcgtcaccatcaaacatgaactgttcagagaggccaggaaataccctctccatcagcttctgcaagacgaaacttcttacattttcgtaagtgtcacccaagaagcagaaagggaagaattttttgatgaaacaagacgactttgtgaccttcggctttttcaaccctttttaaaagttattgaaccagtaggcaaccgtgaagaaaagatcctcaatcgagaaattggttttgttattggcatgccagtgtgtgaatttgatatggttaaagatccagaagtccaagactttcgaaggaacattctgaatgtttgcaaagaagctgtggacctgcgggatctcaactcgcctcatagcagagcaatgtatgtctaccctccaaatgtcgagtcttccccagaactgccaaagcacatctacaacaagttagataaaggacaaatcatagtggtgatttgggtaatagtctctccaaacaacgacaagcagaagtacactctgaagatcaatcatgactgtgtgccagagcaagtcattgctgaagccatcaggaaaaagactcggagcatgttgttgtcctctgagcagctgaaactctgtgtcttagaatatcagggcaagtatattctgaaagtgtgtggctgtgacgaatacttcctggaaaagtaccctctgagtcagtacaagtacataagaagctgtataatgctggggaggatgcccaacttgatgctgatggccaaagaaagcctatactctcagctgccgattgatagcttcaccatgccgtcatactccaggcgcatctccacagccacaccctacatgaatggagagacatctacgaaatccctctgggtcataaatagtgcgctcagaataaaaattctttgtgcaacctatgtaaatgtaaatattcgagacattgataagatctatgttcgaacaggtatctaccatggaggagaacccttatgtgacaatgtgaacactcaaagagtaccttgttccaatcctaggtggaatgaatggctgaattatgatatatacattcctgatcttcctcgtgctgcgcgcctttgcctttcaatctgctctgttaaaggccgaaagggtgctaaggaggagcactgtccgttggcctggggaaacataaacttgtttgattatacagacaccctagtgtccgggaaaatggctttgaatctctggcctgtaccgcatgggttagaagatctgctgaaccctattggtgttactgggtcaaatccaaataaagaaactccatgcttagagttggagtttgattggttcagcagtgtggtgaagtttccagacatgtctgtgatcgaagaacatgccaattggtccgtgtcccgagaagctggattcagttactcccatacaggactgagtaacagactagccagagacaatgagttaagagaaaatgacaaggaacagctccgagcactttgcacccgggacccactatctgaaatcactgaacaagagaaagacttcctatggagccacagacactactgcgtaactattcctgaaatcctacccaaattgcttctgtctgtcaagtggaattccagagacgaagtggcccagatgtactgcttagtaaaagattggcctccaatcaaaccagagcaagccatggaactcctggactgtaactatccagatcctatggttcggagttttgctgttcggtgcttagaaaaatatttaacagatgacaaactttctcagtacctcattcaacttgtacaggtcttaaaatatgaacagtatttggataacctgcttgtgagatttttactcaagaaagcattgacaaatcaaaggattggccattttttcttttggcatttaaaatctgagatgcacaataagactgtcagtcagaggtttggcctgctattggagtcctactgccgtgcctgtgggatgtatctgaagcacctgaacagacaagtagaggccatggagaagctcatcaacctaacggacatccttaagcaggagaagaaggatgagacacaaaaggtacagatgaagtttttggttgaacagatgagacagccagacttcatggatgctttgcagggttttctgtcccctctgaatcctgctcaccaactaggaaacctcaggcttgaagagtgtcgaattatgtcctctgcaaaaaggccactgtggttgaattgggagaacccagacatcatgtcagagctactgtttcagaacaatgagatcatctttaaaaatggcgacgacttacggcaagatatgttaacccttcagatcatccgaatcatggagaacatctggcaaaaccaaggccttgaccttcgcatgctaccttatggctgtctatccattggggactgtgtgggtctcatcgaggtggtgagaaactctcacaccatcatgcaaatccagtgcaaaggaggcctgaagggggcgctgcagttcaacagccacacactgcatcaatggctcaaggacaagaacaagggcgagatatatgatgcagccattgacctgttcactcggtcctgcgctgggtactgcgtggcaacctttatcttgggaattggagaccggcacaacagcaacatcatggtgaaagatgacggacagctgtttcatatagattttgggcactttttggatcacaagaagaaaaaatttggctataagcgggaacgtgtgccatttgtgttgacacaggatttcttgattgtgattagtaagggagcacaagagtacaccaagaccagagagtttgagaggtttcaggagatgtgttacaaggcttacctagcaattcggcagcatgccaatctcttcatcaaccttttttcaatgatgcttggctctggaatgccagaactacaatcttttgatgacattgcatatatccgaaagactctagccttggacaaaactgagcaagaagctttggaatatttcacaaagcaaatgaatgatgcacatcatggtggatggacgacaaaaatggattggatcttccacaccatcaagcagcatgctttgaactgagatgggagctgggactgcgagctggctcccggcttctccactgcatggcagtgagtggcagcaggcaggcagtggcatgggatggcacagtcaggaacaacattaggacttgagcaagaacataaacaacgtgctctataattgaaacactgtacacgcaagcagggtttgatagcactaaactagtttatttcaaaatccagctttagaataacgagcaatttcatgttatgccttaagtccaaaaaaggtaaactttgaagattgtttgtatctttttttaaaaaaacaaaacaaaacaaaaatccccaaaatacatacaaatgatggagacaaaactagaatgctgttgtttgtctgccagtgttctgtctaacacgtggacacgcccaaggctgtgactgctataggtctgagtaagctaaagcttatattaagttacatgaattggagaagaaggaaaattctgattttcccattgctgttcagacttaacgatttgaagtggggattttgatccctgcttaatgaggaacaacacttggggtgaagggactcgctttttgctttgaacaaacaacactttgatggacttggggtctcacctgcggttttgaaagcagtcacaatacttgcagacagctgcgtttttgttgggtgttgttttttgttgtttttttctctggacagtatttacaaggatctgacttatttcctagggaaattctgggctggcatcaagtatagcagtaagggcagaggagaggccgcagggagcccctgttcctgacctgtacagtgttcactttcagctgattgtttctccttttgcaattgaactgaatacttttttttcatgcatgttttccagaaaatagaagtgagtattaatgttattaaaaagattatttttttttattaaaggctatttatattatagaaactatcattaatatatattctttatttacataatctgtcccatagtcatgcattgttttgcaccccaaattttttatcgttggtaacagcatggttagcttttctctcggtctgtagatgaggctcaggcactattccatttatccaatacccgtgtatgactccttaaggaacagattgaatcgcacacgctttcctgccgctgctggccgttttttacacgacgccctcatccattcctccgtagttgagacagcacaatcacatgaaacccgttactaaaatgaatacaaaaccgactatcatcctgactcttaatccttctgcagaggtctagtcatgagtgactctttacattatgagagactggaaaccatgaattttttaccttcgtaagctacgtatccgtacttcaatgataaaagtaggacattaacccattttactatcatgtcccaattccaagtggtgaggtctcactccagtgtcattaaatcccattcaggcacggtgcattagtgagcattctgaaatgcatccatctaagatgtagggctaatgttagtggtcgctctagatttctactcagtgtttgaatgattcatgtcctagaaaatagctttagcagatactcagatgccacaccaaaaaaagaagaaaaaaagaaaaaaaaaagaataaataaaaaggaaaaaaaaaagaaaaactgtgcaataatctcctgacagttcctagctcaggcgttcctggggagcatcgttatgaagagcgcacgctgtacacgctagaaaacagaatccctgtaatacagtgctcaccttgaggccagacacctatatagacgttttgaatagtgaacaggggactctaatagaaatactcttaatatctgcctatttttagaacccttaaagggcataattattgaagatttaggtacttcactaaagcatgtatatattattgccaacaagaaaaataaacctgaagattaggggaacttggttctgtaaactgtcttggaatagttaagcagaatttaagctctgttttatgcagaaaaccagatagattcttttgcagatatagaaaacttcctaacttatttaaacttggcatttaacactttgtgttacttagatatacagttgctaggtactaacatcccattcttctctatatcagggattattacagtcaaactcagtgacatggtacaaatctacaactttgatggtgggaactgaagaattacagagaactgtgttttcccgagtgccaaaagaaacaaaaacaaaacaaaacaaacaaaccccacaaaaaaaagaaaaaaaaaaaaaagccgcgagcctccttgcacaaaattgataggtttttttttgtgtgtatgtgtgtgtttgtgtgtgtgtatgtttaacattagtccatcagttgccgtagtatcacctcccaggtctctgcacaattaaaacacagccacatagcttattttgtcatttacaaccacattgattttatttgaaagaaagtctatagtctgtgaagggtataagtaaagaaaggagaactggttgtattcaaaaaggcaaaagccaaacttgaattgcagctggggtgatcaatatctgcttccagagagcaataatgtgccacttactcccaggtgcttcagtaccagaaagtgctgtgggactcggtcacctctgtagatgaccgtccttgtcagtgaatgactattgtggaaatgacttgggctccatagtttcactaagtcacttgaggatgtctcatcagcaattatttcaggaaggaaagaaagcaaatctaaagaaagaaactaaatacactgtagcaagaaataactcttcaatcatgctttaactttttaccatagtctcagctatacaaaaaactttagtttgaagattttacattgctgttaatttgaaatctgttgttcttactgtggagtttgatttgttcgtttgtttgctttctgttggtttttttttttttttttaagatgtttctaaatagattttttaaaaaaaagaaagaagaagaagaatggaatctggttgctattttaaggtagaacctgagactttttgtggttcttcatgtcctctgtaaaatttggtgtcaagagtcatcaactctgaggttgtcccttctgttctgctttatattactgcccatcaggaaatgggaacctggtgaatatataatgaattgtaaaatattttaaatgtgtaactttttcaactgtgaaactgactattggttttttttttttttgatgaaaacagctgctcataaagtattttgtgtaaagtgtagttcttattaatcaggaaatgattacgtgattagatgtgtgccctcttgacttttatctgaaagagattggtaattatcacagagacagagcacgatccatctgtgttctctgctcgtcaggagccagctgatgtggcgtcacagaaaagacgaacctgttttaatggtacagtagaaacctcacagcacgtggacttcgctgtgtttcttaacataatttttgtaagcttgatgtccatgctttccagctctttgaagaaatttatttccagcattatgttaatcttttctgaatattacagtttccacttttttcctgtttctctggaaactgcagacctgggctggacccccacactacagaatattaatgaattacttttgatgtctacaacattgctaaaataccaaattcaaaggcattttgtggcgtcatagattgtggtatgtctgcttcagatgtttggggagatgggggtgtggtggaagggcctgagcagggagaagcacaaaggggcatggaagttacagggatgctgtccacgtactagaaaggaatcagttccaggttggaattttgaaggctgaactcagtcttgacatcatctttaattagtaactcttgatgacagaggagtccagctgagctgttttaaacagacaaacaaaagcatttcagttattaaaactgtaaacagatcatgtcgtggcctggaaagcctttttttttttccttataaaaatattgtttttactctctggaaagatgttgggctccagctcaaaagaattgcattcctgatagccctggtagctgtctccaaaggtttgtaagggaaatggccatgttaccactcagtgctctcacaggacagcaaagagaatctcattgtaggttttcaagtcaagattgggcatgcgctgctgttcatggaccaggagacaggatgggtcaaggaatggggctaaaatctattgctccagccacttgggaaagctttattgttaaagcaattcaaggtgccagttcttgagtgcggcgctcatagcatgctctcctgtgttgctttgctagcactggccaaggctctgtaacgaaaggtgtaaacagataccaaggttctaaaatgcagaaaggacttgttgttaggagtcacccagattgcattggcaatcctgggtgagtttttgtgggattgtgcacctccatccattttattatgcggtgccttttcctttgcttggcttttgggtatggtagggtatcagccgtgtgctaattacagcaaagggaatgggaacagagcagttatcacacttctcaggtgtcacaaagagtgttggtgggcaggactgaaatgaggctccatcctgtgtgctgttggctgatttttaactcactaccagcagtagatgccatttctcgtggtaataagtaccaaaaggaaaatactttataggccacgtggactttatataacctcatcttgtgtcacaagcttgtggcagaaatatacatacacatatacatactatatgtatgtatgtgtatatatatatatatttttttttttttttgagacatggtttctctgtatagccctgtctgtcctggaactcactctgtagaccaggctggcctcaaactcagaaatctgcctgcctctgcctcccaagtaccgggattaaaggcgtgtgccaacacctgcccggccggaagtatatatttttaaatactgtttttgttgatcttctaggttagctgaaggaagaacctttggtgtttccaattaaagcatgggaatttgggtcagttgttagcccaacaaatgtgtgtggagtggagctctgggcttgagcccagcacatcataaacggggtctgatgacatatgcctgtaattccccacctcaggaggtagagaacagaagttcagggccatcctcagcctacattactaacataatgtaatgcatgcttggggtactctggctccaaaacatccccactaaacttgttctagtacaaattcacaagtgtaattatttctgttggttcataagaaagaaatacttaaatagatttaatgtatgttcctaagagtagctaagaaatgtgatttttctggaaatgtttttgattatgaaacccaaacaaatttgttgtggtgatgatggtggatttcttagggttttgtcattttattgttggtacaaggtctcagtgtagcccaggctggcctcaaattcaagatcctctggacttagcttcggggtgctgagtttacagtaccctcactccaggctccaagaatccgtgcttcaaatgcagctgatggttctattgtcatttggtcttagctgaataaaatct

SEQ ID NO: 36 - protein, 1068 aa, Mus musculus
MPPRPSSGELWGIHLMPPRILVECLLPNGMIVTLECLREATLVTIKHELFREARKYPLHQLLQDETSYIFVSVTQEAEREEFFDETRRLCDLRLFQPFLKVIEPVGNREEKILNREIGFVIGMPVCEFDMVKDPEVQDFRRNILNVCKEAVDLRDLNSPHSRAMYVYPPNVESSPELPKHIYNKLDKGQIIVVIWVIVSPNNDKQKYTLKINHDCVPEQVIAEAIRKKTRSMLLSSEQLKLCVLEYQGKYILKVCGCDEYFLEKYPLSQYKYIRSCIMLGRMPNLMLMAKESLYSQLPIDSFTMPSYSRRISTATPYMNGETSTKSLWVINSALRIKILCATYVNVNIRDIDKIYVRTGIYHGGEPLCDNVNTQRVPCSNPRWNEWLNYDIYIPDLPRAARLCLSICSVKGRKGAKEEHCPLAWGNINLFDYTDTLVSGKMALNLWPVPHGLEDLLNPIGVTGSNPNKETPCLELEFDWFSSVVKFPDMSVIEEHANWSVSREAGFSYSHTGLSNRLARDNELRENDKEQLRALCTRDPLSEITEQEKDFLWSHRHYCVTIPEILPKLLLSVKWNSRDEVAQMYCLVKDWPPIKPEQAMELLDCNYPDPMVRSFAVRCLEKYLTDDKLSQYLIQLVQVLKYEQYLDNLLVRFLLKKALTNQRIGHFFFWHLKSEMHNKTVSQRFGLLLESYCRACGMYLKHLNRQVEAMEKLINLTDILKQEKKDETQKVQMKFLVEQMRQPDFMDALQGFLSPLNPAHQLGNLRLEECRIMSSAKRPLWLNWENPDIMSELLFQNNEIIFKNGDDLRQDMLTLQIIRIMENIWQNQGLDLRMLPYGCLSIGDCVGLIEVVRNSHTIMQIQCKGGLKGALQFNSHTLHQWLKDKNKGEIYDAAIDLFTRSCAGYCVATFILGIGDRHNSNIMVKDDGQLFHIDFGHFLDHKKKKFGYKRERVPFVLTQDFLIVISKGAQEYTKTREFERFQEMCYKAYLAIRQHANLFINLFSMMLGSGMPELQSFDDIAYIRKTLALDKTEQEALEYFTKQMNDAHHGGWTTKMDWIFHTIKQHALN

SEQ ID NO: 37 - DNA, 4335 bp, Oryctolagus cuniculus
ccgtcgccgccgccgccgccgcccgcgcggtttgggacccgatgcggttggagccgcggatcctggaggagccccgagcgtgtctgctttggaacaacaatatatataattccttcaagtagttttaaatgtaaaacttgtaaaggatcagaacaatgcctccacgaccatcatcaggtgaactgtggggcatccacttgatgcccccaagaatcttagtagaatgtttactgccaaatggaatgatagtgactttagaatgcctccgtgaggctacattaattactataaagcatgaactatttaaagaagcaagaaaataccctctccatcaacttcttcaagatgaatcttcttacattttcgtaagtgttacccaagaagcagaaagggaagaattttttgatgaaacaaggcgcctttgtgaccttcggctttttcaaccctttttaaaagtaattgaaccagtaggcaaccgtgaagaaaagatcctgaatcgagaaattggttttgttattggcatgccagtgtgtgaatttgatatggttaaagatccagaagtacaggacttccgaagaaatattctgaatgtttgtaaagaagctgtggatcttagagatctgaattcacctcatagtagagcaatgtatgtctatcctccaaatgtagaatcttcaccagaactgccaaagcacatatataataaattagataaagggcaaataatagtggtgatttgggtaatagtttctccaaataatgataagcagaagtataccctgaaaatcaaccatgactgtgtgccagaacaagtaattgctgaagcaatcaggaagaaaacccggagcatgttgctatcctctgaacaactaaaactatgtgttttagaatatcagggcaagtatattttaaaagtgtgtggatgtgatgaatacttcttagaaaaatatcctctgagtcagtataagtatataagaagctgtataatgcttgggaggatgcccaatttgatgctgatggctaaagaaagcctttattctcaactgccaatggactgttttacaatgccatcttattccagacgcatctccactgctacaccatatatgaatggagaaacatctacaaaatccctttgggttataaatagtgcactcagaataaaaattctttgtgctacctatgtgaatgtaaatattcgagacattgacaagatctatgttcgaacaggtatctaccatggaggagaacctttatgtgacaatgtgaacactcaaagagtaccttgttccaatcccaggtggaatgaatggctgaattatgatatatacattcctgatcttcctcgtgctgctcgactttgcctttctatatgctctgttaaaggccgaaagggtgctaaggaggaacactgtccactggcttggggaaatataaacttgtttgattacactgacactctggtatctggaaaaatggctctgaatctttggccagtacctcatggattagaagatttactgaaccctattggtgttactgggtcaaatccaaataaagaaactccatgcttagagttggagtttgactggtttagcagtgtggtaaagtttccagatatgtcagtgattgaggaacatgccaattggtctgtatccagagaagcaggatttagttattcccatgcaggactgagtaacagactagcaagagacaatgaattaagagaaaatgataaagaacagctccgagcaatctgtacacgcgatcctctatctgaaatcactgagcaagagaaagattttctgtggagccacagacattattgtgtaactatcccagagattctacccaaattgcttctgtctgttaaatggaattctagagatgaagttgcccagatgtactgcttggtaaaagattggcctccaataaaacctgagcaggccatggagctcctggactgcaactacccagatccgatggttcgagcttttgctgttcgatgcttggaaaaatatttaacagatgacaaactttctcagtatctgattcagctagtacaggtcctaaaatatgaacagtatttggataaccttctcgtgagatttttactcaagaaagcattgactaaccaaaggattgggcactttttcttttggcatttaaaatctgagatgcacaataaaacagttagtcagaggtttggcctgcttttggagtcctactgccgggcatgtggaatgtatttgaagcacctgaataggcaagttgaggctatggaaaagctcattaacttgactgacattctcaaacaggagaagaaggatgaaacacaaaaggtacaaatgaagtttttagttgagcaaatgaggcaaccagatttcatggatgctctacagggctttctgtctcctttaaaccctgctcatcaactgggaaatctcaggcttgaagagtgtcgaataatgtcctctgcaaaaaggccactgtggttgaattgggagaacccagacatcatgtcagagttactgtttcagaacaatgagatcatctttaaaaatggggatgatttacggcaagatatgctaacacttcaaattattcgcattatggaaaatatctggcaaaatcaaggtcttgatcttcgaatgttaccttatggttgtctgtcaattggtgactgtgtgggacttattgaggtggtgagaaattctcacactatcatgcagattcagtgcaaaggtggcctgaaaggtgcactgcagttcaatagccatacactgcatcagtggctcaaagacaagaacaaaggagaaatatatgatgcagccattgacctgttcacccgttcatgtgctggctattgcgttgcaactttcatcttgggaattggagatcggcacaacagtaacatcatggtgaaagatgatggacaactgtttcatatagatttcggacactttttggaccacaagaagaaaaaatttggttataagcgagaacgtgtaccatttgttctgacacaggatttcttaatagtgattagtaaaggagcccaagaatgcacaaaaactagagaatttgagaggtttcaagagatgtgttacaaggcttatctagctattcggcagcatgccaatctcttcataaatcttttctcaatgatgcttggctctggaatgccagaactgcaatcttttgatgacattgcatatattcgaaagaccctagccttagataaaactgagcaggaggctttggaatatttcatgaaacaaatgaacgatgcacatcatggtggctggacaacaaaaatggattggatcttccacacaattaagcagcatgcattgaactgaaatgatatctaagaaactgagagctcaatatctggattctacaccgcactgttaataactgtcagcaggcaaagactgattgcataggaattgcacaatccatgaacagcattagaatttacagcaagaacagaaataaaatagtatataatttaaaataatgtaaacgcaaacagggtttgatagcactaaactagttcatttcaaaattaagctttagaataatgcgcaatttcatgttatgccttaagtccaaaaaggtaaactttgaagattgtttgtatctttttttaaaaacaaaacaaaacaaaaatcccctaaatatatataaatgatggagaaggaaaaagaatgatgttctatttgtcttgcaaatgctctgcgtttcgacatgtggatacaactataaggctgttattgcattaggactgagtcaactggagtttatgttgaattacatagaatggaaaaggatgacagtttcttatttttccattgctgttcaatttatagtttgaagtgggttttttgactccttgtttaatgaagaaaagtgcttggggtggaagggactctcgagatttctccagagactttttctttttaataaatcaaaccttttgatgatttgggggtcttatctgcacaattttggaagcagtcacaaatgagacctgtaataaggtggtgtttttggttttgggttttttgctttttgtttctttttgacagtattcttaatacctagggaaattctgggctcccacaaagtgaagtaatcatcatagaaacagaatgagcaggagtagttctcattccaggattgtacagtattcaccttaagttgattttttttctccttttgcaattgaactgaacacatttttcatgcatgttttccagaaaatagaagtattaatgttattaaaaagattattttttttattaaaggctatttatattatagaaacta

SEQ ID NO: 38 - DNA, 3505 bp, Cavia porcellus
  misc_feature (1224)..(1225): n is a, c, g, or t
acagccataaatctagttacttaaagtagttttatatgtaaaacttgtaaaggatcagaacaatgcctccacgaccatcatcaggtgaactgtggggcatccacttgatgcccccaagaatcctcgtagaatgtttactaccaaatggaatgatcgtgactttagaatgcctccgtgaggctacattaataaccataaagcatgaactgtttaaggaagcaagaaaataccctctccatcaacttcttcaagacgaatcttcttacattttcgtaagtgttactcaagaagcagaaagggaagaattttttgatgaaacaagacgactatgtgaccttcggcttttccaaccctttttaaaagtaattgaaccagttggcaaccgtgaggaaaagatcctcaatcgagaaatcggttttgttatcggcatgccagtgtgtgaatttgatatggttaaagatccagaagtacaggacttcagaagaaatattttgaatgtttgtaaagaagctgtggaccttagggacctcaattcacctcatagtagagcaatgtatgtctatcctccaaatgtagaatcatcaccagagctgccaaagcacatatacaataaattagacaaaggacaaataattgtggtgatttgggtaatagtttctccaaacaatgacaagcagaagtatactttgaaaatcaaccatgactgtgtgccagaacaagtaattgctgaagcaatcaggaaaaaaactcgaagtatgttgctatcctctgaacaactaaaactctgtgttttagaatatcagggcaagtatattttaaaagtatgtggatgtgatgaatacttcctagaaaaatatcctctgagtcagtataagtatataagaagctgtataatgcttgggaggatgcccaatttgatgctgatggctaaagaaagcctttactctcagctgccaatggactgttttacaatgccatcctattccagacgcatctctacagctacaccgtatatgaatggagaaacatctacaaaatccctttgggttataaatagtgcactcagaataaaaattctttgtgcaacttatgtaaatgtaaatattcgagacattgataagatctatgttcgaacgggtatctaccatggaggagaacccttatgtgacaatgtgaacactcagagagtaccttgttccaatcctaggtggaatgaatggctgnnatacgatatatacattcccgatctctcactttttagatatgagcattgtccattggcctggggaaatataaacttgtttgattacacagacacactagtatctggaaaaatggccttgaatctttggccagtacctcatggattagaagacttgctgaatcctattggtgttactgggtcaaatccaaataaagaaactccatgcttagaattagagtttgattggttcagcagtgtggtaaagtttccagatatgtcagtgattgaggagcatgcaaattggtctgtatcccgagaagcaggatttagttattcacatgcaggactgagtaacagactagctcgagacaatgaattaagagaaaatgacaaagaacagctccgagcaatttgtacacgagaccctctgtctgaaatcactgagcaagagaaagattttctgtggagtcacagacactattgtgtaactatccctgaaattctacccaaattgcttctgtccgttaaatggaactctagagatgaagtagctcagatgtactgcttagtgaaagactggcccccaattaaacctgagcaggcaatggaacttctggactgcaactacccagaccctatggttcgaggttttgctgttcgatgcttggaaaaatacttgacagatgacaaactttctcagtaccttatccagctagtacaggtcctaaaatatgaacaatatttggataatcttcttgtgagatttttactcaagaaagcattaacaaatcaaaggattggacactttttcttttggcatttaaaatctgagatgcacaataaaacagtgagtcaaagatttggtctgcttttggagtcctattgccgcgcctgtgggatgtacctaaagcacctgaacaggcaagttgaggccatggaaaagctcatcaacttaactgacatcctcaaacaggagaagaaggatgaaacacagaaggtacagatgaaattcttagttgagcaaatgaggcaaccagatttcatggatgcactacaaggctttttgtctcctctaaaccctgctcatcaactgggaaatctcaggcttgaagagtgtcgaattatgtcttctgcaaaaaggccactgtggttgaattgggagaacccagacatcatgtcagagttactgtttcagaacaatgagatcatctttaaaaatggggatgatttacggcaagatatgctaacgcttcagattattcgcataatggaaaatatctggcaaaatcaaggccttgatcttcgaatgctgccgtatggttgtctctccattggggactgtgtaggactgatcgaggtggtgagaaattctcacacgatcatgcagattcagtgcaaaggtggcctgaaaggtgcactgcagttcaatagccacacgctgcatcagtggctcaaagacaagaacaaaggagaaatatacgatgcagccattgacctatttacacggtcgtgtgccggatactgcgtagctaccttcattttgggaattggtgaccgtcacaacagtaacatcatggtgaaagatgatggacagctgtttcatatagactttggacactttttggatcacaagaagaaaaaatttggttataaacgagaacgtgtaccatttgttttgacacaagatttcttaatagtgataagcaaaggggcccaagaatgtacaaagaccagagaatttgaaaggtttcaggagatgtgttacaaggcgtatctagctattcggcagcatgctaatctcttcataaatcttttctcaatgatgcttggctctggaatgccagaactacagtcttttgatgacattgcatatattcgaaagaccctagccttagataaaactgagcaagaggctttggaatatttcatgaaacaaatgaatgatgcacatcatggtggctggacaacaaaaatggattggatcttccacacaattaagcagcatgcattgaactgaaatgataagtgagaaactgaaagcccaatgatctggattctacactgcactgttaataactgacagcaggcaaagactgattgcataggaattgcacaatccatgaaaagcattagaacttacagcaagaaacagaaataaaatactatctaatttaaataatgtaaatgcaaacagggtttgatagcactaaactagttcatttcaaagttaagctttagaataatgcgcaatttcatgttatgccttaagtccaaaaaaaggtaaactttgaagattgtttg

SEQ ID NO: 39 - protein, 1052 aa, Cavia porcellus
  misc_feature (388)..(388): Xaa can be any naturally occurring amino acid
MPPRPSSGELWGIHLMPPRILVECLLPNGMIVTLECLREATLITIKHELFKEARKYPLHQLLQDESSYIFVSVTQEAEREEFFDETRRLCDLRLFQPFLKVIEPVGNREEKILNREIGFVIGMPVCEFDMVKDPEVQDFRRNILNVCKEAVDLRDLNSPHSRAMYVYPPNVESSPELPKHIYNKLDKGQIIVVIWVIVSPNNDKQKYTLKINHDCVPEQVIAEAIRKKTRSMLLSSEQLKLCVLEYQGKYILKVCGCDEYFLEKYPLSQYKYIRSCIMLGRMPNLMLMAKESLYSQLPMDCFTMPSYSRRISTATPYMNGETSTKSLWVINSALRIKILCATYVNVNIRDIDKIYVRTGIYHGGEPLCDNVNTQRVPCSNPRWNEWLXYDIYIPDLSLFRYEHCPLAWGNINLFDYTDTLVSGKMALNLWPVPHGLEDLLNPIGVTGSNPNKETPCLELEFDWFSSVVKFPDMSVIEEHANWSVSREAGFSYSHAGLSNRLARDNELRENDKEQLRAICTRDPLSEITEQEKDFLWSHRHYCVTIPEILPKLLLSVKWNSRDEVAQMYCLVKDWPPIKPEQAMELLDCNYPDPMVRGFAVRCLEKYLTDDKLSQYLIQLVQVLKYEQYLDNLLVRFLLKKALTNQRIGHFFFWHLKSEMHNKTVSQRFGLLLESYCRACGMYLKHLNRQVEAMEKLINLTDILKQEKKDETQKVQMKFLVEQMRQPDFMDALQGFLSPLNPAHQLGNLRLEECRIMSSAKRPLWLNWENPDIMSELLFQNNEIIFKNGDDLRQDMLTLQIIRIMENIWQNQGLDLRMLPYGCLSIGDCVGLIEVVRNSHTIMQIQCKGGLKGALQFNSHTLHQWLKDKNKGEIYDAAIDLFTRSCAGYCVATFILGIGDRHNSNIMVKDDGQLFHIDFGHFLDHKKKKFGYKRERVPFVLTQDFLIVISKGAQECTKTREFERFQEMCYKAYLAIRQHANLFINLFSMMLGSGMPELQSFDDIAYIRKTLALDKTEQEALEYFMKQMNDAHHGGWTTKMDWIFHTIKQHALN

SEQ ID NO: 40 - DNA, 6632 bp, Canis lupus familiaris
gccgccgcaaggggggctgggacccgatgtggttagagccgcggagcctggagcagccccgagcatttctgctttgggacagccacacatataattccttaaaatagttttatatgtaaaacttgtaaaggatcagaacaatgcctccaagaccatcatcaggtgaactgtggggcatccacttgatgcccccaagaatcctagtagaatgtttactaccaaatggaatgatagtgacgttagaatgcctccgtgaggctacattaataactataaagcatgaattatttaaagaagcaagaaagtaccctctccatcaacttcttcaagatgaatcttcttacattttcgtaagtgttacccaagaagcagaaagggaagaattttttgatgaaacaagacggctttgtgaccttcggctttttcaaccctttttaaaagtaattgagccagtaggcaaccgagaagaaaagatcctcaatcgagaaattggttttgctattggcatgccagtgtgtgaatttgatatggttaaagatccagaagtacaggacttccgaagaaatattctgaatgtttgtaaagaagctgtggatcttcgggatcttaattcacctcatagtagagcaatgtatgtctatcctccaaatgtagaatcttcaccagaactgccaaagcacatatataataaattagataaagggcaaataatagtggtgatttgggtaatagtttctccaaataatgacaaacagaagtatactctgaaaatcaaccatgactgtgttccagaacaagtaattgctgaagcaatcagaaaaaaaactagaagtatgttgctatcatctgaacaactaaaactctgtgttttagaatatcagggcaagtatattttaaaagtatgtggatgtgatgaatacttccttgaaaaatatcctctaagtcagtataagtacataagaagctgtataatgcttggaaggatgcccaatttgatgttgatggctaaagaaagcctttactcccaattgccaatggactgtttcacaatgccatcttattccagacgcatctccacagctacaccatatatgaatggagaaacatctacaaaatccctttgggttataaatagcgcactcagaataaaaatcctttgtgcaacctatgtaaatgtaaatattcgagacattgacaagatttatgttcgaacaggtatctatcatggaggagaacccttatgtgataatgttaacactcaaagagtaccttgttctaatcccaggtggaatgaatggctaaattacgatatatacattcctgatcttcctcgtgctgctcgactttgcctttccatttgttctgttaaaggccgaaagggtgctaaagaggaacactgtccattggcctggggaaatataaacttgtttgattacacagatactctagtatctggaaaaatggctctgaatctttggccagtacctcatggattagaagatttgctgaaccctattggtgttactgggtcaaatccaaataaagaaactccatgcttagagttggagtttgactggttcagcagtgtggtaaagttcccagatatgtcagtgattgaagagcatgccaactggtcggtgtctcgggaagcaggatttagttattcccatgcaggactgagtaacagactggctagagacaacgaattaagagaaaatgataaagaacagctccgagcaatttgtacccgagatcctctctctgaaatcactgagcaagagaaagattttctgtggagccacagacactattgtgtaactatccctgaaattctacccaaactgcttctgtccgttaaatggaattctagagatgaagtagctcagatgtactgcttagtaaaagattggcctccaatcaaacctgaacaagctatggagcttctggactgtaattacccagatcctatggttcgaggttttgctgttcggtgcttggaaaaatacttaacagatgacaagctttctcagtacctaattcagctagtacaggtcctaaaatacgaacaatatttggataacctgcttgtgagatttttactcaagaaagcattgactaatcaaaggattgggcattttttcttttggcatttaaaatctgagatgcacaataaaacggttagtcagaggtttggcctgcttttggagtcctattgccgtgcttgtgggatgtatttgaagcacctaaataggcaagttgaggctatggaaaagctcattaacttaactgacattctcaaacaagagaagaaggatgaaacacaaaaggtacagatgaagtttttagttgagcaaatgcggcgaccagatttcatggatgctctacaaggttttctatctcctctaaatcctgctcatcaactaggaaatctcaggcttgaagagtgtcgaattatgtcctctgcaaaaaggccactgtggttgaattgggagaacccagacatcatgtcagagttactctttcagaacaatgagatcatctttaaaaatggggatgatttacgacaagatatgctaacacttcaaataattcgcattatggaaaatatctggcaaaatcaaggtcttgatcttcgaatgttaccttatggttgtctgtcaatcggtgactgtgtgggacttattgaggtggtgcgaaattctcacactattatgcagattcagtgcaaaggtggcctgaaaggtgcactgcagttcaacagccacacactacaccagtggctcaaagacaagaacaaaggagaaatatatgatgcagccattgacctgttcacacgttcatgtgctggatattgtgttgctaccttcattttgggaattggagatcgtcacaatagtaacatcatggttaaagatgatggacaactgtttcatatagattttggacactttttggaccataagaagaaaaaatttggttataaacgggaacgtgtgccatttgttttgacacaggatttcttaatagtgattagtaaaggagcccaggaatgcacaaaaacaagagaatttgagaggtttcaggagatgtgttacaaggcttacctagctattcggcagcatgccaatctcttcataaatcttttctcaatgatgcttggctctggaatgccagaactacaatcttttgatgatattgcatacattcgaaagaccctagctttagataaaactgaacaagaggctttggaatatttcatgaaacaaatgaatgatgcacatcatggtggctggacaacaaaaatggattggatcttccacaccattaagcagcatgctttgaactgaaatgataactgagaaaccgaaagctcattatctggattctatactgcactgttaataactgtcaacaggcaaagactgattgcataggaattgcacaatccatgaacagcattagaatttacacaagaacagaaataaaatactatataatttaaataatgtaaacgcaaacagggtttgagagcactaaactagttcatttcaaaattaagctttagaataatgcgcaatttcatgttatgccttaaagtccaaaaaggtaaactttgaagattgtttgtatctttttttaaaaaagaaaacaaaacaaaaaaaccccaaaatatatagaaattatggagaaggaaaaagaatgatgttctttttttgtcttgcaaatgttctatgttttgaaattgtggacacagcgaagtctattattgcattaggtccaaggaaactgaagtttggtgttaaattacattgagattagaaaaataatgaagatttcttatttttccattgctgttcaatttatagtttgaagtgggtttttttgactccttgtttaatgaagaaaaatgcttggggtggaagggactcttgagatttcaccagagacttcctttttaataaatcaaaccttttgatgatttgaggtcttatctgcaaagttttggaagcagtcacaaatgagacctgttataagatggtgtttttgggttttttttttctggacagtatttacaagaatctgattcttacttcccagggaaattctgggctcccacaaagtaaaataatcattatagagaaagaatgagcaggactagttcttgctccagaattgtacagtattcaccttaggttgatttttttttctccttttgcaattgaattgaatacatttttcatgcatgtttccagaaaatagaagtgagtattaatgttattaaaaagattattttttttattaaaggctatttatattatagaaactatcattaatatatattctttatttacatgatctgtcccatagtcatgcattgttttgcaccccaaattttttattgttcgtagcagcatggtcagctttcctcttggtttgtgggtgaggctcaggcactatcccatttataccaatgactagtgtataattgcataaggaaaacagattaaagttcatcctctttctttttatttctttgttttcatgtaactcccccattttccatctcttatagttgataatgcctcagtcatgaaaccagttaccaaaattaacacaatatagagtatcttcctgattgcttcaacccctctgctgaggtatgctcatgaataatactttataatatgggggaatagaaaccacaaactttttacctttttaggctatttatgcaatatctggataataaaagtaggattttaaaccattttaaggtcatgtcccatttccaagcaattagggctcactgtccaactttattaaattgcatttgagtacaggatacattcttaaacactttggaaaacattgacccaaggtgtaggggctaatgctaatcatctctctagactctgatattttactcagtatttgaaatgaatgattaatgccctaggaaatagctttagcaaatgtccaggtgccacaccagaaaaagtgcaataatttactgacagttttctagattaggcatattattggaatacaactttataaaaagtgcacattatatactctagtaaaacagcatcactaaaacaatattcatttatgaaatcagttacctataatagaagtcttgaatagtgaataagggactctaatacaaatactcttaatatttggctattttagagcccttaaagggcctaattattggagacttaggtacttcactaaagcatgtatataatattgccaacaagaaaaataaatttgaagattaggggaacttatttctgtaaactgtcttggaatagttaagaagaatttaaactcccattttaagcaggaagccaaatagattcttttgcagatatagatttcataacttcttaaagcttctttaacattttgtgccttttagatatattcagttaatacatactaacatcccagccttttctatatcagggattaattacaggaaaactcaatgaaatggtacaaatctggaactctgatggtggagactgaagacttaacagagaacagcgtttttacctgagtgccaaaaaagctttgagcttccttgcacaaaatttatatgatctttgcatgtctcacatcagtccagctagtccccttcccctgagacctctctaccattaaaacacaagccacatagcttatttcatcatttacatttattttcaatagttattacaaccaagtctattctgttggaagaagtgtagacaaattttacaaagaatgattaaacaatctcgctgaaaacaaagtaaattttaaacaaatccaagcagagtttaagcaaacaacattaaaaataagaaaaaagggtcaagtcgtgctcagaaggcaaagccaaaaattgaactgaatgctacatggggtgactaggatgtcaagtcaggggtaagctgtttccaggtacttcggtgtcagaccactttcatggattggtccgttcctgtggccaaccatccttgtcattgaacattgtataactgattattgactctacggtttcatgtagtcacttgagaaatagttccttcaaggtattttgtagggggaaaaaaccaagcaggtttaaggaaaataaaacctaattttaaacacattctagtaagatagactctgaaaatcatgttttaactttttaatcatattctcagctatacagaatcatttattttgaagatttttagactgctgttaatttgaaatctgttaatcatattgtagaatttggtttttaaaaaaaagatgtttctaattggattttttaaagaagaatggaatttggtcactattttatgatagaacctaagctttttgtggttctcagtgtcctctgtaaaattcagtgtcaaagtaatctactttgaggttttcccttttaatctgctttatattacaagccctttaggaaatgggaacgtggtgaatatacaatgaattgtaaaatattttaatgtgtaattttttcaactgtgaaactatgaatattggttttttgatgaaaacagctgctgataaagtattttgtgtaaagtgtagttcttattaatcaggaaaataatcaatgacttgattagaatgta

SEQ ID NO: 41 - protein, 1068 aa, Canis lupus familiaris
MPPRPSSGELWGIHLMPPRILVECLLPNGMIVTLECLREATLITIKHELFKEARKYPLHQLLQDESSYIFVSVTQEAEREEFFDETRRLCDLRLFQPFLKVIEPVGNREEKILNREIGFAIGMPVCEFDMVKDPEVQDFRRNILNVCKEAVDLRDLNSPHSRAMYVYPPNVESSPELPKHIYNKLDKGQIIVVIWVIVSPNNDKQKYTLKINHDCVPEQVIAEAIRKKTRSMLLSSEQLKLCVLEYQGKYILKVCGCDEYFLEKYPLSQYKYIRSCIMLGRMPNLMLMAKESLYSQLPMDCFTMPSYSRRISTATPYMNGETSTKSLWVINSALRIKILCATYVNVNIRDIDKIYVRTGIYHGGEPLCDNVNTQRVPCSNPRWNEWLNYDIYIPDLPRAARLCLSICSVKGRKGAKEEHCPLAWGNINLFDYTDTLVSGKMALNLWPVPHGLEDLLNPIGVTGSNPNKETPCLELEFDWFSSVVKFPDMSVIEEHANWSVSREAGFSYSHAGLSNRLARDNELRENDKEQLRAICTRDPLSEITEQEKDFLWSHRHYCVTIPEILPKLLLSVKWNSRDEVAQMYCLVKDWPPIKPEQAMELLDCNYPDPMVRGFAVRCLEKYLTDDKLSQYLIQLVQVLKYEQYLDNLLVRFLLKKALTNQRIGHFFFWHLKSEMHNKTVSQRFGLLLESYCRACGMYLKHLNRQVEAMEKLINLTDILKQEKKDETQKVQMKFLVEQMRRPDFMDALQGFLSPLNPAHQLGNLRLEECRIMSSAKRPLWLNWENPDIMSELLFQNNEIIFKNGDDLRQDMLTLQIIRIMENIWQNQGLDLRMLPYGCLSIGDCVGLIEVVRNSHTIMQIQCKGGLKGALQFNSHTLHQWLKDKNKGEIYDAAIDLFTRSCAGYCVATFILGIGDRHNSNIMVKDDGQLFHIDFGHFLDHKKKKFGYKRERVPFVLTQDFLIVISKGAQECTKTREFERFQEMCYKAYLAIRQHANLFINLFSMMLGSGMPELQSFDDIAYIRKTLALDKTEQEALEYFMKQMNDAHHGGWTTKMDWIFHTIKQHALN

SEQ ID NO: 42 - DNA, 3757 bp, Felis catus
tttctgctttgggacagccacgcatctaattccttaaaacagttttatatgtaaaacttgtaaaggatcagaacaatgcctccaagaccatcatcaggtgaactgtggggcatccacttgatgcccccaagaatcctagtagaatgtttactaccaaatggaatgatagtgacgttagaatgcctccgtgaggctacattaataactataaagcatgaattatttaaagaagcaagaaaatatcctctccatcaacttcttcaagatgaatcttcttacattttcgtaagtgttacccaagaagcagaaagggaagaattttttgatgaaacaagacgactttgtgacctgcggctttttcaaccctttttaaaagtaattgagccagtaggcaaccgtgaagaaaagatcctcaatcgagaaattggttttgctattggcatgccagtgtgtgaatttgatatggttaaagatccagaagtacaggacttccgaagaaatattctgaatgtttgtaaagaagctgtggatcttcgggatcttaattcacctcatagtagagcaatgtatgtctatcctccaaatgtagaatcttcaccagaactgccaaagcacatatataataaactagataaagggcaaataatagtggtgatttgggtaatagtttctccaaataatgacaagcagaagtatactctgaaaatcaaccatgactgtgtgccagaacaagtaattgctgaagcaatcaggaaaaaaactcgaagtatgttgctatcatctgaacaactaaaactctgtgttttagaataccagggcaagtatattttaaaagtgtgtggatgtgatgaatacttccttgaaaaatatcctctaagtcagtataagtacataagaagctgtataatgcttgggaggatgcccaatttgatgctgatggctaaagaaagcctttactcccaactgccaatggactgtttcacaatgccatcttattccagacgcatctccacagctacaccatatatgaatggagaaacatctacaaagtccctttgggttataaatagtgcactcagaataaaaatcctttgtgcaacctatgtgaatgtaaatattcgagacatcgacaagatctatgttcgaacaggtatctatcatggaggagaacccttatgtgataatgtgaacactcaaagagtaccttgttctaatcccaggtggaatgaatggctaaactacgatatatacattcctgatcttcctcgtgctgctcgactttgcctttccatttgttctgttaaaggccgaaagggtgctaaagaggaacactgtccattggcctggggaaatataaacttgtttgattacacagatactctagtatctggaaaaatggctttgaatctttggccagtacctcatggattagaagatttgctgaaccctattggtgttactgggtcaaatccaaataaagaaaccccatgcttagagttggagtttgactggttcagcagtgtggtaaagttcccagatatgtcagtgattgaagagcatgccaactggtctgtgtctcgagaagcaggatttagttattcccatgcaggactgagtaacagactagctagagacaacgaattaagagaaaatgataaagaacagctccgagcaatttgtacccgagatcctctatctgaaatcactgagcaagagaaagattttctgtggagccacagacactattgtgtaactatccctgaaattctacccaaactgcttctgtctgttaaatggaattctagagatgaagtagctcagatgtactgcttagtaaaagattggcctccaatcaaacctgaacaggcaatggagcttctggattgtaattacccagatcctatggttcgaggttttgctgttcgatgcttggaaaaatatttaacagatgacaagctttctcagtacttaattcagctagtacaggtcctaaaatatgaacagtatttggataacctgcttgtgagatttttactcaagaaagcattgactaatcaaaggattgggcactttttcttttggcatttaaaatctgagatgcacaataaaacagttagtcagaggtttggcctgcttttggagtcgtattgtcgtgcatgtgggatgtatttgaagcacctaaataggcaagttgaagctatggaaaagctcattaacttaactgacattctcaaacaagaaaagaaggatgaaacacaaaaggtacagatgaagtttttagttgagcaaatgcggagaccagatttcatggatgctctacagggttttctgtctcctctaaatcctgctcatcaactaggaaatctcaggcttgaagagtgtcgaattatgtcctctgcaaaaaggccactgtggttgaattgggagaacccagacatcatgtcagagttactctttcagaacaatgagatcatctttaaaaatggggatgatttacggcaagatatgttaacactgcagatcattcgcattatggaaaatatctggcaaaatcaaggccttgatcttcgaatgttaccttatggttgtctgtcaatcggtgactgtgtgggacttattgaggtggttagaaattctcacactattatgcagattcaatgcaaaggtggcctgaaaggcgcactgcagttcaacagccacactctacaccagtggctcaaagacaagaacaaaggcgaaatatacgatgcagccattgacctgttcacacgttcatgtgctggatattgtgttgctaccttcatactgggaatcggagatcgtcacaatagtaacatcatggttaaagatgatggacaactatttcatatagattttggacactttttggatcataagaagaaaaaatttggttataaacgggaacgtgtgccgtttgttttgacacaagatttcttaatagtgattagtaaaggagcccaagaatgcacaaagacaagagaattcgaaaggtttcaggagatgtgttacaaggcttatctagctattcggcagcatgccaatctcttcataaatctcttctcaatgatgcttggctctggaatgccagaactgcaatcttttgatgatattgcatacattcgaaagaccctagctttagataaaactgaacaagaggctttggaatatttcatgaaacaaatgaatgatgcacatcatggtggctggacaacaaaaatggattggatcttccacacaattaagcagcatgctttgaactgaaatgataactgagaaaccaaaagctcattatctggattctatactgcactgttaataactgtcaacaggcaaagactgattgcataggaattgcacaatccatgaacagcattagaatttacacaagaacagaaataaaatactatataatttaaataatgtaaacgcaaacagggtttgagagcactaaactagttcatttcaaaattaagctttagaataatgcgcaatttcatgttatgccttaagtccaaaaaggtaaactttgaagattgtttgtatctttttttaaaaaagaaaacaaaacaaaaaaaccccaaaatatatagaaatggtggagaaggaaaaagaatgatgttctttttttgtcttgcaaatgttctatgttttgaaattgtggacacaacaaagtctattattgcattaggtccaaggaaactgaagtttgatgttaaattgcattaagattagaaaa

SEQ ID NO: 43 - protein, 1068 aa, Felis catus; identical to SEQ ID NO: 41

SEQ ID NO: 44 - DNA, 3207 bp, Bos taurus
atgcctccaagaccatcatcaggtgaactgtggggcatccacttgatgcccccaagaatcctagtagaatgtttactaccaaatgggatgatagtgactttagaatgcctccgtgaggctacgttaataacgataaagcatgaactatttaaagaagcaagaaaataccctctccatcaacttcttcaagatgaatcttcttacattttcgtaagtgttacccaagaagcagaaagggaagaattttttgatgaaacaagacgactttgtgaccttcggctttttcaaccctttttaaaagtaattgaaccagtaggcaaccgtgaagaaaagatcctcaatcgagaaattggttttgctatcggcatgccagtgtgtgaattcgatatggttaaagatccagaagtacaggacttccgaagaaatattctcaatgtttgtaaagaagctgtggatcttagggatcttaattcacctcatagtagagcaatgtatgtttatcctccaaatgtagaatcttcaccagaactgccaaagcacatatataataaattggataaagggcaaataatagtggtgatttgggtaatagtttctccaaataatgacaaacagaagtatactctgaaaatcaaccatgactgtgtgccagaacaagtaattgctgaagcaatcaggaaaaaaactcgaagtatgttgctatcatctgaacaactaaaactctgtgttttagaatatcagggcaagtatattttaaaagtgtgtggatgtgatgaatacttcctagaaaaatatcctctgagtcagtataagtatataagaagctgtataatgcttgggaggatgcccaatttgatgctgatggctaaagaaagcctctattctcaactgccaatggactgttttacaatgccatcatattccagacgcatctccacagctacgccatatatgaatggagaaacatctacaaaatccctttgggttataaatagtgcactcagaataaaaattctttgtgcaacctatgtgaatgtaaatattcgagacattgacaagatttatgttcgaacaggtatctaccatggaggagaacccttatgtgataatgtgaacactcaaagagtaccttgttccaatcccaggtggaatgaatggctgaattacgatatatacattcctgatcttcctcgtgctgctcgactttgcctttccatttgttctgttaaaggccgaaagggtgctaaagaggaacactgtccattggcctggggaaatataaacttgtttgattacacagatactctagtatctggaaaaatggctttgaatctttggccagtacctcatggactagaagatttgctgaaccctattggtgttactggatcaaatccaaataaagaaactccatgtttagagttggagtttgactggttcagcagtgtggtaaagtttccagatatgtcagtgattgaagagcatgccaattggtctgtatcccgtgaagcaggatttagttattcccatgcaggactgagtaacagactagctagagacaatgaattaagagaaaatgataaagaacagctccgagcaatttgtacacgagatcctctatctgaaatcactgagcaagagaaagattttctgtggagccacagacactattgtgtaactatccccgaaattctacccaaattgcttctgtctgttaaatggaactctagagatgaagtagctcagatgtactgcttggtaaaagattggcctccaatcaagcctgaacaggctatggagcttctggactgcaattacccagatcctatggttcgaggttttgctgttcggtgcttagaaaaatatttaacagatgacaaactttctcagtacctaattcagctagtacaggtactaaaatatgaacagtatttggataacctgcttgtgagatttttactcaaaaaagcgttaactaatcaaaggatcggtcactttttcttttggcatttaaaatctgagatgcacaataaaacagttagtcagaggtttggcctgcttttggagtcctattgccgtgcatgtgggatgtatctgaagcaccttaataggcaagttgaggctatggaaaagctcattaacttgactgacattctcaaacaagagaagaaggatgaaacacaaaaggtacagatgaagtttttagttgagcaaatgcggcgaccagatttcatggatgctctccagggctttctgtctcctctaaaccctgctcatcagctgggaaatctcaggcttgaagagtgtcgaattatgtcttctgcaaaaaggccactgtggttgaattgggagaacccagacatcatgtcagaattactctttcagaacaatgagatcatctttaaaaatggggatgatttacggcaagatatgctaacccttcagattattcgcattatggaaaatatctggcaaaatcaaggtcttgatcttcgaatgttaccttatggatgtctgtcaatcggtgactgtgtgggacttatcgaggtggtgagaaattctcacactataatgcagattcagtgtaaaggaggcctgaaaggtgcactgcagtttaacagccacacactccatcagtggctcaaagacaagaacaagggggaaatatatgatgcggccatcgatttgtttacacgatcatgtgctggatattgtgttgccaccttcattttgggaattggagatcgtcacaatagtaatatcatggttaaagatgatggacaactgtttcatatagattttggacactttttggatcacaagaagaaaaaatttggttataaacgagagcgcgtgccgtttgttttgacacaagatttcttaatagtgattagtaaaggagcccaagaatgcacaaagacaagagaatttgagaggtttcaggagatgtgttacaaggcttatctagctattcggcagcatgccaatctcttcataaatcttttctcaatgatgcttggctctggaatgccagaactgcaatcttttgatgatattgcatacattcgaaagaccctagctttagataaaactgagcaagaggctttggagtatttcatgaaacaaatgaatgatgcacaccatggtggctggacaacaaaaatggattggatcttccacacaattaagcagcatgctttgaactga

SEQ ID NO: 45 - protein, 1068 aa, Bos taurus; identical to SEQ ID NO: 41

SEQ ID NO: 46 - DNA, 3452 bp, Gallus gallus
cggggctcgcgcgaaagcccggcggcgcaatgaaggtgagggccggcgcgcggtgaggtgggatcccggggcggcccccagacttgcatggtttaactcatacgaatcactgcttgaaagacttcaagtacaaaattgaaagactttaaaatgccaccccgaccatcatctggtgaactatggggcatccacttgatgcccccgaggatccttgtggagtgtcttctcccaaatggaatgatagtgactctagaatgcctccgtgaggccacactgctaactatcaaacatgaactttttaaagaagcaagaaaataccctctctatcagctccttcaagatgaatcttcttacatttttgtaagtgttacgcaagaagcagaaagagaagaattttttgatgaaacacggagactttgtgacctgcggctatttcaacctttcctaaaagtcattgaaccagtaggtaacagagaagaaaagatccttaatagagaaataggttttgctattggcatgcccatctgtgagtttgacatggttaaggatcctgaagtacaagatttcagaagaaacattcttaatgtttgtaaagaagcagtagatcttcgagatgccaatgctccacatagtagagcattatatgtctgtcctccaaatgtagaatcttcacctgagctacccaaacacatatacaataaactagataaagggcaaataatagtggtgatatgggtaatagtttcacctaacaacgataagcagaagtacaccttaaaaatcaatcatgactgtgtgcctgagcaagttattgctgaagcaattaggaagaaaacacgaagtatgttgctgtcatctgaacaactgaagctttgcgtgttggagtaccagggcaagtatattctgaaagtgtgtggctgtgatgaatacttgctagaaaaatatccactgagccagtataagtacataagaagttgtataatgcttggtcgcatgcccaatctcatgctgatggctaaagaaagcctatatacccagctgccgctcgatacctttacaatgccatcttactccaggcgtatctctacagctacaccctacatgaatggagaagctacagccaagtccctctggactataaacagtgctctcagaataagaatcctctgtgcaacctatgtaaatgtgaacattagagacattgacaaaatctacgttagaacaggtatctaccatggaggagaacctttatgtgacaatgtgaatactcagagggtaccttgttctaatcccagatggaatgaatggctgtcgtatgacatgtacattcctgatcttccacgtgctgctcggctctgcctctctatctgttctgttaaaggccggaagggtgctaaagaggagcactgtccattggcttggggaaacataaacatgtttgactacacggacactcttgtatctgggaaaatggctttgaatctttgggcagtaccccatggactggaggatttgttgaatcctataggtgttactggatcaaatccgaataaggaaactccatgtttagagctggaatttgattggtttagcaatcctgttaagtttccagatatgacagtgattgaagaacatgccaattggacgatctcacgtgaactgggctttaactacagctatgcgggactgagtaacagaatagctagagacaatgaattaagagaaagtgacaaggagcaactgagagccatatgtacgcgagatcctttgtctgaaatcactgagcaagagaaggacttcctctggagccacagacactattgtgtaaatacgccagaaattctgcccaaattacttctgtctgttaaatggaattctagagatgaagtggctcagatgtactgtttggtaaaagattggcctccaatcaagccagagcaagcaatggagcttttggattgtaattatccagatccaatggtgcgggcttttgcagttcggtgtctagagaagtacttaacagatgacaaactgtctcagtacttaatccagctagtacaggttctgaaatatgagcagtacttagataatcaactcgtgagatttttactcaagaaggcactgaccaatcaacggataggacacttcttcttttggcatttaaagtctgaaatgcacaataaaactgtaagtcagaggtttggtttacttctggagtcctattgtcgagcatgtggaatgtacctaaagcatctgagcaggcaggtggaggctatggagaagttgattaacctcacagatattctcaagcaggaaaagaaagatgagacccagaaggtgcagatgaagtttcttgttgaacaaatgagacgtccagattttatggatgctttacaaggctttatctctcctcttaatcctgctcatcaactgggaaatcttcggcttgaggagtgcagaataatgtcatctgcaaaaaggcccctgtggttaaactgggaaaacccagatattatgtctgaattgctatttcagaacaatgagataatctttaaaaatggagatgacttgcgtcaagacatgctgacacttcagataattagaattatggaaaacatctggcaaaaccaaggtcttgatcttcggatgttgccttacggttgtttgtctattggtgactgtgtgggactcattgaggtagtgagaagttctcatacaatcatgcagattcagtgtaaaggaggcttaaagggagcattgcagttcaacagccatacattgcatcagtggctcaaggacaagaacaaaggagaaatgtatgatgcagctattgacttgtttacacgttcttgtgctggctactgtgtcgctacctttatactgggcattggtgatcgccacaacagtaacatcatggtgaaagatgatggacaactgtttcatattgactttggccacttccttgaccacaagaagaagaaatttggctacaaaagagagcgtgtgccctttgtcttaacacaggactttttaatagtgattagtaaaggagcccaagaatgtaccaaaacaagggagtttgaaaggtttcaagagatgtgttataaggcatatctagcaattcggcagcatgccaatctgttcataaatctcttctccatgatgcttggctcaggaatgccagaactgcagtcctttgacgatattgcatacattcgaaagacccttgcattggacaaaactgagcaggaagctcttgagtacttcatgaagcaaatgaatgatgctcaccatggtggctggacaacaaaaatggactggatcttccacacaataaagcaacatgctttgaactgaaatgaaagtgaagaaaacaactaataacccgctttgtgggtactacactgttaatacctgttagcagcaaagactggttgcataggaattgcaca

SEQ ID NO: 47 - protein, 1068 aa, Gallus gallus
MPPRPSSGELWGIHLMPPRILVECLLPNGMIVTLECLREATLLTIKHELFKEARKYPLYQLLQDESSYIFVSVTQEAEREEFFDETRRLCDLRLFQPFLKVIEPVGNREEKILNREIGFAIGMPICEFDMVKDPEVQDFRRNILNVCKEAVDLRDANAPHSRALYVCPPNVESSPELPKHIYNKLDKGQIIVVIWVIVSPNNDKQKYTLKINHDCVPEQVIAEAIRKKTRSMLLSSEQLKLCVLEYQGKYILKVCGCDEYLLEKYPLSQYKYIRSCIMLGRMPNLMLMAKESLYTQLPLDTFTMPSYSRRISTATPYMNGEATAKSLWTINSALRIRILCATYVNVNIRDIDKIYVRTGIYHGGEPLCDNVNTQRVPCSNPRWNEWLSYDMYIPDLPRAARLCLSICSVKGRKGAKEEHCPLAWGNINMFDYTDTLVSGKMALNLWAVPHGLEDLLNPIGVTGSNPNKETPCLELEFDWFSNPVKFPDMTVIEEHANWTISRELGFNYSYAGLSNRIARDNELRESDKEQLRAICTRDPLSEITEQEKDFLWSHRHYCVNTPEILPKLLLSVKWNSRDEVAQMYCLVKDWPPIKPEQAMELLDCNYPDPMVRAFAVRCLEKYLTDDKLSQYLIQLVQVLKYEQYLDNQLVRFLLKKALTNQRIGHFFFWHLKSEMHNKTVSQRFGLLLESYCRACGMYLKHLSRQVEAMEKLINLTDILKQEKKDETQKVQMKFLVEQMRRPDFMDALQGFISPLNPAHQLGNLRLEECRIMSSAKRPLWLNWENPDIMSELLFQNNEIIFKNGDDLRQDMLTLQIIRIMENIWQNQGLDLRMLPYGCLSIGDCVGLIEVVRSSHTIMQIQCKGGLKGALQFNSHTLHQWLKDKNKGEMYDAAIDLFTRSCAGYCVATFILGIGDRHNSNIMVKDDGQLFHIDFGHFLDHKKKKFGYKRERVPFVLTQDFLIVISKGAQECTKTREFERFQEMCYKAYLAIRQHANLFINLFSMMLGSGMPELQSFDDIAYIRKTLALDKTEQEALEYFMKQMNDAHHGGWTTKMDWIFHTIKQHALN

SEQ ID NO: 48 - DNA, 2949 bp, Homo sapiens
cgcctcccttccccctccccgcccgacagcggccgctcgggccccggctctcggttataagatggcggcgctgagcggtggcggtggtggcggcgcggagccgggccaggctctgttcaacggggacatggagcccgaggccggcgccggcgccggcgccgcggcctcttcggctgcggaccctgccattccggaggaggtgtggaatatcaaacaaatgattaagttgacacaggaacatatagaggccctattggacaaatttggtggggagcataatccaccatcaatatatctggaggcctatgaagaatacaccagcaagctagatgcactccaacaaagagaacaacagttattggaatctctggggaacggaactgatttttctgtttctagctctgcatcaatggataccgttacatcttcttcctcttctagcctttcagtgctaccttcatctctttcagtttttcaaaatcccacagatgtggcacggagcaaccccaagtcaccacaaaaacctatcgttagagtcttcctgcccaacaaacagaggacagtggtacctgcaaggtgtggagttacagtccgagacagtctaaagaaagcactgatgatgagaggtctaatcccagagtgctgtgctgtttacagaattcaggatggagagaagaaaccaattggttgggacactgatatttcctggcttactggagaagaattgcatgtggaagtgttggagaatgttccacttacaacacacaactttgtacgaaaaacgtttttcaccttagcattttgtgacttttgtcgaaagctgcttttccagggtttccgctgtcaaacatgtggttataaatttcaccagcgttgtagtacagaagttccactgatgtgtgttaattatgaccaacttgatttgctgtttgtctccaagttctttgaacaccacccaataccacaggaagaggcgtccttagcagagactgccctaacatctggatcatccccttccgcacccgcctcggactctattgggccccaaattctcaccagtccgtctccttcaaaatccattccaattccacagcccttccgaccagcagatgaagatcatcgaaatcaatttgggcaacgagaccgatcctcatcagctcccaatgtgcatataaacacaatagaacctgtcaatattgatgacttgattagagaccaaggatttcgtggtgatggaggatcaaccacaggtttgtctgctaccccccctgcctcattacctggctcactaactaacgtgaaagccttacagaaatctccaggacctcagcgagaaaggaagtcatcttcatcctcagaagacaggaatcgaatgaaaacacttggtagacgggactcgagtgatgattgggagattcctgatgggcagattacagtgggacaaagaattggatctggatcatttggaacagtctacaagggaaagtggcatggtgatgtggcagtgaaaatgttgaatgtgacagcacctacacctcagcagttacaagccttcaaaaatgaagtaggagtactcaggaaaacacgacatgtgaatatcctactcttcatgggctattccacaaagccacaactggctattgttacccagtggtgtgagggctccagcttgtatcaccatctccatatcattgagaccaaatttgagatgatcaaacttatagatattgcacgacagactgcacagggcatggattacttacacgccaagtcaatcatccacagagacctcaagagtaataatatatttcttcatgaagacctcacagtaaaaataggtgattttggtctagctacagtgaaatctcgatggagtgggtcccatcagtttgaacagttgtctggatccattttgtggatggcaccagaagtcatcagaatgcaagataaaaatccatacagctttcagtcagatgtatatgcatttggaattgttctgtatgaattgatgactggacagttaccttattcaaacatcaacaacagggaccagataatttttatggtgggacgaggatacctgtctccagatctcagtaaggtacggagtaactgtccaaaagccatgaagagattaatggcagagtgcctcaaaaagaaaagagatgagagaccactctttccccaaattctcgcctctattgagctgctggcccgctcattgccaaaaattcaccgcagtgcatcagaaccctccttgaatcgggctggtttccaaacagaggattttagtctatatgcttgtgcttctccaaaaacacccatccaggcagggggatatggtgcgtttcctgtccactgaaacaaatgagtgagagagttcaggagagtagcaacaaaaggaaaataaatgaacatatgtttgcttatatgttaaattgaataaaatactctctttttttttaaggtgaaccaaagaacacttgtgtggttaaagactagatataatttttccccaaactaaaatttatacttaacattggatttttaacatccaagggttaaaatacatagacattgctaaaaattggcagagcctcttctagaggctttactttctgttccgggtttgtatcattcacttggttattttaagtagtaaacttcagtttctcatgcaacttttgttgccagctatcacatgtccactagggactccagaagaagaccctacctatgcctgtgtttgcaggtgagaagttggcagtcggttagcctgggttagataaggcaaactgaacagatctaatttaggaagtcagtagaatttaataattctattattattcttaataatttttctataactatttctttttataacaatttggaaaatgtggatgtcttttatttccttgaagcaataaactaagtttctttttataaaaa

SEQ ID NO: 49 - protein, 766 aa, Homo sapiens [sequence omitted]

SEQ ID NO: 50 - DNA, 3906 bp, Rattus norvegicus
atggcggcgctgagtggcggcggtggcagcagcagcggtggcggtggcggcggcggcggcggcggtggtggcggcggcggcggcggcgccgaacagggacaggctctgttcaatggcgacatggagccggaggccggcgctggcgccgcggcctcttcggccgcggacccggccattcctgaagaggtgtggaatatcaagcaaatgattaagttgacacaggaacatatagaggccctattggacaagtttggtggggagcataacccaccgtcaatatacctggaggcctatgaagagtacaccagcaagctagatgcccttcagcagagagagcagcagctgttggaatccctggtttttcaaactcccacagatgtatcacggaacaaccccaagtcaccacagaaacctatcgttcgtgtcttcctgcccaacaaacagaggacagtggtgcccgcaagatgtggtgtaacggtccgagacagtctaaagaaagcactaatgatgaggggtctcatcccagagtgctgtgctgtttacagaattcaggacggagagaagaaaccaattggctgggacactgacatttcctggcttactggagaggagctacatgttgaagtactagagaatgttcctctgacaacccacaacttcgtacggaaaacttttttcaccttagcattttgtgacttttgccgaaagctgcttttccagggtttccgctgtcaaacatgtggttataagtttcaccagcgttgtagtacagaggttccactgatgtgtgttaattatgaccaacttgatttgctgtttgtctccaagttctttgagcatcacccagtaccacaggaggaggccttctcagcagagactacccttccatctggatgctcttccgcacccccctcagactctattgggccccaaatcctcaccagtccatctccttcaaaatccattccaattccacagcccttccggccagcagatgaagatcatcgcaatcagtttgggcaacgagaccgctcctcctccgctcccaatgttcatataaacacaatcgaacctgtcaatattgatgaaaaattcccagaagtggaattacaggatcaaagggatttgattagagaccaggggtttcgtggggatggagcccctttgaaccagctgatgcgctgtcttcggaaataccaatcccggactcccagccccctcctccattctgtccccagtgaaatagtgtttgattttgagcctggcccagtgttcagagggtcaaccacaggcttgtcggccaccccacctgcctcattacctggctcactcactaacgtgaaagccttacagaaatctccaggacctcagcgggaaaggaagtcctcctcctcctcctcctccacggaagacagaagtcggatgaaaacacttggtagaagagattcaagtgatgattgggagattcctgatggacagattacagtgggacagagaattggatctgggtcctttggaactgtctacaagggaaagtggcatggcgacgtggcagtgaaaatgctgaatgtgacagcacccacacctcagcagttacaggccttcaaaaacgaagtcggagtactcaggaaaactcgacatgtgaacatcctccttttcatgggctattctacaaagccacagctggctattgttacacagtggtgtgaaggctccagcttatatcaccatctccacatcattgagaccaaatttgagatgatcaaacttatagatattgcacggcagactgcacagggcatggattacttacacgccaagtcaatcatccacagagacctcaagagtaataatatatttcttcatgaagacctcacggtaaaaataggtgactttggtttagccacagtgaagtcccgatggagtgggtcccatcagtttgaacagttgtctggatctattttgtggatggcacccgaagtaatcagaatgcaagataaaaacccatatagctttcagtcagacgtgtatgcatttgggattgttctgtatgaactgatgactggtcagctaccttattcaaacatcaacaacagggatcagataatttttatggtgggacgaggatacctatctccagatctcagtaaggtacggagtaactgtccaaaagccatgaagagattaatggcagagtgcctcaaaaagaaaagagacgagagaccactctttccccaaattctcgcctctattgagctgctggcccgctcattgccaaaaattcaccgcagtgcatcagaaccctccttgaatcgggctggtttccaaacagaagattttagtctgtatgcttgtgcttctccaaaaacacccatccaagcagggggatatggagaatttgcagccttcaagtagccactccatcatggcagcatctactctttatttcttaagtcttgtgttcatacaatttgttaacatcaaaacacagttctgttcctcaaattttttttaaagatacaaaattttcaatgcataagctcgtgtggaacagaatggaatttcctattcaacaaaagagggaagaatgttttaggaaccagaattctctgctgcccgtgtttcttcttcaacacaaatatcatgtgcatacaactctgcccattcccaagaagaaagaggagagaccccgaattctgcccttttggtggtcaggcatgatggaaagaatttgctgctgcagcttgggaaaaattgctatggaaagtctgccagtcaactttgcccttctaaccaccagatccatttgtggctggtcatctgatggggcgatttcaatcaccaagcatcgttcttgcctgttgtgggattatgtcgtggagcactttccctatccaccaccgttaatttccgagggatggagtaaatgcagcataccctttgtgtagcacctgtccagtcctcaaccaatgctatcacagtgaagctctttaaatttaagtggtgggtgagtgttgaggagagactgccttgggggcagagaaaaggggatgctgcatcttcttcctcacctccagctctctcacctcgggttgccttgcacactgggctccgcctaaccactcgggctgggcagtgctggcacacattgccgccttttctcattgggtccagcaattgagcagagggttgggggattgtttcctccacaatgtagcaaattctcaggaaaatacagtccatatcttcctctcagctcttccagtcaccaaatacttacgtggctcctttgtccaggacataaaacaccgtggacaacacctaattaaaagcctacaaaactgcttactgacagttttgaatgtgagacatttgtgtaatttaaatgtaaggtacaggtcttaatttcttctattaagtttcttctatttttatttaaacgaagaaaataattttcaggtttaattggaataaacgaatacttcccaaaagactatataccctgaaaattatatttttgttaattgtaaacaacttttaaaaaatggttattatccttttctctacctaaaattatgggaaatcttagcataatgacaattatttatactttttaaataaatggtacttgctggatccacactaacatctttgctaacattcccattgtttcttccaacttcactcctacactacatcctccatcctctttctagtcttttatctataatatgcaacctaaaataaaagtggtggtgtctccattcattcttcttcttccttttttccccaagcctggtcttcaaaaggttgggtaatttagtagctgagttccctaggtagaaatagaactattagggacattggggttgtaggaaagcgtgaggcctgtcaccagttgttctt

SEQ ID NO: 51 - protein, 804 aa, Rattus norvegicus
MAALSGGGGSSSGGGGGGGGGGGGGGGGGAEQGQALFNGDMEPEAGAGAAASSAADPAIPEEVWNIKQMIKLTQEHIEALLDKFGGEHNPPSIYLEAYEEYTSKLDALQQREQQLLESLVFQTPTDVSRNNPKSPQKPIVRVFLPNKQRTVVPARCGVTVRDSLKKALMMRGLIPECCAVYRIQDGEKKPIGWDTDISWLTGEELHVEVLENVPLTTHNFVRKTFFTLAFCDFCRKLLFQGFRCQTCGYKFHQRCSTEVPLMCVNYDQLDLLFVSKFFEHHPVPQEEAFSAETTLPSGCSSAPPSDSIGPQILTSPSPSKSIPIPQPFRPADEDHRNQFGQRDRSSSAPNVHINTIEPVNIDEKFPEVELQDQRDLIRDQGFRGDGAPLNQLMRCLRKYQSRTPSPLLHSVPSEIVFDFEPGPVFRGSTTGLSATPPASLPGSLTNVKALQKSPGPQRERKSSSSSSSTEDRSRMKTLGRRDSSDDWEIPDGQITVGQRIGSGSFGTVYKGKWHGDVAVKMLNVTAPTPQQLQAFKNEVGVLRKTRHVNILLFMGYSTKPQLAIVTQWCEGSSLYHHLHIIETKFEMIKLIDIARQTAQGMDYLHAKSIIHRDLKSNNIFLHEDLTVKIGDFGLATVKSRWSGSHQFEQLSGSILWMAPEVIRMQDKNPYSFQSDVYAFGIVLYELMTGQLPYSNINNRDQIIFMVGRGYLSPDLSKVRSNCPKAMKRLMAECLKKKRDERPLFPQILASIELLARSLPKIHRSASEPSLNRAGFQTEDFSLYACASPKTPIQAGGYGEFAAFK

SEQ ID NO: 52 - DNA, 9728 bp, Mus musculus
ccctcaggctcggctgcgccggggccgccggcgggttccagaggtggcctccgccccggccgctccgcccacgccccccgcgcctccgcgcccgcctccgcccgccctgcgcctcccttccccctccccgccccgcggcggccgctcggcccggctcgcgcttcgaagatggcggcgctgagtggcggcggtggcagcagcagcggtggcggcggcggcggtggcggcggcggtggcggtggcgacggcggcggcggcgccgagcagggccaggctctgttcaatggcgacatggagccggaggccggcgctggcgccgcggcctcttcggctgcggacccggccattcctgaagaggtatggaatatcaagcaaatgattaagttgacacaggaacatatagaggccctattggacaaatttggtggagagcataacccaccatcaatatacctggaggcctatgaagagtacaccagcaagctagatgcccttcagcaaagagaacagcagcttttggaatccctggtttttcaaactcccacagatgcatcacggaacaaccccaagtcaccacagaaacctatcgttagagtcttcctgcccaacaaacagaggacagtggtacccgcaagatgtggtgttacagttcgagacagtctaaagaaagcactgatgatgagaggtctcatcccagaatgctgtgctgtttacagaattcaggatggagagaagaaaccaattggctgggacacggacatttcctggcttactggagaggagttacatgttgaagtactggagaatgtcccacttacaacacacaactttgtacggaaaacttttttcaccttagcattttgtgacttttgccgaaagctgcttttccagggtttccgttgtcaaacatgtggttataaatttcaccagcgttgtagtacagaggttccactgatgtgtgtaaattatgaccaacttgatttgctgtttgtctccaagttctttgagcatcacccagtaccacaggaggaggcctccttcccagagactgcccttccatctggatcctcttccgcacccccctcagactctactgggccccaaatcctcaccagtccatctccttcaaaatccattccaattccacagcccttccgaccagcagatgaagatcatcgcaatcagtttgggcaacgagaccggtcctcctcagctcccaatgttcatataaacacaattgagcctgtgaatatcgatgaaaaattcccagaagtggaattacaggatcaaagggatttgattagagaccaggggtttcgtggtgatggagcccccttgaaccaactgatgcgctgtcttcggaaataccaatcccggactcccagccccctcctccattctgtccccagtgaaatagtgtttgattttgagcctggcccagtgttcagagggtcaaccacaggcttgtccgccaccccgcctgcctcattacctggctcactcactaacgtgaaagccttacagaaatctccaggtcctcagcgggaaaggaagtcatcttcttcctcatcctcggaggacagaagtcggatgaaaacacttggtagaagagattcaagtgatgactgggagattcctgatggacagattacagtgggacagagaattggatctgggtcatttggaactgtctacaagggaaagtggcatggtgatgtggcagtgaaaatgttgaatgtgacagcacccacacctcaacagctacaggccttcaaaaatgaagtaggagtgctcaggaaaactcgacatgtgaatatcctccttttcatgggctattctacaaagccacaactggcaattgttacacagtggtgtgagggctccagcttatatcaccatctccacatcattgagaccaaatttgagatgatcaaacttatagatattgctcggcagactgcacagggcatggattacttacacgccaagtcaatcatccacagagacctcaagagtaataatatatttcttcatgaagacctcacggtaaaaataggtgactttggtctagccacagtgaaatctcggtggagtgggtcccatcagtttgaacagttgtctggatctattttgtggatggcaccagaagtaatcagaatgcaagataaaaacccgtatagctttcagtcagacgtgtatgcgtttgggattgttctgtacgaactgatgaccggccagctaccttattcaaacatcaacaacagggatcagataatttttatggtgggacgaggatacctatctccagatctcagtaaggtacggagtaactgtccaaaagccatgaagagattaatggcagagtgcctcaaaaagaaaagagacgagagaccactctttccccaaattctcgcctccattgagctgctggcccgctcattgccaaaaattcaccgcagtgcatcagaaccttccttgaatcgggctggtttccaaacagaagattttagtctgtatgcttgtgcttctccgaaaacacccatccaagcagggggatatggagaatttgcagccttcaagtagccagtccatcatggcagcatctactctttatttcttaagtcttgtgttcatacagtttgttaacatcaaaacacagttctgttcctcaaaaaattttttaaagatacaaaattttcaatgcataagttcatgtggaacagaatggaatttcctattcaacaaaagagggaagaatgttttaggaaccagaattctctgctgcccgtgtttcttcttcaacataactatcacgtgcatacaagtctgcccattcccaagaagaaagaggagagaccctgaattctgcccttttggtggtcaggcatgatggaaagaatttgctgctgcagcttgggaaaattgctatggaaagtctgccagtcgactttgcccttctaaccaccagatcagcctgtggctggtcatctgatggggcgatttccatcaccaagcatcgttcttgcctattctgggattatgttgtggagcactttccctgtccagcaccgttcatttctgagggatggagtaaatgcagcattcccttgtgtagcgcctgttcagtcctcagcagctgctgtcacagcgaagctttttacagttaagtggtgggggagagttgaggagagcctgcctcggggcagagaaaagggggtgctgcatcttcttcctcacctccagctctctcacctcgggttgccttgctcactgggctccgcctaaccactcaggctgctcagtgctggcacacattgccttcttttctcattgggtccagcaattgaggagagggttgggggattgtttcctcctcaatgtagcaaattctcaggaaaatacagtccatatcttcctctcagctcttccagtcaccaaatacttacgtggctcctttgtccaggacataaaacaccgtggacaacacctaattaaaagcctacaaaactgcttactgacagttttgaatgtgagacacttgtgtaatttaaatgtaaggtacaggttttaatttctgagtttcttctatttttatttaaaagaagaaaataattttcagttttaattggaataaatgagtacttcccacaagactatataccctgaaaattatatttttgttaattgtaaacaacttttaaagaataattattatccttttctctacctaaaaattatggggaatcttagcataatgacaattatttatactttttaaataaatggtacttgctggatccacactaacatctttgctaacaatcccattgtttcttccaacttaactcctacactacatcctacatcctctttctagtcttttatctataatatgcaacctaaaataaacgtggtggcgtctccattcattctccctcttcctgttttccccaagcctggtcttcaaaaggttgggtaatcggtccctgagctccctagctggcaatgcaactattagggacattggagttgcaggagagcaggaagcctgtccccagctgttcttctagaaccctaaatcttatctttgcacagatcaaaagtatcacctcgtcacagttctccttagcctttacttacaggtaatataaataaaaatcaccatagtagtaaagaaaacaactggatggattgatgaccagtacctctcagagccaggaatcttgaatctccaggatttatacgtgcaaatttaaggagatgtacttagcaacttcaagccaagaacttccaaaatactagcgaatctaaaataaaatggaattttgagttatttttaaagttcaaattataattgataccactatgtatttaagcctactcacagcaagttagatggattttgctaaactcattgccagactgtggtggtggtggtggtagtgtgcacctttaatccaagcaactcagcaatcagaatgaggtaaatctctgtgaatacaaggcctgcctagtctgcagcgctagttccaggatagccagggctacacacacaaaaaccctctctcaaaaaaaacaaaattaattagttgataataaaaaataactaaagtatcatcaaaggaaggcctactggaagttttatatattcccagtaaattgaaaaatattctgaagttattaaccagttagcaacaatgtgtttttaagtcttacataaacagagcaaagtcttcaaatgtttcagagctgagaagataattgtgcttgatatgaaaaatagcctctccatatgatgtgccacattgaaaggcgtcattacccttttaaatacttcttaatgtggctttgttccctttacccaggattagctagaaagagctaggtaggcttcggccacagttgcacatttcgggcctgctgaagaatgggagctttgaaggctggccttggtggaggagcccctcagtgctggagggtggggcgtgtacgcagcatggaagtggtctagacagagtgcaaagggacagacttctttctcattttagtatagggtgatgtctcacttgaaatgagaaagtagagttgatattaaacgaagctgtgcccagaaaccaggctcagggtattgtgagattttctttttaaatagagaatataaaagatagaaataaatatttaaaccttccttcttattttctatcaaatagattttttttatcatttgcaaacaacataaaaaaaggtttcttttgtggggttttctttccttcttttttttttttttttttttttaagactgcagataatcttgttgagctcctcggaaaatacaaggaagtccgtgtttgtgcagagcgctttatgagtaactgtatagacagtgtggctgcttcactcatcccagagggctgcagctgtcggcccatgaagtggctgcagtgcctcgtgagatctgctttgttttgtttggagtgaagtctttgaaaggtttgagtgcaactatataggactgtttttaaataagtagtattcctcatgaactttctcattgttaagctacaggacccaaactctaccactaagatattattaacctcaaaatgtagtttatagaaggaatttgcaaatagaatatccagttcgtacttatatgcatcttcaacaaagattctctgtgacttgttggatttggttcctgaacagcccatttctgtatttgaggttaggagggcataatgaggcatcctaaaagacaatctgatataaactgtatgctagatgtatgctggtaggggagaaagcattctgtaaagacatgatttaagacttcagctctgtcaaccagaaaccttgtaaatacttcctgtcttggtgcagccccgcccctttgatcacacgatgttgtcttgtgcttgtcagacactgtcagagctgctgttcgtccctctgcagatctcacctgtccccactgcacacccacctcctgcctcttgcagacctcagcatctagctttagttggaaacagttcagggttcaggtgacttcttaaaaaaaaaaaaaaaccctacctcctcagaatgaggtaatgaatagttatttatttaaagtatgaagagtcaggagcgctcgaacatgaaggtgatttaagatggttcctttcgtgtgtattgtagctgagcacttgtttttgtcctaaagggcattatacatttaagcagtgattctgtttaaagatgtttttctttaaaggtgtagctcagagtatctgttgttggaattggtgccagagtctgcttaatagatttcagaatcctaagcttaagtcagtcgcatgaagttaagtagttatggtaacactttgctagccatgatataattctactttttaggagtaggtttggcaaaactgtatgccttcaaagtgagttggccacagctttgtcacatgcacagatactcatctgaagagactgcccagctaagagggcggaaggatacccttttttcctacgattcgcttctttgtccacgttggcattgttagtactagtttatcagcaccttgaccagcagatgtcaaccaataagctatttttaaaaccatagccagagatggagaggtcactgtgagtagaaacagcaggacgcttacaggagtgaaatggtgtagggaggctctagaaaaatatcttgacaatttgccaaatgatcttactgtgccttcatgatgcaataaaaaagctaacattttagcagaaatcagtgatttacgaagagagtggccagtctggtttaactcagctgggataatatttttagagtgcaatttagactgcgaagataaatgcactaaagagtttatagccaattcacatttgaaaaataagaaaatggtaaattttcagtgaaatatttttttaaagcacataatccctagtgtagccagaaatatttaccacatagagcagctaggctgagatacagtccagtgacatttctagagaaaccttttctactcccacgggctcctcaaagcatggaaattttatacaaaatgtttgacattttaagatactgctgtagtttagttttgaaatagtatgtgctgagcagcaatcatgtactaactcagagagagaaaacaacaacaaattgtgcatctgatttgttttcagagaaatgctgccaacttagatactgagttctcagagcttcaagtgtaaacttgcctcccaagtcctgtttgcaaatgaagttggctagtgctactgactgctccagcacatgatggaaggcagggggctgtctctgaagtgtcttctataaagggacaatagaatagtgagagacctggtcagtgtgtgtcagctggacactccatgctatgggacttgcatcttctgtcctcaccatccccaagacattgtgctttcctcagttgtcctctagctgtttcactcagacaccaagatgaattactgatgccagaaggggccaaaatggccagtgtgttttgggggttgtatcagttgactggacaataactttaatagtttcagatcatttatttttacttccattttgacagacatttaaatggaaatttagtcctaacttttgtcatttgaaaggaaaaattaacagttcctataagatacttttgaggtggaatctgacatcctaattttttttcttttcagtgggtttgcagcgagggtcttgtatgcactaggcaagggttctaccactaagccacatttcccaggaaataaaatgttaacagttaaaacatacacacaaatacacaaacaccttattaccactttagtaaagtgagagatgtgcgtcctttgtctcagtctccacgatttcagctgccccttgtatgaataactcagtctcgctaaactgtttacttttatttacctggtttgactagttgcagctatataaccagttgtgcatgaggacaacagccagtgtgtttgttttgtttttggttttttgtggtacattttttgtaaagaattctgtagattgaagtgctctttgaaaacagaactgagatatatttattcttgttagcatcaaaaaacattttgtgcaaatgatttgcttttcctggcaggctgagtaccatatccagcgcccacaattgcgggttcccatctaccatgtccacaggggagacagacgggaagcacatgaggggtgtgtttacagagttgtaggagttatgtagttctcttgttgccttggaaatcactgttgttttaagactgttgaacccgtgtgtttggctgggctgtgagttacatgaagaaactgcaaactagcatatgcagacaaagctcacagactaggcgtaaatggaggaaaatggaccaaaataaggcagggtgacacataaaccttgggcttcggagaaaactaagggtggagatgaactataatcacctgaatacaatgtaagagtgcaataagtgtgcttattctaagctgtgaacttcttttaaatcattcctttctaatacatttatgtatgttccattgctgactaaaaccagctatgagaacatatgcctttttattcatgttaactaccagtttaagtggctaaccttaatgtcttatttatcttcattttgtattagtttacataccaggtatgtgtgtgtgctgtactcttcttccctttatttgaaaacacttttcactgggtcatctccttggccattccacaacacaactttggtttggctttcaatgtcaccttatttgatggcctgtgtcccagtagcagaatttatggtattcccattgctggctgctcttccgaccctttgcttctacagcacttgtctctcctaagatagtcagaaactaactgatcaggggatggacttcaccattcatcgtgtctcttcaattctattaaatagaccactcttgggctttagaccaggaaaaaggagacagctctagccatctaccaagcctcaccctaaaaggtcacccgtacttcttggtctgaggacaagtctccactccagtaagggagaggggaggaaatgcttcctgtttgaaatgcagtgaattcctatggctcctgtttcaccacccgcacctatggcaacccatatacattcctcttgtctgtaactgccaaaggttgggtttatgtcacttcagttccactcaagcattgaaaaggttctcatggagtctggggtgtgcccagtgaaaagatggggactttttcattatccacagacctctctatacctgctttgcaaaaattataatggagtaactatttttaaagcttatttttcaattcataagaaaaagacatttattttcaatcaaatggatgatgtctcttatcccttatccctcaatgtttgcttgaattttgtttgttccctatacctactccctaattctttagttccttcctgctcaggtcccttcatttgtactttggagtttttctcatgtaaatttgtataatggaaaatattgttcagtttggatagaaagcatggagaaataaataaaaaaagatagctgaaaatcaaattgaagaaatttatttctgtgtaaagttatttaaaaactctgtattatatttaaagaaaaaagcccaaccccccaaaaagtgctatgtaattgatgtgaatatgcgaatactgctataataaagattgactgcatggagaaa

SEQ ID NO: 53 - protein, 804 aa, Mus musculus
MAALSGGGGSSSGGGGGGGGGGGGGDGGGGAEQGQALFNGDMEPEAGAGAAASSAADPAIPEEVWNIKQMIKLTQEHIEALLDKFGGEHNPPSIYLEAYEEYTSKLDALQQREQQLLESLVFQTPTDASRNNPKSPQKPIVRVFLPNKQRTVVPARCGVTVRDSLKKALMMRGLIPECCAVYRIQDGEKKPIGWDTDISWLTGEELHVEVLENVPLTTHNFVRKTFFTLAFCDFCRKLLFQGFRCQTCGYKFHQRCSTEVPLMCVNYDQLDLLFVSKFFEHHPVPQEEASFPETALPSGSSSAPPSDSTGPQILTSPSPSKSIPIPQPFRPADEDHRNQFGQRDRSSSAPNVHINTIEPVNIDEKFPEVELQDQRDLIRDQGFRGDGAPLNQLMRCLRKYQSRTPSPLLHSVPSEIVFDFEPGPVFRGSTTGLSATPPASLPGSLTNVKALQKSPGPQRERKSSSSSSSEDRSRMKTLGRRDSSDDWEIPDGQITVGQRIGSGSFGTVYKGKWHGDVAVKMLNVTAPTPQQLQAFKNEVGVLRKTRHVNILLFMGYSTKPQLAIVTQWCEGSSLYHHLHIIETKFEMIKLIDIARQTAQGMDYLHAKSIIHRDLKSNNIFLHEDLTVKIGDFGLATVKSRWSGSHQFEQLSGSILWMAPEVIRMQDKNPYSFQSDVYAFGIVLYELMTGQLPYSNINNRDQIIFMVGRGYLSPDLSKVRSNCPKAMKRLMAECLKKKRDERPLFPQILASIELLARSLPKIHRSASEPSLNRAGFQTEDFSLYACASPKTPIQAGGYGEFAAFK

SEQ ID NO: 54 - DNA, 2232 bp, Oryctolagus cuniculus
atggggaatgtgtggaatatcaaacaaatgattaagttgacacaggagcatatagaggccctattggacaaatttggtggggagcataatccaccatcaatatatctggaggcctacgaagaatacaccagcaagctagatgccctccaacaaagagaacagcagttattggaatccctagtttttcaaaatcccacagatgtgtcacggagcaaccccaagtcaccacaaaaacctattgttagagtcttcctgcccaacaaacagaggacagtggtacctgcaagatgtggagttacggttcgagacagtctaaagaaagcgctgatgatgagaggtctgatcccagaatgctgtgctgtttacagaattcaggatggagagaagaagccaattggctgggacactgatatttcctggctcactggagaagagctgcatgtggaagtgttagagaatgtcccactcaccacacataactttgtacggaaaacttttttcaccttagcattttgtgacttctgtagaaagctgcttttccagggtttccgctgtcaaacatgtggctacaaatttcaccagcgttgtagtacggaagttccactgatgtgtgttaattatgaccaacttgatttgctgtttgtctccaagttctttgaacaccacccagtaccacaggaggaggcctccttagcagagactgccctcacatctgggtcatcgccttccgcacctccctcagactctattgggcaccaaattctcaccagtccgtccccttcaaaatccattccgattccacagtccttccgaccagcagatgaagatcatcgaaatcagtttgggcaacgagaccggtcttcatcagcgcctaatgttcacattaacacaatagaacctgtcaatattgatgaaaaattcccagaagtggaattacaggatcaaagggacttgattagagaccaagggtttcgtggtgatggagcccctttgaaccagctgatgcgctgtcttcggaaataccaatcccggactcccagtcccctcctaccttctgtccccagtgacatagtgtttgattttgagcctggcccagtgttcagaggatcgaccacgggtttgtctgccactccccctgcctcattacctggctcactcactagtgtgaaagctgtacagagatccccaggacctcagcgagagaggaagtcgtcttcctcctcagaagacaggaatcgaatgaaaactcttggtagacgggattcaagtgatgattgggagattcctgatgggcagatcaccgtgggacagagaattggatctggatcatttggaaccgtctacaagggaaaatggcacggtgatgtggcagtaaaaatgttgaatgtgacagcacctacacctcagcagttacaggccttcaaaaatgaagtaggagtactcaggaaaacacgacatgtgaatatcctacttttcatgggctattccacaaagccacagctggctattgttacccagtggtgtgagggctccagtttatatcaccatctccacatcattgagaccaaattcgagatgatcaaacttatagatattgcacggcagactgcacagggcatggattacttacacgccaagtcaatcatccacagagacctcaagagtaataatatatttcttcatgaagacctcacagtaaaaataggtgattttggtctagccacagtgaaatctcgatggagtgggtcccatcagtttgaacaattgtctggatccattttgtggatggcaccagaagtaatcagaatgcaagacaaaaacccatatagctttcagtcagatgtatatgcatttgggattgttctgtatgaattgatgactgggcagttaccttactcaaacatcaacaacagggaccagatcatttttatggtgggacgtggctacctgtctccagacctcagtaaggtacggagtaactgtccgaaagccatgaagagattaatggcagagtgcctcaaaaagaaaagagatgagagaccactctttccccaaattctcgcctccattgagctgctggcccgctcattgccaaaaatccaccgcagtgcatcagaaccctccttgaatcgggctggtttccagacagaggattttagtctatatgcttgtgcttctccaaaaacacccatccaggcagggggatatggagaatttgcagccttcaagtag

SEQ ID NO: 55 - protein, 743 aa, Oryctolagus cuniculus
MGNVWNIKQMIKLTQEHIEALLDKFGGEHNPPSIYLEAYEEYTSKLDALQQREQQLLESLVFQNPTDVSRSNPKSPQKPIVRVFLPNKQRTVVPARCGVTVRDSLKKALMMRGLIPECCAVYRIQDGEKKPIGWDTDISWLTGEELHVEVLENVPLTTHNFVRKTFFTLAFCDFCRKLLFQGFRCQTCGYKFHQRCSTEVPLMCVNYDQLDLLFVSKFFEHHPVPQEEASLAETALTSGSSPSAPPSDSIGHQILTSPSPSKSIPIPQSFRPADEDHRNQFGQRDRSSSAPNVHINTIEPVNIDEKFPEVELQDQRDLIRDQGFRGDGAPLNQLMRCLRKYQSRTPSPLLPSVPSDIVFDFEPGPVFRGSTTGLSATPPASLPGSLTSVKAVQRSPGPQRERKSSSSSEDRNRMKTLGRRDSSDDWEIPDGQITVGQRIGSGSFGTVYKGKWHGDVAVKMLNVTAPTPQQLQAFKNEVGVLRKTRHVNILLFMGYSTKPQLAIVTQWCEGSSLYHHLHIIETKFEMIKLIDIARQTAQGMDYLHAKSIIHRDLKSNNIFLHEDLTVKIGDFGLATVKSRWSGSHQFEQLSGSILWMAPEVIRMQDKNPYSFQSDVYAFGIVLYELMTGQLPYSNINNRDQIIFMVGRGYLSPDLSKVRSNCPKAMKRLMAECLKKKRDERPLFPQILASIELLARSLPKIHRSASEPSLNRAGFQTEDFSLYACASPKTPIQAGGYGEFAAFK

SEQ ID NO: 56 - DNA, 2186 bp, Cavia porcellus
atggcggcgctcagcggcggcggtggcgcggagcagggccaggctctgttcaacggggacatggagctcgaggccggcgccggcgccgcagcctcttcggctgcagaccctgccattcccgaggaggtatggaatatcaaacaaatgattaagttgacgcaggaacacatagaggccctattggacaaatttggtggagagcataatccaccatcaatatacctggaggcctatgaagaatacaccagcaaactagatgccctccaacaaagagaacagcagttactggaatccctcgggaatggaactgatttttctgtttctagctctgcatcactggacaccgttacatcttcttcttcttctagcctttcagtactaccttcatctctttcagtttttcaaaatcctacagatgtgtcacggagcaaccccaaatcaccacaaaaacctattgttagagtcttcctgcccaacaaacagaggacagtggtacctgcaaggtgtggagttacagtccgagacagtctgaagaaagcactcatgatgagaggtcttatcccagagtgctgtgctgtgtacagaattcaggatggagaaaagaaaccaattggctgggacactgacatttcctggcttactggggaagaattacatgtagaagtattggagaatgttccacttacaacacacaattttgtatgtatctttatattttttttgctgtttgtctccaagttctttgaacaccacccaataccacaggaggaggcttccttagcagagaccacccttacatctggatcatccccttctgcacccccctcagagtccattgggcccccaattctcaccagcccatctccttcaaaatccattccaattccacagcctttccggccaggagaggaagatcatcgaaatcaatttgggcagcgagaccggtcctcatctgctcccaatgtgcatataaacacaatagaacctgtcaatattgatgatttgattagagaccaagggtttcgtagtgatggaggatcaactacaggtttgtctgccaccccacctgcctcattacctggctcactcactaatgtgaaagccttacagaaatctccaggacctcagcgagaaaggaagtcatcttcatcctcagaagacagaaatcgaatgaaaacgcttggtagacgggactcaagtgatgattgggagattcctgatgggcagattacagtgggacaaagaattggatctgggtcatttggaacagtctacaaggggaagtggcatggtgacgtggcagtgaaaatgttgaatgtgacagcacccacacctcaacagttacaggccttcaaaaatgaagtaggagtactcaggaaaacacgacatgtgaatatcctactcttcatgggctattccacaaagccacagctagctattgttacccagtggtgtgagggctccagcttataccaccatctccacatcatcgagaccaaatttgagatgatcaaacttatagatattgcacgacagactgcccagggcatggattacttacacgccaagtcaatcatccacagagacctcaagagtaataatatatttcttcacgaagacctcacggttaaaataggtgattttggtctagccacagtgaaatctcgatggagtgggtcccatcagtttgaacagttgtctggatccattttgtggatggcaccagaagtaatcagaatgcgagataaaaacccatacagttttcagtccgatgtatatgcatttgggattgttctatatgaattgatgactgggcagttaccctattcaaatatcaacaacagggaccagataatttttatggtgggacgaggatatctatctccagatctcagcaaggtacggagtaactgtccaaaagccatgaagaggttaatggcggagtgcctcaaaaagaaaagagatgagagaccactctttccccaaattctcgcctctattgagctgctggcccgctcattgccaaaaattcaccgcagtgcatcagaaccctccttgaatcgggctggtttccaaacagaggattttagtctctatgcttgtgcttctccaaaaacacccatccaggcagggggatatggtgcgtttcctgtccactgatgcaaattaaatgagtgagaaataaa

SEQ ID NO: 57 - protein, 719 aa, Cavia porcellus
MAALSGGGGAEQGQALFNGDMELEAGAGAAASSAADPAIPEEVWNIKQMIKLTQEHIEALLDKFGGEHNPPSIYLEAYEEYTSKLDALQQREQQLLESLGNGTDFSVSSSASLDTVTSSSSSSLSVLPSSLSVFQNPTDVSRSNPKSPQKPIVRVFLPNKQRTVVPARCGVTVRDSLKKALMMRGLIPECCAVYRIQDGEKKPIGWDTDISWLTGEELHVEVLENVPLTTHNFVCIFIFFLLFVSKFFEHHPIPQEEASLAETTLTSGSSPSAPPSESIGPPILTSPSPSKSIPIPQPFRPGEEDHRNQFGQRDRSSSAPNVHINTIEPVNIDDLIRDQGFRSDGGSTTGLSATPPASLPGSLTNVKALQKSPGPQRERKSSSSSEDRNRMKTLGRRDSSDDWEIPDGQITVGQRIGSGSFGTVYKGKWHGDVAVKMLNVTAPTPQQLQAFKNEVGVLRKTRHVNILLFMGYSTKPQLAIVTQWCEGSSLYHHLHIIETKFEMIKLIDIARQTAQGMDYLHAKSIIHRDLKSNNIFLHEDLTVKIGDFGLATVKSRWSGSHQFEQLSGSILWMAPEVIRMRDKNPYSFQSDVYAFGIVLYELMTGQLPYSNINNRDQIIFMVGRGYLSPDLSKVRSNCPKAMKRLMAECLKKKRDERPLFPQILASIELLARSLPKIHRSASEPSLNRAGFQTEDFSLYACASPKTPIQAGGYGAFPVH

SEQ ID NO: 58 - DNA, 3229 bp, Canis lupus familiaris
gtaatgctggattttcatggaataagtttgacctgtgctgcagtggcctccagcaaggtacccgcaagatgtggagttacagtccgggacagtctaaagaaagctctgatgatgagaggtctaatcccagagtgctgtgctgtttacagaattcaggatggagagaagaaaccgattggctgggacactgatatttcctggctcactggagaggaattgcatgtagaagtgttggaaaatgttccgcttaccacacacaactttgtacggaaaacttttttcaccttagcattttgtgacttttgtcgaaagctgcttttccagggttttcgctgtcaaacatgtggttataaatttcaccagcgttgtagtacagaggttccactgatgtgtgttaattatgaccaacttgatttgctgtttgtctccaagttctttgaacaccacccaataccacaggaggaggcctccatagcagagactgcccttacgtctggatcatccccttctgctcccccctccgattctcctgggcccccaattctgaccagtccgtctccttcaaaatccattccaattccacagcctttccgaccagcagatgaagatcatcgaaatcagtttggacaacgagaccggtcctcatcagctccaaatgtgcatataaacacaatagaacccgtcaacattgatgacttgattagagaccaagggtttcgtagtgatggaggatcaaccacaggtttgtctgccaccccccctgcctcattgcctggctcactcactaatgtaaaagcattacagaaatctccaggacctcagcgggaaagaaaatcatcttcatcctcagaagataggaatcgaatgaaaacacttggtagacgggattcaagtgatgattgggagatacctgatgggcagatcacagtgggacagagaattggatccgggtcatttgggacagtctacaagggaaagtggcatggtgacgtggcagtgaaaatgttgaatgtgacagcacccacacctcagcagttacaggccttcaaaaatgaagtaggagtactcaggaaaactcgacatgtgaatatcctactctttatgggctattcaacaaagccccaactggctattgttacccagtggtgtgagggctccagcttatatcaccatctccacatcattgagaccaaatttgagatgataaagcttatagatattgcacggcagactgcacagggcatggattacttacacgccaagtcaatcatccacagagacctcaagagtaataatatttttcttcatgaagacctcacagtaaaaataggtgattttggtctagccacagtgaaatctcgatggagtgggtcccatcagtttgaacagttgtctggatccattttgtggatggcaccagaagtgatccgaatgcaagacaaaaacccatatagcttccagtcagatgtatacgcatttgggattgttctatatgaattgatgacagggcagttaccttattcaaacatcaacaacagggaccagataatttttatggtgggacgaggatatctttctccagatctcagtaaggtacggagtaactgtccaaaagccatgaagagattgatggcagagtgcctaaaaaagaaaagagatgagaggccactctttccccaaattctcgcctctattgagctgctggcccgctcattgccaaaaattcaccgcagtgcatcagaaccctccttgaatcgggctggcttccaaacagaggattttagtctctatgcttgcgcttctccaaaaacacccatccaggcagggggatacggagaatttgcagccttcaagtagccacaccatcatggcaacaactactcttatttcttaagtcttgtgttcgtacaatttgttaacatcaaaacacagttctgttcctcaaatctttttttaaagatacagaattttcaatgcataagctggtgtggaacagaatggaatttcccatccaacaaaagagggaagaatgttttaggaaccagaattctctgctgccagtgtttcttcttcaacacaaataccacgtgcatacaagtctgcccactcccaggaaggaagaggagagcctgagttctgaccttttgatggtcaggcatgatggaaagaaactgctgctacagcttgggagattggctgtggagagcctgcccgtcagctctgcccttctaaccgccagatgagtgtgtggctggtcacctgacagggcagctgcaatcgccaagcatcgttctctttcctgtcctgggattttgtcgtggagctctttccccctagtcaccaccggttcatttctgagggatggaacaaaaatgcagcatggcctttctgtgtggtgcatgtccggtctttgacaaatttttatcaagtgaagctcttgtatttaaatggagaatgagaggcgagggggggggatcacgttttggtgtaggggcaaagggaatgctgcatctttttcctgacccactgggtttctggcctttgtttccttgctcactgagggtgtctgcctataaccacgcaggctggaaagtgctggcacacattgccttctcttctcactgggtccagcaatgaagacaagtgttggggatttttttttttgccctccacaatgtagcaagttctcaggaaaatacagttaatatcttcctcctaagctcttccagtcatcaagtacttatgtggctactttgtccagggcacaaaatgccatggcggtatccaattaaaagcctacaaaactgcttgataacagttttgaatgtgtgagacatttatgtaatttaaatgtaaggtacaagttttaatttctgagtttctctattatatttttattaaaaagaaaataattttcagatttaattgaattggaataaaataatacttcccaccagaattatatatcctggaaaattgtatttttgttatataaacaacttttaaagaaagatcattatccttttctctacctaaatatggggagtcttagcataatgacagatatttataatttttaaattaatggtacttgctggatccacactaacatctttgctaatatctcatgttttcctccaacttactcctacactacatcctccatcctctttccagtcttttatctagaatatgcaacctaaaataaaaatggtggtgtctccattca

SEQ ID NO: 59 - protein, 617 aa, Canis lupus familiaris
MLDFHGISLTCAAVASSKVPARCGVTVRDSLKKALMMRGLIPECCAVYRIQDGEKKPIGWDTDISWLTGEELHVEVLENVPLTTHNFVRKTFFTLAFCDFCRKLLFQGFRCQTCGYKFHQRCSTEVPLMCVNYDQLDLLFVSKFFEHHPIPQEEASIAETALTSGSSPSAPPSDSPGPPILTSPSPSKSIPIPQPFRPADEDHRNQFGQRDRSSSAPNVHINTIEPVNIDDLIRDQGFRSDGGSTTGLSATPPASLPGSLTNVKALQKSPGPQRERKSSSSSEDRNRMKTLGRRDSSDDWEIPDGQITVGQRIGSGSFGTVYKGKWHGDVAVKMLNVTAPTPQQLQAFKNEVGVLRKTRHVNILLFMGYSTKPQLAIVTQWCEGSSLYHHLHIIETKFEMIKLIDIARQTAQGMDYLHAKSIIHRDLKSNNIFLHEDLTVKIGDFGLATVKSRWSGSHQFEQLSGSILWMAPEVIRMQDKNPYSFQSDVYAFGIVLYELMTGQLPYSNINNRDQIIFMVGRGYLSPDLSKVRSNCPKAMKRLMAECLKKKRDERPLFPQILASIELLARSLPKIHRSASEPSLNRAGFQTEDFSLYACASPKTPIQAGGYGEFAAFK

SEQ ID NO: 60 - DNA, 1889 bp, Canis lupus familiaris
ggaatatcaaacaaatgattaagttgacacaggaacatatagaagccctattggacaagtttggtggggagcataatccaccatcaatatatctggaggcctatgaagaatacaccagcaaactagatgccctccaacagcgagaacaacagttattggaatccctggggaatggaactgatttttctgtttctagctctgcatcaacggacaccgttacatcttcttcctcttctagcctttcagtgctaccttcatctctttcagtttttcaaaatcccacagatatatcacggagcaatcccaagtcaccacaaaaacctatcgttagagtcttcctgcccaataaacagaggacggtggtacccgcaagatgtggagttacagtccgggacagtctaaagaaagctctgatgatgagaggtctaatcccagagtgctgtgctgtttacagaattcaggatggagagaagaaaccgattggctgggacactgatatttcctggctcactggagaggaattgcatgtagaagtgttggaaaatgttccgcttaccacacacaactttgtacggaaaacttttttcaccttagcattttgtgacttttgtcgaaagctgcttttccagggttttcgctgtcaaacatgtggttataaatttcaccagcgttgtagtacagaggttccactgatgtgtgttaattatgaccaacttgatttgctgtttgtctccaagttctttgaacaccacccaataccacaggaggaggcctccatagcagagactgcccttacgtctggatcatccccttctgctcccccctccgattctcctgggcccccaattctgaccagtccgtctccttcaaaatccattccaattccacagcctttccgaccagcagatgaagatcatcgaaatcagtttggacaacgagaccggtcctcatcagctccaaatgtgcatataaacacaatagaacccgtcaacattgatgacttgattagagaccaagggtttcgtagtgatggaggatcaaccacaggtttgtctgccaccccccctgcctcattgcctggctcactcactaatgtaaaagcattacagaaatctccaggacctcagcgggaaagaaaatcatcttcatcctcagaagataggaatcgaatgaaaacacttggtagacgggattcaagtgatgattgggagatacctgatgggcagatcacagtgggacagagaattggatccgggtcatttgggacagtctacaagggaaagtggcatggtgacgtggcagtgaaaatgttgaatgtgacagcacccacacctcagcagttacaggccttcaaaaatgaagtaggagtactcaggaaaactcgacatgtgaatatcctactctttatgggctattcaacaaagccccaactggctattgttacccagtggtgtgagggctccagcttatatcaccatctccacatcattgagaccaaatttgagatgataaagcttatagatattgcacggcagactgcacagggcatggattacttacacgccaagtcaatcatccacagagacctcaagagtaataatatttttcttcatgaagacctcacagtaaaaataggtgattttggtctagccacagtgaaatctcgatggagtgggtcccatcagtttgaacagttgtctggatccattttgtggatggcaccagaagtgatccgaatgcaagacaaaaacccatatagcttccagtcagatgtatacgcatttgggattgttctatatgaattgatgacagggcagttaccttattcaaacatcaacaacagggaccagctcagatcatgatcacggtgtcatgagatcaagccccac

SEQ ID NO: 61 - protein, 615 aa, Canis lupus familiaris
MIKLTQEHIEALLDKFGGEHNPPSIYLEAYEEYTSKLDALQQREQQLLESLGNGTDFSVSSSASTDTVTSSSSSSLSVLPSSLSVFQNPTDISRSNPKSPQKPIVRVFLPNKQRTVVPARCGVTVRDSLKKALMMRGLIPECCAVYRIQDGEKKPIGWDTDISWLTGEELHVEVLENVPLTTHNFVRKTFFTLAFCDFCRKLLFQGFRCQTCGYKFHQRCSTEVPLMCVNYDQLDLLFVSKFFEHHPIPQEEASIAETALTSGSSPSAPPSDSPGPPILTSPSPSKSIPIPQPFRPADEDHRNQFGQRDRSSSAPNVHINTIEPVNIDDLIRDQGFRSDGGSTTGLSATPPASLPGSLTNVKALQKSPGPQRERKSSSSSEDRNRMKTLGRRDSSDDWEIPDGQITVGQRIGSGSFGTVYKGKWHGDVAVKMLNVTAPTPQQLQAFKNEVGVLRKTRHVNILLFMGYSTKPQLAIVTQWCEGSSLYHHLHIIETKFEMIKLIDIARQTAQGMDYLHAKSIIHRDLKSNNIFLHEDLTVKIGDFGLATVKSRWSGSHQFEQLSGSILWMAPEVIRMQDKNPYSFQSDVYAFGIVLYELMTGQLPYSNINNRDQLRS

SEQ ID NO: 62 - DNA, 3521 bp, Felis catus
  misc_feature (630)..(649): n is a, c, g, or t
atgcctaacctcagtctctgccaccacggccaatttgctcatgtgcccactgtgtcggcactgggatattttgtgatttgccttggccattgtccactgtccttgacattgcctgaaggagaaccactgatgctaatgttgaaggtgacctttgcaggctctccactactcataccaaagatgcggccccctgataatcccagagccactgtctgcacatgggcaaaacaggctacattctgtgcagactggggagaaaggttccaagaacacagtgccatagttttgggcagagagtttcaacacagcatagtgtctatggcagtatctggatttggccgggggaagtgcccaagaggagacagtcaggctgtgtcctacggccaaggacctgcacttatttttgcatgcagtggtttagcacagggaagagaacgaagtaggaaatcggagccatggaaacggcagagcggaggaaacgtgcacgcgcgagggtgggcacgaaaggaaagaaccctccccagaagactgcgcgagggcgctcctaggattacgtcacgcaccccgcgaaaactgaaatgtactgtgtgtggtcttttaattgaactatcttccttatgtgcacttaannnnnnnnnnnnnnnnnnnngcggcggcggcggtggcgcggagcagggccaggctctgttcaacggggacatggagcccgaagccggcgccgcggcctcttcggctgcggaccctgccattcccgaggaggtgtggaatatcaaacaaatgattaagttgacacaggaacatatagaggccctattggacaaatttggtggggagcataatccaccatcaatatatctagaggcctatgaagaatacaccagcaagctagatgccctccaacagagagaacaacagttattggaatccctggggaatggaactgatttttctgtttctagctctgcatcaacagacaccgttacatcttcctcctcttctagcctttcagtgctaccttcatctctttcagtttttcaaaaccccacagatgtgtcacggagcaatcccaagtcaccacagaaacctatcgttagagtcttcctgcctaataaacagaggacagtggtacctgcaagatgtggagttacagtccgggacagtctaaagaaagctctgatgatgagaggtctaatccctgagtgctgtgctgtttacagaattcaggatggagagaagaaaccaattggctgggacactgatatctcctggctcaccggagaggaattgcatgtagaagtgttggaaaatgttccacttacaactcacaactttgtatgtacggaaaacgttttcaccttagcattttgtgacttttgtcgaaagctgcttttccaaggttttcgctgtcaaacgtgtggttataaatttcaccagcgttgtagtacagaggttccactgatgtgtgttaattatgaccaacttgatttgctgtttgtctccaagttctttgaacaccacccaataccacaggaggaggcctccatagcagagactgccctaacgtctggatcgtccccttctgcccccccctccgattctactgggccccaaattctcaccagtccgtctccttcaaaatccattccaattccacagcctttccgaccagcagatgaagatcatcgaaatcaatttggacagcgagaccggtcctcatcagctccaaatgtgcatataaatacaatagaacctgtcaatattgatgacttgattagagaccaggggtttcgtagtgatggaggatcaaccacaggcttgtctgccaccccccctgcctcattgccgggctctctcactaatgtaaaagcattacagaaatctccagggcctcagcgggaaaggaaatcttcttcatcctcagaagataggaatcgaatgaaaacacttggtagaagggattcaagtgatgattgggagattcctgatgggcagatcacagtgggacagagaattggatccgggtcatttgggacagtctacaagggaaagtggcatggtgatgtggcagtgaaaatgttgaatgtgacagcacccacacctcagcagttacaggccttcaaaaatgaagtaggagtactcaggaaaactcggcatgtgaacatcctgctcttcatgggctattcaacaaagccccagctggctattgtcacccagtggtgtgagggctccagcttataccaccatctccacatcatcgagaccaaattcgagatgatcaagctgatagatattgctcggcagactgcgcagggcatggattacttacacgccaagtcaatcatccacagagacctcaagagtaataatatttttcttcacgaagacctcacagtaaaaataggtgattttggtctagccacagtgaaatctcgatggagtgggtcccatcagtttgaacagttgtctggatccattttgtggatggcaccagaagtaattcgaatgcaagataaaaacccatatagctttcagtcagatgtatatgcatttgggattgttctatatgaattgatgactggacagttaccttattcaaacatcaacaacagggaccagataatttttatggtgggacgaggatatctttctccagatctcagtaaggtacgaagtaactgtccaaaagccatgaagagattgatggcagagtgcctaaaaaagaaaagagatgagaggccactgtttccccaaattcttgcctctattgagctgctggcccgctcattgccaaaaattcaccgcagtgcatcagaaccctccttgaatcgggctggcttccagacagaggattttagtctctatgcttgtgcttctccaaaaacacccatccaggcagggggatatggtgcgtttcccgtccactgagataagttagatgagtgcgcgagtgcagggggccggggccaaggaggtggaaatgtgcgtgcttctgtactaagttggatagcatcttcttttttaaaaaaagatgaaccaaagaatgtgtatgtttttaaagactagatataattatttcctgatctaaaatgtatacttagctttggattttcaatatccaagggttttcaaaatgcacagacattgctgaacatttgcagtacctcttctggaggctttacttcctgttacaaattggttttgtttactggcttatcctaattattaaacttcaattaaacttttctcctgcaccttttgttatgagctatcacatgtcccttagggactcgcaagagcagtactgcccccgtgtacgggcttgcaggtagaaaggggatgacgggttttaacacctgtgtgaggcaaggcagtccgaacagatctcatttaggaagccacgagagttgaataagttatttttattcttagtattttttctgtaactactttttattataacttggaaaatatggatgtcctttatacaccttagcaatagactgaatttctttttataaatt

SEQ ID NO: 63 - protein, 974 aa, Felis catus
  misc_feature (210)..(217): Xaa can be any naturally occurring amino acid
MPNLSLCHHGQFAHVPTVSALGYFVICLGHCPLSLTLPEGEPLMLMLKVTFAGSPLLIPKMRPPDNPRATVCTWAKQATFCADWGERFQEHSAIVLGREFQHSIVSMAVSGFGRGKCPRGDSQAVSYGQGPALIFACSGLAQGRERSRKSEPWKRQSGGNVHARGWARKERTLPRRLREGAPRITSRTPRKLKCTVCGLLIELSSLCALXXXXXXXXGGGGGAEQGQALFNGDMEPEAGAAASSAADPAIPEEVWNIKQMIKLTQEHIEALLDKFGGEHNPPSIYLEAYEEYTSKLDALQQREQQLLESLGNGTDFSVSSSASTDTVTSSSSSSLSVLPSSLSVFQNPTDVSRSNPKSPQKPIVRVFLPNKQRTVVPARCGVTVRDSLKKALMMRGLIPECCAVYRIQDGEKKPIGWDTDISWLTGEELHVEVLENVPLTTHNFVCTENVFTLAFCDFCRKLLFQGFRCQTCGYKFHQRCSTEVPLMCVNYDQLDLLFVSKFFEHHPIPQEEASIAETALTSGSSPSAPPSDSTGPQILTSPSPSKSIPIPQPFRPADEDHRNQFGQRDRSSSAPNVHINTIEPVNIDDLIRDQGFRSDGGSTTGLSATPPASLPGSLTNVKALQKSPGPQRERKSSSSSEDRNRMKTLGRRDSSDDWEIPDGQITVGQRIGSGSFGTVYKGKWHGDVAVKMLNVTAPTPQQLQAFKNEVGVLRKTRHVNILLFMGYSTKPQLAIVTQWCEGSSLYHHLHIIETKFEMIKLIDIARQTAQGMDYLHAKSIIHRDLKSNNIFLHEDLTVKIGDFGLATVKSRWSGSHQFEQLSGSILWMAPEVIRMQDKNPYSFQSDVYAFGIVLYELMTGQLPYSNINNRDQIIFMVGRGYLSPDLSKVRSNCPKAMKRLMAECLKKKRDERPLFPQILASIELLARSLPKIHRSASEPSLNRAGFQTEDFSLYACASPKTPIQAGGYGAFPVH

SEQ ID NO: 64 - DNA, 3853 bp, Bos taurus
ctcagctgcgccgggtctcacaagacggttcccgaggtggcccaggcgccgtcccaccgccgacgccgcccgggccgcccgggccgtccctccccgctgccccccgtcctccgcctccgcctccccccgccctcagcctcccttccccctccccgcccagcagcggtcgctcgggcccggctctcggttataagatggcggcgctgagtggcggcggcggcggcggcggcggtggcgcggagcagggccaggctctgttcaacggggacatggagcccgaggccggcgccgcggcctcttcggctgcggaccccgccattcccgaggaggtgtggaatatcaaacaaatgattaagttgacacaggagcatatagaggccctattggacaaatttggtggggagcataatccaccatcaatatatctggaggcctatgaagaatacaccagcaagctagatgccctccaacaaagagaacaacagttattggaatccctggggaatggaactgatttttctgtttctagctctgcatcaacggacaccgttacatcttcttcctcttctagcctttcagtgctgccttcatctctttcagtttttcaaaatcccacagatgtgtcacggagcaaccccaagtcaccacaaaaacctatcgttagagtcttcctgcccaataaacagaggacagtggtacctgcacggtgtggagtcacagtccgggacagcctgaagaaggcactgatgatgagaggtctaatcccagagtgctgtgctgtttacagaattcaggatggggagaagaaaccaattggctgggacactgatatttcctggcttactggagaggagttgcatgtagaagtgttggagaatgttccacttacaacacacaactttgtacggaaaacttttttcaccttagcattttgtgacttctgtagaaagctgcttttccagggattccgctgtcaaacatgtggttataaatttcaccagcgttgtagtacagaggttccactgatgtgtgttaattatgaccaactagatttgctgtttgtctccaagttctttgaacaccacccaataccacaggaggaggcctccttagcagagactacccttccatgtggctcatccccttctgcacccccctccgattctattgggcccccaattctcaccagtccatctccttcaaaatccattccaattccacagcctttccgaccagcagatgaagatcatcgaaatcagtttggacaacgagaccggtcctcatcagctccaaatgtgcatataaacacaatagaacccgtcaatattgatgacttgattagagaccaagggtttcgtagtgatggaggatcaaccacaggtttatccgccacaccccctgcctcattacctggctcactctctaatgtgaaagcattgcagaaatctccaggacctcagcgagaaagaaagtcctcttcatcctcagaagacaggaatcgaatgaaaacgcttggtagacgggattcaagtgacgattgggagattcctgatggacagatcacagtgggacaaagaattggatcagggtcatttgggacagtctacaagggaaagtggcatggtgatgtggcagtgaaaatgttgaatgtgacagcacccacacctcagcagttacaggccttcaaaaatgaagtaggagtactcaggaaaacgcgacatgtgaatatcctcctcttcatgggttattcaacaaagccacaactggctattgttacccagtggtgtgagggctccagtttatatcatcatctccacatcattgagaccaaattcgagatgatcaaacttatagatattgcacggcagactgcacagggcatggattacttacacgccaagtcaatcatccacagagacctcaagagtaataatatttttcttcatgaagacctcacagtaaaaataggtgattttggtctagccacagtgaaatctcgatggagtgggtcccatcagtttgaacagttgtctggatccattttgtggatggcaccagaagtaatcagaatgcaagataaaaacccatatagctttcagtcagatgtatatgcatttgggattgttctgtatgaattgatgaccggacagttaccttattcaaatatcaacaacagggaccagataatttttatggtgggacgaggatatctgtctccagatctcagtaaggtacggagtaactgtccaaaagccatgaagagattaatggcagagtgcctaaaaaagaaaagagatgaaagaccactctttccccaaattctcgcctctattgagctgctggcccgctcattgccaaaaattcaccgcagtgcatcagaaccctccttgaatcgggctggcttccaaacagaggattttagtctatatgcttgtgcttctccaaaaacacccattcaggcagggggatatggtacgtttcctgttcactgaaacaaaccgagtgagtgacagcatgtaggagggtagggacaaaagaaagtgaacaaatgtttgcttatatatttgttaaattgaataggattttctttttctttaaaggtgaacaagagaacatgtgtgtttttaaagtttggatatagttttcttcccagtctaaaacccatagttagcattacattttcaacatcgaatttttttttaattcatagacattgctgaaaatttataataccttttccagaggctttacttcccattccaagtttgttttgtttacttggttagtctaatcattaaactttaaactttccccacctaccttttgctgttagctatcccgcatccattaggggctccaagaacagcactgtctgcgtgtgtgtgttggcaggtgggaagctgatggtaagttaggctgtgttagtgaaggtaaactgaccaggtctaattaggagtcactagaattgaataagcttatttttattaatattttttcttataactatttctttttgtaataatttagaaaatataattgttctttattcccttacagcagtataaattattggtgcaggtaaccaaagatattactgaggagtggcatgtttgacatgagtgacatggtttaactttggatttttagttaatatttctttatatattaaggatgtcttacacattatagaagtcaaatttactgacaaaggtattgcctcctcttcctccccaaaaacacagcaaaattctctgggaactcgtagcattgttggttttcttttggatgactatggttgccaaacaaccaagtaattgattttttttaaattattattgctttagattatactcacctctcatgatgcctgttagcaatcacctttatccatgtgtcttgtaaaatatctttcctccttatattctttgcccaacaagagtctacttgttatgaatgagtactattttctttttttgattccccagtataattagtatgtttagtgctttctaggacttccactttcttatgttaaaaaaaaaaacaaactaatgtggcagtcagtatattcttactgtgaatcagagtctttactgggaatcaaagtgaaagaagcagctgttctgacttcagagtcagcctagggaccaaaaccagcctcttaaatacaccttcatttattcagtttggatttgtgatgattttcattatagctgacagttcaaggttattcagtggcacacagatagcatctgcataaatgcctttcttcttgaaaataaaggagaaaattgggaagactttacaccaatagtttagtctttaagtaccacagataacacacaccataaat

SEQ ID NO: 65 - protein, 765 aa, Bos taurus
MAALSGGGGGGGGGAEQGQALFNGDMEPEAGAAASSAADPAIPEEVWNIKQMIKLTQEHIEALLDKFGGEHNPPSIYLEAYEEYTSKLDALQQREQQLLESLGNGTDFSVSSSASTDTVTSSSSSSLSVLPSSLSVFQNPTDVSRSNPKSPQKPIVRVFLPNKQRTVVPARCGVTVRDSLKKALMMRGLIPECCAVYRIQDGEKKPIGWDTDISWLTGEELHVEVLENVPLTTHNFVRKTFFTLAFCDFCRKLLFQGFRCQTCGYKFHQRCSTEVPLMCVNYDQLDLLFVSKFFEHHPIPQEEASLAETTLPCGSSPSAPPSDSIGPPILTSPSPSKSIPIPQPFRPADEDHRNQFGQRDRSSSAPNVHINTIEPVNIDDLIRDQGFRSDGGSTTGLSATPPASLPGSLSNVKALQKSPGPQRERKSSSSSEDRNRMKTLGRRDSSDDWEIPDGQITVGQRIGSGSFGTVYKGKWHGDVAVKMLNVTAPTPQQLQAFKNEVGVLRKTRHVNILLFMGYSTKPQLAIVTQWCEGSSLYHHLHIIETKFEMIKLIDIARQTAQGMDYLHAKSIIHRDLKSNNIFLHEDLTVKIGDFGLATVKSRWSGSHQFEQLSGSILWMAPEVIRMQDKNPYSFQSDVYAFGIVLYELMTGQLPYSNINNRDQIIFMVGRGYLSPDLSKVRSNCPKAMKRLMAECLKKKRDERPLFPQILASIELLARSLPKIHRSASEPSLNRAGFQTEDFSLYACASPKTPIQAGGYGTFPVH

SEQ ID NO: 66 - DNA, 4936 bp, Bos taurus
ctcagctgcgccgggtctcacaagacggttcccgaggtggcccaggcgccgtcccaccgccgacgccgcccgggccgcccgggccgtccctccccgctgccccccgtcctccgcctccgcctccccccgccctcagcctcccttccccctccccgcccagcagcggtcgctcgggcccggctctcggttataagatggcggcgctgagtggcggcggcggcggcggcggcggtggcgcggagcagggccaggctctgttcaacggggacatggagcccgaggccggcgccgcggcctcttcggctgcggaccccgccattcccgaggaggtgtggaatatcaaacaaatgattaagttgacacaggagcatatagaggccctattggacaaatttggtggggagcataatccaccatcaatatatctggaggcctatgaagaatacaccagcaagctagatgccctccaacaaagagaacaacagttattggaatccctggggaatggaactgatttttctgtttctagctctgcatcaacggacaccgttacatcttcttcctcttctagcctttcagtgctgccttcatctctttcagtttttcaaaatcccacagatgtgtcacggagcaaccccaagtcaccacaaaaacctatcgttagagtcttcctgcccaataaacagaggacagtggtacctgcacggtgtggagtcacagtccgggacagcctgaagaaggcactgatgatgagaggtctaatcccagagtgctgtgctgtttacagaattcaggatggggagaagaaaccaattggctgggacactgatatttcctggcttactggagaggagttgcatgtagaagtgttggagaatgttccacttacaacacacaactttgtacggaaaacttttttcaccttagcattttgtgacttctgtagaaagctgcttttccagggattccgctgtcaaacatgtggttataaatttcaccagcgttgtagtacagaggttccactgatgtgtgttaattatgaccaactagatttgctgtttgtctccaagttctttgaacaccacccaataccacaggaggaggcctccttagcagagactacccttccatgtggctcatccccttctgcacccccctccgattctattgggcccccaattctcaccagtccatctccttcaaaatccattccaattccacagcctttccgaccagcagatgaagatcatcgaaatcagtttggacaacgagaccggtcctcatcagctccaaatgtgcatataaacacaatagaacccgtcaatattgatgacttgattagagaccaagggtttcgtagtgatggaggatcaaccacaggtttatccgccacaccccctgcctcattacctggctcactctctaatgtgaaagcattgcagaaatctccaggacctcagcgagaaagaaagtcctcttcatcctcagaagacaggaatcgaatgaaaacgcttggtagacgggattcaagtgacgattgggagattcctgatggacagatcacagtgggacaaagaattggatcagggtcatttgggacagtctacaagggaaagtggcatggtgatgtggcagtgaaaatgttgaatgtgacagcacccacacctcagcagttacaggccttcaaaaatgaagtaggagtactcaggaaaacgcgacatgtgaatatcctcctcttcatgggttattcaacaaagccacaactggctattgttacccagtggtgtgagggctccagtttatatcatcatctccacatcattgagaccaaattcgagatgatcaaacttatagatattgcacggcagactgcacagggcatggattacttacacgccaagtcaatcatccacagagacctcaagagtaataatatttttcttcatgaagacctcacagtaaaaataggtgattttggtctagccacagtgaaatctcgatggagtgggtcccatcagtttgaacagttgtctggatccattttgtggatggcaccagaagtaatcagaatgcaagataaaaacccatatagctttcagtcagatgtatatgcatttgggattgttctgtatgaattgatgaccggacagttaccttattcaaatatcaacaacagggaccagataatttttatggtgggacgaggatatctgtctccagatctcagtaaggtacggagtaactgtccaaaagccatgaagagattaatggcagagtgcctaaaaaagaaaagagatgaaagaccactctttccccaagtaggaaagactctcctaagcaagagacaaaattcagaagttatcagggaaaaagataagcagattctcgcctctattgagctgctggcccgctcattgccaaaaattcaccgcagtgcatcagaaccctccttgaatcgggctggcttccaaacagaggattttagtctatatgcttgtgcttctccaaaaacacccattcaggcagggggatatgaagcagatttggctcttacatcaaataaaaatagagtagaagttgggatttagagatttcctgacatgcaagaaggaataagcaagaaaaaaaggtttgttttccccaaatcatatctattgtcttttacttctattttttcttaaattttttgtgatttcagagacatgtagagttttattgatacctaaactatgagttcttttttttttttttttttcattattttgatttttttggccaagaggcatatgggatcttagcttgagaaagcaacaattttcttgatgtcattttgggtgagggcacatattgctgtgaacagtgtggtgatagccaccagggaccaaactcacacccgctgcattgaaaggtgaagtcttaaacactggaccagcagagaaattcctactctatgagttctttttgtcatcccctccccgcaccctccacccccaacctaaagtctgatgatgaaatcaacaactattccattagaagcagtagattctggtagcatgatctttagtttgttagtaagattttgtgctttgtggggttgtgtcgttttaaggctaatatttaagtttgtcaaatagaatgctgttcagattgtaaaaatgagtaataaacatctgaagttttttttaagttatttttaacatggtatatacagttgagcttagagtttatcattttctgatattctcttacttagtagatgaattctagccattttttataaagatttctgttaagcaaatcctgttttcacatgggcttcctttaagggattttagattctgctggatatggtgactgctcataagactgttgaaaattacttttaagatgtattagaatacttctgaaaaaaaatagcaaccttaaaaccataagcaaaagtagtaagggtgtttatacatttctagagtccctgtttaggtaatagcctcctatgattgtactttaaatgttttgctctccaaggttttagtaacttggctttttttctaatcagtgccaaactcccccagtttttttaactttaaatatgaggtaataaatcttttacccttccttgatcttttgacttataataccttggtcagttgtttcttaaaaggaatccttaaatggaaagagacaatatcactgtctgcagttctgattagtagttttattcagaatggaaaaacagattattcatttttgaaaattgttcaggggtatgttcattgttaggaccttggactttggagtcagtgcctagctatgcattccaggtctgccattttctggctgtgaaattttggacaagttacttaaccactttaaaccccagctttaagaagtaaattaaccccagtaaattaagaagtaatagcagccacttcgtagagttgttatgaggctcagatgcagtgcaaatgtgtataaagtattcagggagtcacctggtatactataatagacactagaatagttgccaatattatcagcatacaatctgaggattctgtcagccaatcattagcaatctgttgtttgttgggacatgccagtgttctccagttgaaatcagtagcaatctaaaaatggatagattattcctcatttaaatagtgtgttcatataagtgattgcttggatccttatcagaagttgctgttactgaaaaatgataaggctgactaaattgtgatagttgtcagttactaaccaactcccagaaatgaataagaggaacctatctctagttcctagtagaaggtatggacaaaatagtaggtgaaaaataatgtcttgaacccccaaattaagtaagctttaaagagtacaatacctcaaagggtctttgcggtttaaaatttgtatgctgagaatgatgttcattgacatgtgcctatatgtaattttttgatagtttaaaaggtgaaatgaactacagatgggagaggtctgaattttcttgccttcagtcaaatgtgtaatgtggacatattatttgacctgtgaattttatcttttaaaaaagattaattcctgcttcttccttcctaatagttgcattataataatgaaaatgagttgataatttggggggaaagtattctacaaatcaaccttattattttaccattggtttctgagaaattttgttcatttgaaccgtttatagcttgattagaatcatagcatgtaaaacccaactgagggattatctgcagacttaatgtagtattatgtaagttgtcttctttcatttcgaccttttttgcttttgttgttgctagatctgtagtatgtagctagtcacctttcagcgaggtttcagcgaggcttttctgtgtctctaggttatttgagataacttttttaaaattagctcttgtcctcc

SEQ ID NO: 67 - protein, 797 aa, Bos taurus
MAALSGGGGGGGGGAEQGQALFNGDMEPEAGAAASSAADPAIPEEVWNIKQMIKLTQEHIEALLDKFGGEHNPPSIYLEAYEEYTSKLDALQQREQQLLESLGNGTDFSVSSSASTDTVTSSSSSSLSVLPSSLSVFQNPTDVSRSNPKSPQKPIVRVFLPNKQRTVVPARCGVTVRDSLKKALMMRGLIPECCAVYRIQDGEKKPIGWDTDISWLTGEELHVEVLENVPLTTHNFVRKTFFTLAFCDFCRKLLFQGFRCQTCGYKFHQRCSTEVPLMCVNYDQLDLLFVSKFFEHHPIPQEEASLAETTLPCGSSPSAPPSDSIGPPILTSPSPSKSIPIPQPFRPADEDHRNQFGQRDRSSSAPNVHINTIEPVNIDDLIRDQGFRSDGGSTTGLSATPPASLPGSLSNVKALQKSPGPQRERKSSSSSEDRNRMKTLGRRDSSDDWEIPDGQITVGQRIGSGSFGTVYKGKWHGDVAVKMLNVTAPTPQQLQAFKNEVGVLRKTRHVNILLFMGYSTKPQLAIVTQWCEGSSLYHHLHIIETKFEMIKLIDIARQTAQGMDYLHAKSIIHRDLKSNNIFLHEDLTVKIGDFGLATVKSRWSGSHQFEQLSGSILWMAPEVIRMQDKNPYSFQSDVYAFGIVLYELMTGQLPYSNINNRDQIIFMVGRGYLSPDLSKVRSNCPKAMKRLMAECLKKKRDERPLFPQVGKTLLSKRQNSEVIREKDKQILASIELLARSLPKIHRSASEPSLNRAGFQTEDFSLYACASPKTPIQAGGYEADLALTSNKNRVEVGI

SEQ ID NO: 68 - DNA, 4154 bp, Bos taurus
ctcagctgcgccgggtctcacaagacggttcccgaggtggcccaggcgccgtcccaccgccgacgccgcccgggccgcccgggccgtccctccccgctgccccccgtcctccgcctccgcctccccccgccctcagcctcccttccccctccccgcccagcagcggtcgctcgggcccggctctcggttataagatggcggcgctgagtggcggcggcggcggcggcggcggtggcgcggagcagggccaggctctgttcaacggggacatggagcccgaggccggcgccgcggcctcttcggctgcggaccccgccattcccgaggaggtgtggaatatcaaacaaatgattaagttgacacaggagcatatagaggccctattggacaaatttggtggggagcataatccaccatcaatatatctggaggcctatgaagaatacaccagcaagctagatgccctccaacaaagagaacaacagttattggaatccctggggaatggaactgatttttctgtttctagctctgcatcaacggacaccgttacatcttcttcctcttctagcctttcagtgctgccttcatctctttcagtttttcaaaatcccacagatgtgtcacggagcaaccccaagtcaccacaaaaacctatcgttagagtcttcctgcccaataaacagaggacagtggtacctgcacggtgtggagtcacagtccgggacagcctgaagaaggcactgatgatgagaggtctaatcccagagtgctgtgctgtttacagaattcaggatggggagaagaaaccaattggctgggacactgatatttcctggcttactggagaggagttgcatgtagaagtgttggagaatgttccacttacaacacacaactttgtacggaaaacttttttcaccttagcattttgtgacttctgtagaaagctgcttttccagggattccgctgtcaaacatgtggttataaatttcaccagcgttgtagtacagaggttccactgatgtgtgttaattatgaccaactagatttgctgtttgtctccaagttctttgaacaccacccaataccacaggaggaggcctccttagcagagactacccttccatgtggctcatccccttctgcacccccctccgattctattgggcccccaattctcaccagtccatctccttcaaaatccattccaattccacagcctttccgaccagcagatgaagatcatcgaaatcagtttggacaacgagaccggtcctcatcagctccaaatgtgcatataaacacaatagaacccgtcaatattgatgacttgattagagaccaagggtttcgtagtgatggaggatcaaccacaggtttatccgccacaccccctgcctcattacctggctcactctctaatgtgaaagcattgcagaaatctccaggacctcagcgagaaagaaagtcctcttcatcctcagaagacaggaatcgaatgaaaacgcttggtagacgggattcaagtgacgattgggagattcctgatggacagatcacagtgggacaaagaattggatcagggtcatttgggacagtctacaagggaaagtggcatggtgatgtggcagtgaaaatgttgaatgtgacagcacccacacctcagcagttacaggccttcaaaaatgaagtaggagtactcaggaaaacgcgacatgtgaatatcctcctcttcatgggttattcaacaaagccacaactggctattgttacccagtggtgtgagggctccagtttatatcatcatctccacatcattgagaccaaattcgagatgatcaaacttatagatattgcacggcagactgcacagggcatggattacttacacgccaagtcaatcatccacagagacctcaagagtaataatatttttcttcatgaagacctcacagtaaaaataggtgattttggtctagccacagtgaaatctcgatggagtgggtcccatcagtttgaacagttgtctggatccattttgtggatggcaccagaagtaatcagaatgcaagataaaaacccatatagctttcagtcagatgtatatgcatttgggattgttctgtatgaattgatgaccggacagttaccttattcaaatatcaacaacagggaccagataatttttatggtgggacgaggatatctgtctccagatctcagtaaggtacggagtaactgtccaaaagccatgaagagattaatggcagagtgcctaaaaaagaaaagagatgaaagaccactctttccccaagtaggaaagactctcctaagcaagagacaaaattcagaagttatcagggaaaaagataagcagattctcgcctctattgagctgctggcccgctcattgccaaaaattcaccgcagtgcatcagaaccctccttgaatcgggctggcttccaaacagaggattttagtctatatgcttgtgcttctccaaaaacacccattcaggcagggggatatggctgagcacattgtccatcacccacaagtggctggttctcatcgcagaatctacgtagggaatcgggcgtgaaattcacttaagagatagagcagaggaagtgttctgtttacaggaatggagatgagagttatgagtaagttgcttagtcagttggctttgttttgaaaattattgtgttatatttgtgttaacctacttgtgttttgacagtatatgtcacataggaagaaacctcagactagcataataacaaagctcagactaggcacagatgtacacagaatggaccaaaatgggatgggggaaggtatgggaataagtctaggggtagggaaaaattgatgtgagggtgggaaataaactgtaattacctgaaataaaatgtaagagtgcaataagtgtgctttttattctaagctgtgaatgggttttttaaaaaaagcattccttcccaatgcatttgcctatgttccatagctgattaaaaccagctatataaacatatgcctttttattcatgttaattaccaatataaatggctaacctttacgtcttatttatcttcatgttatgttagtttacatacagggatgtgtgtgtgtgtgtatgctataaattttccctccttcgtttaaaaacgcgtttgttggatcctctctgtttccttaggccatgccacagctcatagtctcagcttggccttcctgtcacctgatctgaaggactatcacagtgacgtagctcgttcattggttgtacacactctaacccttttccttgctcagcaattactgtgtcttctaaaacaggagtgtacaaccatgagattgcaattaattgtttgacatatgtccctttgaattctatttattagttatgattgattgctctttggtttggaccaagaaaaacgaaatcccacctccccaccttttcacttatttcttactttgaggacaattctgtaagagagaggaaagggaactccttcatgttttaactgcagcaagttaatggccctggtttacaccaaacattatggtgattcacattcacattcctctcctctcttgctgccagaggtttgggttttgttcagttctgctcaagcactgaaaaagttttcatggagtctggagagtgcccagtgaaaagatggtttttaattgtccacagacctttctgttcctgctttgcaaaaattacaaaggagtaactatttttaaagcttatttttcaattcataaaaaagacatttattttcagtcagatgatgtctccttgtcccttaatcctcaatgtttgcttgaatcttttttttttttctgattttctcccatccccacttcttgatacttcttgagttctctttcctgctcaggtcctttcatttgtactttggagttttttctcatgtaaatttgtacaatggaaaatattgttcagtttggatagaacgcatggagaattaaataaaaaagatagctgaaattcagattgaaatttatttgtgtaaagttatttaaaaactctgtactatataaaaggcaaaaaaagttctatgtacttgatgtgaatatgcgaatactgctataataaagattgactgcatgga

SEQ ID NO: 69 - protein, 781 aa, Bos taurus
MAALSGGGGGGGGGAEQGQALFNGDMEPEAGAAASSAADPAIPEEVWNIKQMIKLTQEHIEALLDKFGGEHNPPSIYLEAYEEYTSKLDALQQREQQLLESLGNGTDFSVSSSASTDTVTSSSSSSLSVLPSSLSVFQNPTDVSRSNPKSPQKPIVRVFLPNKQRTVVPARCGVTVRDSLKKALMMRGLIPECCAVYRIQDGEKKPIGWDTDISWLTGEELHVEVLENVPLTTHNFVRKTFFTLAFCDFCRKLLFQGFRCQTCGYKFHQRCSTEVPLMCVNYDQLDLLFVSKFFEHHPIPQEEASLAETTLPCGSSPSAPPSDSIGPPILTSPSPSKSIPIPQPFRPADEDHRNQFGQRDRSSSAPNVHINTIEPVNIDDLIRDQGFRSDGGSTTGLSATPPASLPGSLSNVKALQKSPGPQRERKSSSSSEDRNRMKTLGRRDSSDDWEIPDGQITVGQRIGSGSFGTVYKGKWHGDVAVKMLNVTAPTPQQLQAFKNEVGVLRKTRHVNILLFMGYSTKPQLAIVTQWCEGSSLYHHLHIIETKFEMIKLIDIARQTAQGMDYLHAKSIIHRDLKSNNIFLHEDLTVKIGDFGLATVKSRWSGSHQFEQLSGSILWMAPEVIRMQDKNPYSFQSDVYAFGIVLYELMTGQLPYSNINNRDQIIFMVGRGYLSPDLSKVRSNCPKAMKRLMAECLKKKRDERPLFPQVGKTLLSKRQNSEVIREKDKQILASIELLARSLPKIHRSASEPSLNRAGFQTEDFSLYACASPKTPIQAGGYG

SEQ ID NO: 70 - DNA, 7914 bp, Bos taurus
ctcagctgcgccgggtctcacaagacggttcccgaggtggcccaggcgccgtcccaccgccgacgccgcccgggccgcccgggccgtccctccccgctgccccccgtcctccgcctccgcctccccccgccctcagcctcccttccccctccccgcccagcagcggtcgctcgggcccggctctcggttataagatggcggcgctgagtggcggcggcggcggcggcggcggtggcgcggagcagggccaggctctgttcaacggggacatggagcccgaggccggcgccgcggcctcttcggctgcggaccccgccattcccgaggaggtgtggaatatcaaacaaatgattaagttgacacaggagcatatagaggccctattggacaaatttggtggggagcataatccaccatcaatatatctggaggcctatgaagaatacaccagcaagctagatgccctccaacaaagagaacaacagttattggaatccctggggaatggaactgatttttctgtttctagctctgcatcaacggacaccgttacatcttcttcctcttctagcctttcagtgctgccttcatctctttcagtttttcaaaatcccacagatgtgtcacggagcaaccccaagtcaccacaaaaacctatcgttagagtcttcctgcccaataaacagaggacagtggtacctgcacggtgtggagtcacagtccgggacagcctgaagaaggcactgatgatgagaggtctaatcccagagtgctgtgctgtttacagaattcaggatggggagaagaaaccaattggctgggacactgatatttcctggcttactggagaggagttgcatgtagaagtgttggagaatgttccacttacaacacacaactttgtacggaaaacttttttcaccttagcattttgtgacttctgtagaaagctgcttttccagggattccgctgtcaaacatgtggttataaatttcaccagcgttgtagtacagaggttccactgatgtgtgttaattatgaccaactagatttgctgtttgtctccaagttctttgaacaccacccaataccacaggaggaggcctccttagcagagactacccttccatgtggctcatccccttctgcacccccctccgattctattgggcccccaattctcaccagtccatctccttcaaaatccattccaattccacagcctttccgaccagcagatgaagatcatcgaaatcagtttggacaacgagaccggtcctcatcagctccaaatgtgcatataaacacaatagaacccgtcaatattgatgacttgattagagaccaagggtttcgtagtgatggaggatcaaccacaggtttatccgccacaccccctgcctcattacctggctcactctctaatgtgaaagcattgcagaaatctccaggacctcagcgagaaagaaagtcctcttcatcctcagaagacaggaatcgaatgaaaacgcttggtagacgggattcaagtgacgattgggagattcctgatggacagatcacagtgggacaaagaattggatcagggtcatttgggacagtctacaagggaaagtggcatggtgatgtggcagtgaaaatgttgaatgtgacagcacccacacctcagcagttacaggccttcaaaaatgaagtaggagtactcaggaaaacgcgacatgtgaatatcctcctcttcatgggttattcaacaaagccacaactggctattgttacccagtggtgtgagggctccagtttatatcatcatctccacatcattgagaccaaattcgagatgatcaaacttatagatattgcacggcagactgcacagggcatggattacttacacgccaagtcaatcatccacagagacctcaagagtaataatatttttcttcatgaagacctcacagtaaaaataggtgattttggtctagccacagtgaaatctcgatggagtgggtcccatcagtttgaacagttgtctggatccattttgtggatggcaccagaagtaatcagaatgcaagataaaaacccatatagctttcagtcagatgtatatgcatttgggattgttctgtatgaattgatgaccggacagttaccttattcaaatatcaacaacagggaccagataatttttatggtgggacgaggatatctgtctccagatctcagtaaggtacggagtaactgtccaaaagccatgaagagattaatggcagagtgcctaaaaaagaaaagagatgaaagaccactctttccccaaattctcgcctctattgagctgctggcccgctcattgccaaaaattcaccgcagtgcatcagaaccctccttgaatcgggctggcttccaaacagaggattttagtctatatgcttgtgcttctccaaaaacacccattcaggcagggggatatggagaatttgcagccttcaagtagccacaccatcatgacagcatctactcttatttcttaagtcttgtgttcgtacaatttgttaacatcaaaacacagttctgttcctcaactctttttaaagttaaaatttttcagtgcataagctggtgtggaacagaaggaaatttcccatccaacaaaagagggaagaatgttttaggaaccagaattctctgctgccagtgtttcttcttcaacacaaatatcacaagtctgcccactcccaggaagaaagaggagagaccctgagttctgaccttttgatggtcaggcatgatggaaagaaactgctgctacagcttgggagatttgctctgggaagtctgccagtcaactttgcccttctaaccaccagatcaatatgtggctgatcatctgatggggcagttgcaatcaccaagccttgttctctttcctgttctgggattgtgttgtggaacccttttccctagccaccaccagttcatttctgagggatggaacaaaaatgcagcatgcccttcctgtgtggtgcatgttcagtccttgacaaatttttaccaaaatgaagctactttatttaaaaggagggtgagaggtgaggaggtcactttgggtgtggcggaaagggaatgctgcatctttttcctgggctgctggggctctggccttggcttgccagccggaagcgctggcacgcatcgccttcttttcccattgggtccagcaatgaagacgagtgtttggggttttttttttctccaccatgtagcaagttctcaggaaaatacaattgatatcttcctcctaagctcttccaatcagtcaccaagtacttatgtggttactttgtccagggcacaaaatgcctgtatctaattaaaagcctacaaaactgcttgataacagttttgaatgtgagacatttatgtaatttaaatgtaaggtacaagttttaatttctgagtttcttctattatatttttattaaaaaaagaaaataattttcagattgaattggagtaaaataatattacttcccactagaattatatatcctggaaaattgtatttttgttacataagcagcttttaaagaaagatcattacccttttctctacataaatatatggggagtcttagcctaatgacaaatatttataatttttaaattaatggtacttgctggatccatactaacatctttactaatacctcattgtttcttccaacttactcctacactacatcctacatcttcttcctagtcttttatctagaatatgcaacctcaaataaaaatggtggtgtcctcattcattctcctccttccttttttcccaagcctgatcttcaaaaggttggttaatttggcagctgagttcctccccaggcagagaatagaccaattttaggtgtattgggactgagggaggatgtgtaaagattaacatcagtaaagaaccgctgtggagtaattaagaactttgttctttataactggagaatataacctaaccctaacatccctcagcctttactaaagtgtggcgtaaatcacagtagtagcaaagaaagtgactctggatgtgttcctggccagtacctcccttatcatgaatgtagactctctcatcaagatttaggaatataaatcaaatcaaatgtgcccagccaagctatgtagtaagggacttgaacaatattaggcagaacctataaaataaatcagggaattagaaattatttaaagttttcaaattgtaaattgccccggtgtctttcagcctactgccattatttttgctacaatacctacatttcagaggagggcctactgaaaattccatgcaagtggaaaataatcctcaagttattaatgagtttgaaaagcaatgagttcttaagtctttgtgagtagagcaagatcctacaaaattcagaaatagtaaaaatggattcatgctgatttgaagagcatctgtgtgcataatataatgctgcatctcttttaaaagcagtctatttttctttttaaatttgtccccatagatgcttttgaacatgaacatgcttatgttaccttttccgaggttgggaagagccaggagctctcaggcagggccccctccctcagctgggcaggagctgctcaggaggagctagttatagaggaagcttagcgttggcattttcaaaattcaaggtgataacgctttcttcttcctttctgttttagaatagattgctgtctgatttgaaaaagggaaatagatttgatctcaaatgaatctgtgcccagaagccaggctcagggtattcagagatttgtatagtgccctcaaaaaataacaaaattttagctttccttttttcttcttttctccatcaaattcttttttctctagtttacaaatgacatggaaaaggaatttcccctgagttttgtatgcctttttttttttggcttagactatagataggcgtgttgagctcctaagaaaatacaaggaggaactctttgttgtgcagagcactttatgagtagtttgtgtggataatatgtgactgcttccctgacgagcttgtgaggctgtacttatgtctttcctgtaaggcagcttcagtgccttctgtagtgtatataaggaaagattacgccttctgaaaaatctcagagcaaccataagattattttaaaatatgtagtatgactgatggactttttcatcattaaattagtctagcatctaaacttttaccactgaaataatattgaccaaaaagcaatttataaaaggtatttgtgaatagaaaatacaatgtgatcatttgtacttatgtgcaccttaaaagaggaattctgtctagctgtcaaattctggttccttaacatccagtccttgattgtgattgagatctggtaggacgtgctggggcacgctagcagataaaatcccgtatactttaggatagatgttacatttatgtcagtgttggcaaagagcattgtgtagtaataaagaattcaagacttcagcaatgtcaacctgaaactttgtaaatatttcctagattgttatttgatgcagtcacagctctttatcacacaatgttgtctttccctcatcaggcaattttagaactgctgcacacccctcctcagatctcacctgcccctcctgtacattcacctctccagccttgtgcacacctcatttagctttagtttgaaacacattgcagggttcaggtgacctcttcaaaaactacctcctcagaatgaggtaatgaatagttatttattttaaaatatgaaaagtcaggagctctagaatatgaagatgatctaagattttaacttttatgtatacttgttgagcactctccttttgtcctaaagggcattatacatttaagcagtaatactgaaaaatgtagctcagagtaactgaatgttgttgaaagtggtgccagaatctgttttaggggtacgtatcagaatcttaatcttaaatcggttacatgaaattaaatagttaatggtaacacttgactaacagatataattttaattttcggtaggcttttagcaagacagtaagtacatcttcataatgagttagccacagcttcatcacatgcacagattttcctgttgagagactgcccagttaagagggtagaatgatgaaccatttttcaggattctcttctttgtccaaactggcattgtgagtgctagaatatcagcactttcaaactagtgattccaactattaggctattaaaaagcaaaacaaaccaaacaaaccatagccagacatgggaagtttactatgagtataaacagcaaatagcttacaggtcatacattgaaatggtgtaggtaaggcgttagaaaaataccttgacaatttgccaaatgatcttactgtgccttcatgatgcaataaaaaaaaaaaaaatttagcataaatcagtgatttgtgaagagagcagccaccctggtctaactcagctgtgttaatattttttagcgtgcaatttagactgcaaagataaatgcactaaagagtttatagccaaaatcacatttaaaaaatgagagaaaacacaggtaaattttcagtgaacaaaattatttttttaaagtacataatccctagtatagtcagatatatttatcacatagagcaaataggttgaaatcacaattcagtgacatttctagagaaactttttctactcccataggttcttcaaagcatggaacttttatataacagaaatgtgtgacggtcattttaaattgctgtagtttggggctgaagtactgtgtgctgggcagcaatcacatgtattaactagtgagaaaggagaaattaagatataggacagaatttgattttcttgttcccagattactgctgccaacctagacactgagtttccagaggctgaaacgtaaacttgcagctcagcaactgttttgcaaagttagtgggactgtcctgcttatgctgttcaaaaatgctctgagggccaggtggggcctccaggggctcctctctgaggggacatcagactagctaacgacctggcgggcggatgtgaaccggacacactccatggtgtgcttcttgtatcggtccctcgccaccctcaagaaaggcttcagcgggttctctagacgtctccactaaggtgtgttactaacagccatgggttgttgagcacccgaggagtgcaatagcatctctgcatgattgtatattggcccgaagagaatgaagtggccagtgtactcatgttccatgttgctagctctggtaaactgaaaatactggtaagatttttgttttatcagtacactagagagtaagctttgttttgttgtttttagataatgttttcacttccatttggaaagacatttaaattgagtttcagtcctaaattttgccagtcatggtaattagcagtttctatcaggtatttttaaggtagaagaggatagaaacataagttctaaaagcttaaggtaaccgtggtttattttaaaatgtttaggggtggttagtctctacctcaaaaaaagtgagtgaatcttttatttcagcattcacaagttcggctgttgtttttgtaatacattttttttttaaccttttgacccccctttacctaagtgtcaatgtagttttattaattactaagtcagtttcattaaaatgtttatttagcagttttgactaattgcaatgattaatatagccagttgtgcatgaggacacagccagtgagtatatctgggttttttttgtgatgctttttttcttaagacttctgtagatttatgaagtactcattgaaaacaactaaaatacgtttattcgtgttaatatggaaaaaaaaaaa

SEQ ID NO: 71 - protein, 766 aa, Bos taurus
MAALSGGGGGGGGGAEQGQALFNGDMEPEAGAAASSAADPAIPEEVWNIKQMIKLTQEHIEALLDKFGGEHNPPSIYLEAYEEYTSKLDALQQREQQLLESLGNGTDFSVSSSASTDTVTSSSSSSLSVLPSSLSVFQNPTDVSRSNPKSPQKPIVRVFLPNKQRTVVPARCGVTVRDSLKKALMMRGLIPECCAVYRIQDGEKKPIGWDTDISWLTGEELHVEVLENVPLTTHNFVRKTFFTLAFCDFCRKLLFQGFRCQTCGYKFHQRCSTEVPLMCVNYDQLDLLFVSKFFEHHPIPQEEASLAETTLPCGSSPSAPPSDSIGPPILTSPSPSKSIPIPQPFRPADEDHRNQFGQRDRSSSAPNVHINTIEPVNIDDLIRDQGFRSDGGSTTGLSATPPASLPGSLSNVKALQKSPGPQRERKSSSSSEDRNRMKTLGRRDSSDDWEIPDGQITVGQRIGSGSFGTVYKGKWHGDVAVKMLNVTAPTPQQLQAFKNEVGVLRKTRHVNILLFMGYSTKPQLAIVTQWCEGSSLYHHLHIIETKFEMIKLIDIARQTAQGMDYLHAKSIIHRDLKSNNIFLHEDLTVKIGDFGLATVKSRWSGSHQFEQLSGSILWMAPEVIRMQDKNPYSFQSDVYAFGIVLYELMTGQLPYSNINNRDQIIFMVGRGYLSPDLSKVRSNCPKAMKRLMAECLKKKRDERPLFPQILASIELLARSLPKIHRSASEPSLNRAGFQTEDFSLYACASPKTPIQAGGYGEFAAFK

SEQ ID NO: 72 - DNA, 4670 bp, Bos taurus
ggtgtgtcatagtgcagcagattgaatgcagaagatatgaaaattcagatgtcttctgttaaggtgtggaatatcaaacaaatgattaagttgacacaggagcatatagaggccctattggacaaatttggtggggagcataatccaccatcaatatatctggaggcctatgaagaatacaccagcaagctagatgccctccaacaaagagaacaacagttattggaatccctggggaatggaactgatttttctgtttctagctctgcatcaacggacaccgttacatcttcttcctcttctagcctttcagtgctgccttcatctctttcagtttttcaaaatcccacagatgtgtcacggagcaaccccaagtcaccacaaaaacctatcgttagagtcttcctgcccaataaacagaggacagtggtacctgcacggtgtggagtcacagtccgggacagcctgaagaaggcactgatgatgagaggtctaatcccagagtgctgtgctgtttacagaattcaggatggggagaagaaaccaattggctgggacactgatatttcctggcttactggagaggagttgcatgtagaagtgttggagaatgttccacttacaacacacaactttgtacggaaaacttttttcaccttagcattttgtgacttctgtagaaagctgcttttccagggattccgctgtcaaacatgtggttataaatttcaccagcgttgtagtacagaggttccactgatgtgtgttaattatgaccaactagatttgctgtttgtctccaagttctttgaacaccacccaataccacaggaggaggcctccttagcagagactacccttccatgtggctcatccccttctgcacccccctccgattctattgggcccccaattctcaccagtccatctccttcaaaatccattccaattccacagcctttccgaccagcagatgaagatcatcgaaatcagtttggacaacgagaccggtcctcatcagctccaaatgtgcatataaacacaatagaacccgtcaatattgatgacttgattagagaccaagggtttcgtagtgatggaggatcaaccacaggtttatccgccacaccccctgcctcattacctggctcactctctaatgtgaaagcattgcagaaatctccaggacctcagcgagaaagaaagtcctcttcatcctcagaagacaggaatcgaatgaaaacgcttggtagacgggattcaagtgacgattgggagattcctgatggacagatcacagtgggacaaagaattggatcagggtcatttgggacagtctacaagggaaagtggcatggtgatgtggcagtgaaaatgttgaatgtgacagcacccacacctcagcagttacaggccttcaaaaatgaagtaggagtactcaggaaaacgcgacatgtgaatatcctcctcttcatgggttattcaacaaagccacaactggctattgttacccagtggtgtgagggctccagtttatatcatcatctccacatcattgagaccaaattcgagatgatcaaacttatagatattgcacggcagactgcacagggcatggattacttacacgccaagtcaatcatccacagagacctcaagagtaataatatttttcttcatgaagacctcacagtaaaaataggtgattttggtctagccacagtgaaatctcgatggagtgggtcccatcagtttgaacagttgtctggatccattttgtggatggcaccagaagtaatcagaatgcaagataaaaacccatatagctttcagtcagatgtatatgcatttgggattgttctgtatgaattgatgaccggacagttaccttattcaaatatcaacaacagggaccagataatttttatggtgggacgaggatatctgtctccagatctcagtaaggtacggagtaactgtccaaaagccatgaagagattaatggcagagtgcctaaaaaagaaaagagatgaaagaccactctttccccaagtaggaaagactctcctaagcaagagacaaaattcagaagttatcagggaaaaagataagcagattctcgcctctattgagctgctggcccgctcattgccaaaaattcaccgcagtgcatcagaaccctccttgaatcgggctggcttccaaacagaggattttagtctatatgcttgtgcttctccaaaaacacccattcaggcagggggatatgaagcagatttggctcttacatcaaataaaaatagagtagaagttgggatttagagatttcctgacatgcaagaaggaataagcaagaaaaaaaggtttgttttccccaaatcatatctattgtcttttacttctattttttcttaaattttttgtgatttcagagacatgtagagttttattgatacctaaactatgagttcttttttttttttttttttcattattttgatttttttggccaagaggcatatgggatcttagcttgagaaagcaacaattttcttgatgtcattttgggtgagggcacatattgctgtgaacagtgtggtgatagccaccagggaccaaactcacacccgctgcattgaaaggtgaagtcttaaacactggaccagcagagaaattcctactctatgagttctttttgtcatcccctccccgcaccctccacccccaacctaaagtctgatgatgaaatcaacaactattccattagaagcagtagattctggtagcatgatctttagtttgttagtaagattttgtgctttgtggggttgtgtcgttttaaggctaatatttaagtttgtcaaatagaatgctgttcagattgtaaaaatgagtaataaacatctgaagttttttttaagttatttttaacatggtatatacagttgagcttagagtttatcattttctgatattctcttacttagtagatgaattctagccattttttataaagatttctgttaagcaaatcctgttttcacatgggcttcctttaagggattttagattctgctggatatggtgactgctcataagactgttgaaaattacttttaagatgtattagaatacttctgaaaaaaaatagcaaccttaaaaccataagcaaaagtagtaagggtgtttatacatttctagagtccctgtttaggtaatagcctcctatgattgtactttaaatgttttgctctccaaggttttagtaacttggctttttttctaatcagtgccaaactcccccagtttttttaactttaaatatgaggtaataaatcttttacccttccttgatcttttgacttataataccttggtcagttgtttcttaaaaggaatccttaaatggaaagagacaatatcactgtctgcagttctgattagtagttttattcagaatggaaaaacagattattcatttttgaaaattgttcaggggtatgttcattgttaggaccttggactttggagtcagtgcctagctatgcattccaggtctgccattttctggctgtgaaattttggacaagttacttaaccactttaaaccccagctttaagaagtaaattaaccccagtaaattaagaagtaatagcagccacttcgtagagttgttatgaggctcagatgcagtgcaaatgtgtataaagtattcagggagtcacctggtatactataatagacactagaatagttgccaatattatcagcatacaatctgaggattctgtcagccaatcattagcaatctgttgtttgttgggacatgccagtgttctccagttgaaatcagtagcaatctaaaaatggatagattattcctcatttaaatagtgtgttcatataagtgattgcttggatccttatcagaagttgctgttactgaaaaatgataaggctgactaaattgtgatagttgtcagttactaaccaactcccagaaatgaataagaggaacctatctctagttcctagtagaaggtatggacaaaatagtaggtgaaaaataatgtcttgaacccccaaattaagtaagctttaaagagtacaatacctcaaagggtctttgcggtttaaaatttgtatgctgagaatgatgttcattgacatgtgcctatatgtaattttttgatagtttaaaaggtgaaatgaactacagatgggagaggtctgaattttcttgccttcagtcaaatgtgtaatgtggacatattatttgacctgtgaattttatcttttaaaaaagattaattcctgcttcttccttcctaatagttgcattataataatgaaaatgagttgataatttggggggaaagtattctacaaatcaaccttattattttaccattggtttctgagaaattttgttcatttgaaccgtttatagcttgattagaatcatagcatgtaaaacccaactgagggattatctgcagacttaatgtagtattatgtaagttgtcttctttcatttcgaccttttttgcttttgttgttgctagatctgtagtatgtagctagtcacctttcagcgaggtttcagcgaggcttttctgtgtctctaggttatttgagataacttttttaaaattagctcttgtcctcc

SEQ ID NO: 73 - protein, 761 aa, Bos taurus
MKIQMSSVKVWNIKQMIKLTQEHIEALLDKFGGEHNPPSIYLEAYEEYTSKLDALQQREQQLLESLGNGTDFSVSSSASTDTVTSSSSSSLSVLPSSLSVFQNPTDVSRSNPKSPQKPIVRVFLPNKQRTVVPARCGVTVRDSLKKALMMRGLIPECCAVYRIQDGEKKPIGWDTDISWLTGEELHVEVLENVPLTTHNFVRKTFFTLAFCDFCRKLLFQGFRCQTCGYKFHQRCSTEVPLMCVNYDQLDLLFVSKFFEHHPIPQEEASLAETTLPCGSSPSAPPSDSIGPPILTSPSPSKSIPIPQPFRPADEDHRNQFGQRDRSSSAPNVHINTIEPVNIDDLIRDQGFRSDGGSTTGLSATPPASLPGSLSNVKALQKSPGPQRERKSSSSSEDRNRMKTLGRRDSSDDWEIPDGQITVGQRIGSGSFGTVYKGKWHGDVAVKMLNVTAPTPQQLQAFKNEVGVLRKTRHVNILLFMGYSTKPQLAIVTQWCEGSSLYHHLHIIETKFEMIKLIDIARQTAQGMDYLHAKSIIHRDLKSNNIFLHEDLTVKIGDFGLATVKSRWSGSHQFEQLSGSILWMAPEVIRMQDKNPYSFQSDVYAFGIVLYELMTGQLPYSNINNRDQIIFMVGRGYLSPDLSKVRSNCPKAMKRLMAECLKKKRDERPLFPQVGKTLLSKRQNSEVIREKDKQILASIELLARSLPKIHRSASEPSLNRAGFQTEDFSLYACASPKTPIQAGGYEADLALTSNKNRVEVGI

SEQ ID NO: 74 - DNA, 4816 bp, Bos taurus
ctcagctgcgccgggtctcacaagacggttcccgaggtggcccaggcgccgtcccaccgccgacgccgcccgggccgcccgggccgtccctccccgctgccccccgtcctccgcctccgcctccccccgccctcagcctcccttccccctccccgcccagcagcggtcgctcgggcccggctctcggttataagatggcggcgctgagtggcggcggcggcggcggcggcggtggcgcggagcagggccaggctctgttcaacggggacatggagcccgaggccggcgccgcggcctcttcggctgcggaccccgccattcccgaggaggtgtggaatatcaaacaaatgattaagttgacacaggagcatatagaggccctattggacaaatttggtggggagcataatccaccatcaatatatctggaggcctatgaagaatacaccagcaagctagatgccctccaacaaagagaacaacagttattggaatccctggggaatggaactgatttttctgtttctagctctgcatcaacggacaccgttacatcttcttcctcttctagcctttcagtgctgccttcatctctttcagtttttcaaaatcccacagatgtgtcacggagcaaccccaagtcaccacaaaaacctatcgttagagtcttcctgcccaataaacagaggacagtggtacctgcacggtgtggagtcacagtccgggacagcctgaagaaggcactgatgatgagaggtctaatcccagagtgctgtgctgtttacagaattcaggatggggagaagaaaccaattggctgggacactgatatttcctggcttactggagaggagttgcatgtagaagtgttggagaatgttccacttacaacacacaactttgtacggaaaacttttttcaccttagcattttgtgacttctgtagaaagctgcttttccagggattccgctgtcaaacatgtggttataaatttcaccagcgttgtagtacagaggttccactgatgtgtgttaattatgaccaactagagcccccaattctcaccagtccatctccttcaaaatccattccaattccacagcctttccgaccagcagatgaagatcatcgaaatcagtttggacaacgagaccggtcctcatcagctccaaatgtgcatataaacacaatagaacccgtcaatattgatgacttgattagagaccaagggtttcgtagtgatggaggatcaaccacaggtttatccgccacaccccctgcctcattacctggctcactctctaatgtgaaagcattgcagaaatctccaggacctcagcgagaaagaaagtcctcttcatcctcagaagacaggaatcgaatgaaaacgcttggtagacgggattcaagtgacgattgggagattcctgatggacagatcacagtgggacaaagaattggatcagggtcatttgggacagtctacaagggaaagtggcatggtgatgtggcagtgaaaatgttgaatgtgacagcacccacacctcagcagttacaggccttcaaaaatgaagtaggagtactcaggaaaacgcgacatgtgaatatcctcctcttcatgggttattcaacaaagccacaactggctattgttacccagtggtgtgagggctccagtttatatcatcatctccacatcattgagaccaaattcgagatgatcaaacttatagatattgcacggcagactgcacagggcatggattacttacacgccaagtcaatcatccacagagacctcaagagtaataatatttttcttcatgaagacctcacagtaaaaataggtgattttggtctagccacagtgaaatctcgatggagtgggtcccatcagtttgaacagttgtctggatccattttgtggatggcaccagaagtaatcagaatgcaagataaaaacccatatagctttcagtcagatgtatatgcatttgggattgttctgtatgaattgatgaccggacagttaccttattcaaatatcaacaacagggaccagataatttttatggtgggacgaggatatctgtctccagatctcagtaaggtacggagtaactgtccaaaagccatgaagagattaatggcagagtgcctaaaaaagaaaagagatgaaagaccactctttccccaagtaggaaagactctcctaagcaagagacaaaattcagaagttatcagggaaaaagataagcagattctcgcctctattgagctgctggcccgctcattgccaaaaattcaccgcagtgcatcagaaccctccttgaatcgggctggcttccaaacagaggattttagtctatatgcttgtgcttctccaaaaacacccattcaggcagggggatatgaagcagatttggctcttacatcaaataaaaatagagtagaagttgggatttagagatttcctgacatgcaagaaggaataagcaagaaaaaaaggtttgttttccccaaatcatatctattgtcttttacttctattttttcttaaattttttgtgatttcagagacatgtagagttttattgatacctaaactatgagttcttttttttttttttttttcattattttgatttttttggccaagaggcatatgggatcttagcttgagaaagcaacaattttcttgatgtcattttgggtgagggcacatattgctgtgaacagtgtggtgatagccaccagggaccaaactcacacccgctgcattgaaaggtgaagtcttaaacactggaccagcagagaaattcctactctatgagttctttttgtcatcccctccccgcaccctccacccccaacctaaagtctgatgatgaaatcaacaactattccattagaagcagtagattctggtagcatgatctttagtttgttagtaagattttgtgctttgtggggttgtgtcgttttaaggctaatatttaagtttgtcaaatagaatgctgttcagattgtaaaaatgagtaataaacatctgaagttttttttaagttatttttaacatggtatatacagttgagcttagagtttatcattttctgatattctcttacttagtagatgaattctagccattttttataaagatttctgttaagcaaatcctgttttcacatgggcttcctttaagggattttagattctgctggatatggtgactgctcataagactgttgaaaattacttttaagatgtattagaatacttctgaaaaaaaatagcaaccttaaaaccataagcaaaagtagtaagggtgtttatacatttctagagtccctgtttaggtaatagcctcctatgattgtactttaaatgttttgctctccaaggttttagtaacttggctttttttctaatcagtgccaaactcccccagtttttttaactttaaatatgaggtaataaatcttttacccttccttgatcttttgacttataataccttggtcagttgtttcttaaaaggaatccttaaatggaaagagacaatatcactgtctgcagttctgattagtagttttattcagaatggaaaaacagattattcatttttgaaaattgttcaggggtatgttcattgttaggaccttggactttggagtcagtgcctagctatgcattccaggtctgccattttctggctgtgaaattttggacaagttacttaaccactttaaaccccagctttaagaagtaaattaaccccagtaaattaagaagtaatagcagccacttcgtagagttgttatgaggctcagatgcagtgcaaatgtgtataaagtattcagggagtcacctggtatactataatagacactagaatagttgccaatattatcagcatacaatctgaggattctgtcagccaatcattagcaatctgttgtttgttgggacatgccagtgttctccagttgaaatcagtagcaatctaaaaatggatagattattcctcatttaaatagtgtgttcatataagtgattgcttggatccttatcagaagttgctgttactgaaaaatgataaggctgactaaattgtgatagttgtcagttactaaccaactcccagaaatgaataagaggaacctatctctagttcctagtagaaggtatggacaaaatagtaggtgaaaaataatgtcttgaacccccaaattaagtaagctttaaagagtacaatacctcaaagggtctttgcggtttaaaatttgtatgctgagaatgatgttcattgacatgtgcctatatgtaattttttgatagtttaaaaggtgaaatgaactacagatgggagaggtctgaattttcttgccttcagtcaaatgtgtaatgtggacatattatttgacctgtgaattttatcttttaaaaaagattaattcctgcttcttccttcctaatagttgcattataataatgaaaatgagttgataatttggggggaaagtattctacaaatcaaccttattattttaccattggtttctgagaaattttgttcatttgaaccgtttatagcttgattagaatcatagcatgtaaaacccaactgagggattatctgcagacttaatgtagtattatgtaagttgtcttctttcatttcgaccttttttgcttttgttgttgctagatctgtagtatgtagctagtcacctttcagcgaggtttcagcgaggcttttctgtgtctctaggttatttgagataacttttttaaaattagctcttgtcctcc

SEQ ID NO: 75 - protein, 757 aa, Bos taurus
MAALSGGGGGGGGGAEQGQALFNGDMEPEAGAAASSAADPAIPEEVWNIKQMIKLTQEHIEALLDKFGGEHNPPSIYLEAYEEYTSKLDALQQREQQLLESLGNGTDFSVSSSASTDTVTSSSSSSLSVLPSSLSVFQNPTDVSRSNPKSPQKPIVRVFLPNKQRTVVPARCGVTVRDSLKKALMMRGLIPECCAVYRIQDGEKKPIGWDTDISWLTGEELHVEVLENVPLTTHNFVRKTFFTLAFCDFCRKLLFQGFRCQTCGYKFHQRCSTEVPLMCVNYDQLEPPILTSPSPSKSIPIPQPFRPADEDHRNQFGQRDRSSSAPNVHINTIEPVNIDDLIRDQGFRSDGGSTTGLSATPPASLPGSLSNVKALQKSPGPQRERKSSSSSEDRNRMKTLGRRDSSDDWEIPDGQITVGQRIGSGSFGTVYKGKWHGDVAVKMLNVTAPTPQQLQAFKNEVGVLRKTRHVNILLFMGYSTKPQLAIVTQWCEGSSLYHHLHIIETKFEMIKLIDIARQTAQGMDYLHAKSIIHRDLKSNNIFLHEDLTVKIGDFGLATVKSRWSGSHQFEQLSGSILWMAPEVIRMQDKNPYSFQSDVYAFGIVLYELMTGQLPYSNINNRDQIIFMVGRGYLSPDLSKVRSNCPKAMKRLMAECLKKKRDERPLFPQVGKTLLSKRQNSEVIREKDKQILASIELLARSLPKIHRSASEPSLNRAGFQTEDFSLYACASPKTPIQAGGYEADLALTSNKNRVEVGI

SEQ ID NO: 76 - DNA, 2499 bp, Bos taurus
ctcagctgcgccgggtctcacaagacggttcccgaggtggcccaggcgccgtcccaccgccgacgccgcccgggccgcccgggccgtccctccccgctgccccccgtcctccgcctccgcctccccccgccctcagcctcccttccccctccccgcccagcagcggtcgctcgggcccggctctcggttataagatggcggcgctgagtggcggcggcggcggcggcggcggtggcgcggagcagggccaggctctgttcaacggggacatggagcccgaggccggcgccgcggcctcttcggctgcggaccccgccattcccgaggaggtgtggaatatcaaacaaatgattaagttgacacaggagcatatagaggccctattggacaaatttggtggggagcataatccaccatcaatatatctggaggcctatgaagaatacaccagcaagctagatgccctccaacaaagagaacaacagttattggaatccctggggaatggaactgatttttctgtttctagctctgcatcaacggacaccgttacatcttcttcctcttctagcctttcagtgctgccttcatctctttcagtttttcaaaatcccacagatgtgtcacggagcaaccccaagtcaccacaaaaacctatcgttagagtcttcctgcccaataaacagaggacagtggtacctgcacggtgtggagtcacagtccgggacagcctgaagaaggcactgatgatgagaggtctaatcccagagtgctgtgctgtttacagaattcaggatggggagaagaaaccaattggctgggacactgatatttcctggcttactggagaggagttgcatgtagaagtgttggagaatgttccacttacaacacacaactttgtacggaaaacttttttcaccttagcattttgtgacttctgtagaaagctgcttttccagggattccgctgtcaaacatgtggttataaatttcaccagcgttgtagtacagaggttccactgatgtgtgttaattatgaccaactagatttgctgtttgtctccaagttctttgaacaccacccaataccacaggaggaggcctccttagcagagactacccttccatgtggctcatccccttctgcacccccctccgattctattgggcccccaattctcaccagtccatctccttcaaaatccattccaattccacagcctttccgaccagcagatgaagatcatcgaaatcagtttggacaacgagaccggtcctcatcagctccaaatgtgcatataaacacaatagaacccgtcaatattgatgacttgattagagaccaagggtttcgtagtgatggaggatcaaccacaggtttatccgccacaccccctgcctcattacctggctcactctctaatgtgaaagcattgcagaaatctccaggacctcagcgagaaagaaagtcctcttcatcctcagaagacaggaatcgaatgaaaacgcttggtagacgggattcaagtgacgattgggagattcctgatggacagatcacagtgggacaaagaattggatcagggtcatttgggacagtctacaagggaaagtggcatggtgatgtggcagtgaaaatgttgaatgtgacagcacccacacctcagcagttacaggccttcaaaaatgaagtaggagtactcaggaaaacgcgacatgtgaatatcctcctcttcatgggttattcaacaaagccacaactggctattgttacccagtggtgtgagggctccagtttatatcatcatctccacatcattgagaccaaattcgagatgatcaaacttatagatattgcacggcagactgcacagggcatggattacttacacgccaagtcaatcatccacagagacctcaagagtaataatatttttcttcatgaagacctcacagtaaaaataggtgattttggtctagccacagtgaaatctcgatggagtgggtcccatcagtttgaacagttgtctggatccattttgtggatggcaccagaagtaatcagaatgcaagataaaaacccatatagctttcagtcagatgtatatgcatttgggattgttctgtatgaattgatgaccggacagttaccttattcaaatatcaacaacagggaccagataatttttatggtgggacgaggatatctgtctccagatctcagtaaggtacggagtaactgtccaaaagccatgaagagattaatggcagagtgcctaaaaaagaaaagagatgaaagaccactctttccccaagtaggaaagactctcctaagcaagagacaaaattcagaagttatcagggaaaaagataagcaggaaaagtatgtttctttagtacattccaggcatttgggattacagtaaaaacaatattctcgcctctattgagctgctggcccgctcattgccaaaaattcaccgcagtgcatcagaa

SEQ ID NO: 77 - protein, 744 aa, Bos taurus
MAALSGGGGGGGGGAEQGQALFNGDMEPEAGAAASSAADPAIPEEVWNIKQMIKLTQEHIEALLDKFGGEHNPPSIYLEAYEEYTSKLDALQQREQQLLESLGNGTDFSVSSSASTDTVTSSSSSSLSVLPSSLSVFQNPTDVSRSNPKSPQKPIVRVFLPNKQRTVVPARCGVTVRDSLKKALMMRGLIPECCAVYRIQDGEKKPIGWDTDISWLTGEELHVEVLENVPLTTHNFVRKTFFTLAFCDFCRKLLFQGFRCQTCGYKFHQRCSTEVPLMCVNYDQLDLLFVSKFFEHHPIPQEEASLAETTLPCGSSPSAPPSDSIGPPILTSPSPSKSIPIPQPFRPADEDHRNQFGQRDRSSSAPNVHINTIEPVNIDDLIRDQGFRSDGGSTTGLSATPPASLPGSLSNVKALQKSPGPQRERKSSSSSEDRNRMKTLGRRDSSDDWEIPDGQITVGQRIGSGSFGTVYKGKWHGDVAVKMLNVTAPTPQQLQAFKNEVGVLRKTRHVNILLFMGYSTKPQLAIVTQWCEGSSLYHHLHIIETKFEMIKLIDIARQTAQGMDYLHAKSIIHRDLKSNNIFLHEDLTVKIGDFGLATVKSRWSGSHQFEQLSGSILWMAPEVIRMQDKNPYSFQSDVYAFGIVLYELMTGQLPYSNINNRDQIIFMVGRGYLSPDLSKVRSNCPKAMKRLMAECLKKKRDERPLFPQVGKTLLSKRQNSEVIREKDKQEKYVSLVHSRHLGLQ

SEQ ID NO: 78 - DNA, 2404 bp, Bos taurus
ctcagctgcgccgggtctcacaagacggttcccgaggtggcccaggcgccgtcccaccgccgacgccgcccgggccgcccgggccgtccctccccgctgccccccgtcctccgcctccgcctccccccgccctcagcctcccttccccctccccgcccagcagcggtcgctcgggcccggctctcggttataagatggcggcgctgagtggcggcggcggcggcggcggcggtggcgcggagcagggccaggctctgttcaacggggacatggagcccgaggccggcgccgcggcctcttcggctgcggaccccgccattcccgaggaggtgtggaatatcaaacaaatgattaagttgacacaggagcatatagaggccctattggacaaatttggtggggagcataatccaccatcaatatatctggaggcctatgaagaatacaccagcaagctagatgccctccaacaaagagaacaacagttattggaatccctggggaatggaactgatttttctgtttctagctctgcatcaacggacaccgttacatcttcttcctcttctagcctttcagtgctgccttcatctctttcagtttttcaaaatcccacagatgtgtcacggagcaaccccaagtcaccacaaaaacctatcgttagagtcttcctgcccaataaacagaggacagtggtacctgcacggtgtggagtcacagtccgggacagcctgaagaaggcactgatgatgagaggtctaatcccagagtgctgtgctgtttacagaattcaggatggggagaagaaaccaattggctgggacactgatatttcctggcttactggagaggagttgcatgtagaagtgttggagaatgttccacttacaacacacaactttgtacggaaaacttttttcaccttagcattttgtgacttctgtagaaagctgcttttccagggattccgctgtcaaacatgtggttataaatttcaccagcgttgtagtacagaggttccactgatgtgtgttaattatgaccaactagatttgctgtttgtctccaagttctttgaacaccacccaataccacaggaggaggcctccttagcagagactacccttccatgtggctcatccccttctgcacccccctccgattctattgggcccccaattctcaccagtccatctccttcaaaatccattccaattccacagcctttccgaccagcagatgaagatcatcgaaatcagtttggacaacgagaccggtcctcatcagctccaaatgtgcatataaacacaatagaacccgtcaatattgatgacttgattagagaccaagggtttcgtagtgatggaggatcaaccacaggtttatccgccacaccccctgcctcattacctggctcactctctaatgtgaaagcattgcagaaatctccaggacctcagcgagaaagaaagtcctcttcatcctcagaagacaggaatcgaatgaaaacgcttggtagacgggattcaagtgacgattgggagattcctgatggacagatcacagtgggacaaagaattggatcagggtcatttgggacagtctacaagggaaagtggcatggtgatgtggcagtgaaaatgttgaatgtgacagcacccacacctcagcagttacaggccttcaaaaatgaagtaggagtactcaggaaaacgcgacatgtgaatatcctcctcttcatgggttattcaacaaagccacaactggctattgttacccagtggtgtgagggctccagtttatatcatcatctccacatcattgagaccaaattcgagatgatcaaacttatagatattgcacggcagactgcacagggcatggattacttacacgccaagtcaatcatccacagagacctcaagagtaataatatttttcttcatgaagacctcacagtaaaaataggtgattttggtctagccacagtgaaatctcgatggagtgggtcccatcagtttgaacagttgtctggatccattttgtggatggcaccagaagtaatcagaatgcaagataaaaacccatatagctttcagtcagatgtatatgcatttgggattgttctgtatgaattgatgaccggacagttaccttattcaaatatcaacaacagggaccagataatttttatggtgggacgaggatatctgtctccagatctcagtaaggtacggagtaactgtccaaaagccatgaagagattaatggcagagtgcctaaaaaagaaaagagatgaaagaccactctttccccaagatctctcttcccaccatagacacaaaaatttcagatggctacaggtttacatgtaaaaaacagaattataacaaatgatttttat

SEQ ID NO: 79 - protein, 726 aa, Bos taurus
MAALSGGGGGGGGGAEQGQALFNGDMEPEAGAAASSAADPAIPEEVWNIKQMIKLTQEHIEALLDKFGGEHNPPSIYLEAYEEYTSKLDALQQREQQLLESLGNGTDFSVSSSASTDTVTSSSSSSLSVLPSSLSVFQNPTDVSRSNPKSPQKPIVRVFLPNKQRTVVPARCGVTVRDSLKKALMMRGLIPECCAVYRIQDGEKKPIGWDTDISWLTGEELHVEVLENVPLTTHNFVRKTFFTLAFCDFCRKLLFQGFRCQTCGYKFHQRCSTEVPLMCVNYDQLDLLFVSKFFEHHPIPQEEASLAETTLPCGSSPSAPPSDSIGPPILTSPSPSKSIPIPQPFRPADEDHRNQFGQRDRSSSAPNVHINTIEPVNIDDLIRDQGFRSDGGSTTGLSATPPASLPGSLSNVKALQKSPGPQRERKSSSSSEDRNRMKTLGRRDSSDDWEIPDGQITVGQRIGSGSFGTVYKGKWHGDVAVKMLNVTAPTPQQLQAFKNEVGVLRKTRHVNILLFMGYSTKPQLAIVTQWCEGSSLYHHLHIIETKFEMIKLIDIARQTAQGMDYLHAKSIIHRDLKSNNIFLHEDLTVKIGDFGLATVKSRWSGSHQFEQLSGSILWMAPEVIRMQDKNPYSFQSDVYAFGIVLYELMTGQLPYSNINNRDQIIFMVGRGYLSPDLSKVRSNCPKAMKRLMAECLKKKRDERPLFPQDLSSHHRHKNFRWLQVYM

SEQ ID NO: 80 - DNA, 2331 bp, Bos taurus
ctcagctgcgccgggtctcacaagacggttcccgaggtggcccaggcgccgtcccaccgccgacgccgcccgggccgcccgggccgtccctccccgctgccccccgtcctccgcctccgcctccccccgccctcagcctcccttccccctccccgcccagcagcggtcgctcgggcccggctctcggttataagatggcggcgctgagtggcggcggcggcggcggcggcggtggcgcggagcagggccaggctctgttcaacggggacatggagcccgaggccggcgccgcggcctcttcggctgcggaccccgccattcccgaggaggtgtggaatatcaaacaaatgattaagttgacacaggagcatatagaggccctattggacaaatttggtggggagcataatccaccatcaatatatctggaggcctatgaagaatacaccagcaagctagatgccctccaacaaagagaacaacagttattggaatccctggggaatggaactgatttttctgtttctagctctgcatcaacggacaccgttacatcttcttcctcttctagcctttcagtgctgccttcatctctttcagtttttcaaaatcccacagatgtgtcacggagcaaccccaagtcaccacaaaaacctatcgttagagtcttcctgcccaataaacagaggacagtggtacctgcacggtgtggagtcacagtccgggacagcctgaagaaggcactgatgatgagaggtctaatcccagagtgctgtgctgtttacagaattcaggatggggagaagaaaccaattggctgggacactgatatttcctggcttactggagaggagttgcatgtagaagtgttggagaatgttccacttacaacacacaactttgtacggaaaacttttttcaccttagcattttgtgacttctgtagaaagctgcttttccagggattccgctgtcaaacatgtggttataaatttcaccagcgttgtagtacagaggttccactgatgtgtgttaattatgaccaactagatttgctgtttgtctccaagttctttgaacaccacccaataccacaggaggaggcctccttagcagagactacccttccatgtggctcatccccttctgcacccccctccgattctattgggcccccaattctcaccagtccatctccttcaaaatccattccaattccacagcctttccgaccagcagatgaagatcatcgaaatcagtttggacaacgagaccggtcctcatcagctccaaatgtgcatataaacacaatagaacccgtcaatattgatgacttgattagagaccaagggtttcgtagtgatggaggatcaaccacaggtttatccgccacaccccctgcctcattacctggctcactctctaatgtgaaagcattgcagaaatctccaggacctcagcgagaaagaaagtcctcttcatcctcagaagacaggaatcgaatgaaaacgcttggtagacgggattcaagtgacgattgggagattcctgatggacagatcacagtgggacaaagaattggatcagggtcatttgggacagtctacaagggaaagtggcatggtgatgtggcagtgaaaatgttgaatgtgacagcacccacacctcagcagttacaggccttcaaaaatgaagtaggagtactcaggaaaacgcgacatgtgaatatcctcctcttcatgggttattcaacaaagccacaactggctattgttacccagtggtgtgagggctccagtttatatcatcatctccacatcattgagaccaaattcgagatgatcaaacttatagatattgcacggcagactgcacagggcatggattacttacacgccaagtcaatcatccacagagacctcaagagtaataatatttttcttcatgaagacctcacagtaaaaataggtgattttggtctagccacagtgaaatctcgatggagtgggtcccatcagtttgaacagttgtctggatccattttgtggatggcaccagaagtaatcagaatgcaagataaaaacccatatagctttcagtcagatgtatatgcatttgggattgttctgtatgaattgatgaccggacagttaccttattcaaatatcaacaacagggaccaggtgctttgtcctccatgggagtgtaataaatgctgtgcaagggcttacttcccatgagagaagtgagtgaccaacagaaggataatttttatggtgggacgaggatatctgtctccagatctcagtaaggtacggagtaactgtccaa

SEQ ID NO: 81 - protein, 681 aa, Bos taurus
MAALSGGGGGGGGGAEQGQALFNGDMEPEAGAAASSAADPAIPEEVWNIKQMIKLTQEHIEALLDKFGGEHNPPSIYLEAYEEYTSKLDALQQREQQLLESLGNGTDFSVSSSASTDTVTSSSSSSLSVLPSSLSVFQNPTDVSRSNPKSPQKPIVRVFLPNKQRTVVPARCGVTVRDSLKKALMMRGLIPECCAVYRIQDGEKKPIGWDTDISWLTGEELHVEVLENVPLTTHNFVRKTFFTLAFCDFCRKLLFQGFRCQTCGYKFHQRCSTEVPLMCVNYDQLDLLFVSKFFEHHPIPQEEASLAETTLPCGSSPSAPPSDSIGPPILTSPSPSKSIPIPQPFRPADEDHRNQFGQRDRSSSAPNVHINTIEPVNIDDLIRDQGFRSDGGSTTGLSATPPASLPGSLSNVKALQKSPGPQRERKSSSSSEDRNRMKTLGRRDSSDDWEIPDGQITVGQRIGSGSFGTVYKGKWHGDVAVKMLNVTAPTPQQLQAFKNEVGVLRKTRHVNILLFMGYSTKPQLAIVTQWCEGSSLYHHLHIIETKFEMIKLIDIARQTAQGMDYLHAKSIIHRDLKSNNIFLHEDLTVKIGDFGLATVKSRWSGSHQFEQLSGSILWMAPEVIRMQDKNPYSFQSDVYAFGIVLYELMTGQLPYSNINNRDQVLCPPWECNKCCARAYFP

SEQ ID NO: 82 - DNA, 2319 bp, Bos taurus
ctcagctgcgccgggtctcacaagacggttcccgaggtggcccaggcgccgtcccaccgccgacgccgcccgggccgcccgggccgtccctccccgctgccccccgtcctccgcctccgcctccccccgccctcagcctcccttccccctccccgcccagcagcggtcgctcgggcccggctctcggttataagatggcggcgctgagtggcggcggcggcggcggcggcggtggcgcggagcagggccaggctctgttcaacggggacatggagcccgaggccggcgccgcggcctcttcggctgcggaccccgccattcccgaggaggtgtggaatatcaaacaaatgattaagttgacacaggagcatatagaggccctattggacaaatttggtggggagcataatccaccatcaatatatctggaggcctatgaagaatacaccagcaagctagatgccctccaacaaagagaacaacagttattggaatccctggggaatggaactgatttttctgtttctagctctgcatcaacggacaccgttacatcttcttcctcttctagcctttcagtgctgccttcatctctttcagtttttcaaaatcccacagatgtgtcacggagcaaccccaagtcaccacaaaaacctatcgttagagtcttcctgcccaataaacagaggacagtggtacctgcacggtgtggagtcacagtccgggacagcctgaagaaggcactgatgatgagaggtctaatcccagagtgctgtgctgtttacagaattcaggatggggagaagaaaccaattggctgggacactgatatttcctggcttactggagaggagttgcatgtagaagtgttggagaatgttccacttacaacacacaactttgtacggaaaacttttttcaccttagcattttgtgacttctgtagaaagctgcttttccagggattccgctgtcaaacatgtggttataaatttcaccagcgttgtagtacagaggttccactgatgtgtgttaattatgaccaactagatttgctgtttgtctccaagttctttgaacaccacccaataccacaggaggaggcctccttagcagagactacccttccatgtggctcatccccttctgcacccccctccgattctattgggcccccaattctcaccagtccatctccttcaaaatccattccaattccacagcctttccgaccagcagatgaagatcatcgaaatcagtttggacaacgagaccggtcctcatcagctccaaatgtgcatataaacacaatagaacccgtcaatattgatgacttgattagagaccaagggtttcgtagtgatggaggatcaaccacaggtttatccgccacaccccctgcctcattacctggctcactctctaatgtgaaagcattgcagaaatctccaggacctcagcgagaaagaaagtcctcttcatcctcagaagacaggaatcgaatgaaaacgcttggtagacgggattcaagtgacgattgggagattcctgatggacagatcacagtgggacaaagaattggatcagggtcatttgggacagtctacaagggaaagtggcatggtgatgtggcagtgaaaatgttgaatgtgacagcacccacacctcagcagttacaggccttcaaaaatgaagtaggagtactcaggaaaacgcgacatgtgaatatcctcctcttcatgggttattcaacaaagccacaactggctattgttacccagtggtgtgagggctccagtttatatcatcatctccacatcattgagaccaaattcgagatgatcaaacttatagatattgcacggcagactgcacagggcatggattacttacacgccaagtcaatcatccacagagacctcaagagtaataatatttttcttcatgaagacctcacagtaaaaataggtgattttggtctagccacagtgaaatctcgatggagtgggtcccatcagtttgaacagttgtctggatccattttgtggatggcaccagaagtaatcagaatgcaagataaaaacccatatagctttcagtcagatgtatatgcatttgggattgttctgtatgaattgatgaccggacagttaccttattcaaatatcaacaacagggaccaggtgctttgtcctccatgggagtgtaataaatgctgtgcaagggcttacttcccatgagagaagtgagtgaccaacagaaggtctgtgcaaggaaaagagacaaagccacggatcagaagcacatggccataactga

SEQ ID NO: 83 - protein, 681 aa, Bos taurus; identical to SEQ ID NO: 81

SEQ ID NO: 84 - DNA, 2661 bp, Bos taurus
tcagctgcgccgggtctcacaagacggttcccgaggtggcccaggcgccgtcccaccgccgacgccgcccgggccgcccgggccgtccctccccgctgccccccgtcctccgcctccgcctccccccgccctcagcctcccttccccctccccgcccagcagcggtcgctcgggcccggctctcggttataagatggcggcgctgagtggcggcggcggcggcggcggcggtggcgcggagcagggccaggctctgttcaacggggacatggagcccgaggccggcgccgcggcctcttcggctgcggaccccgccattcccgaggaggtgtggaatatcaaacaaatgattaagttgacacaggagcatatagaggccctattggacaaatttggtggggagcataatccaccatcaatatatctggaggcctatgaagaatacaccagcaagctagatgccctccaacaaagagaacaacagttattggaatccctggggaatggaactgatttttctgtttctagctctgcatcaacggacaccgttacatcttcttcctcttctagcctttcagtgctgccttcatctctttcagtttttcaaaatcccacagatgtgtcacggagcaaccccaagtcaccacaaaaacctatcgttagagtcttcctgcccaataaacagaggacagtggtacctgcacggtgtggagtcacagtccgggacagcctgaagaaggcactgatgatgagaggtctaatcccagagtgctgtgctgtttacagaattcaggatggggagaagaaaccaattggctgggacactgatatttcctggcttactggagaggagttgcatgtagaagtgttggagaatgttccacttacaacacacaactttgtacggaaaacttttttcaccttagcattttgtgacttctgtagaaagctgcttttccagggattccgctgtcaaacatgtggttataaatttcaccagcgttgtagtacagaggttccactgatgtgtgttaattatgaccaactagatttgctgtttgtctccaagttctttgaacaccacccaataccacaggaggaggcctccttagcagagactacccttccatgtggctcatccccttctgcacccccctccgattctattgggcccccaattctcaccagtccatctccttcaaaatccattccaattccacagcctttccgaccagcagatgaagatcatcgaaatcagtttggacaacgagaccggtcctcatcagctccaaatgtgcatataaacacaatagaacccgtcaatattgatgacttgattagagaccaagggtttcgtagtgatggaggatcaaccacaggtttatccgccacaccccctgcctcattacctggctcactctctaatgtgaaagcattgcagaaatctccaggacctcagcgagaaagaaagtcctcttcatcctcagaagacaggaatcgaatgaaaacgcttggtagacgggattcaagtgacgattgggagattcctgatggacagatcacagtgggacaaagaattggatcagggtcatttgggacagtctacaagggaaagtggcatggtgatgtggcagtgaaaatgttgaatgtgacagcacccacacctcagcagttacaggccttcaaaaatgaagtaggagtactcaggaaaacgcgacatgtgaatatcctcctcttcatgggttattcaacaaagccacaactggctattgttacccagtggtgtgagggctccagtttatatcatcatctccacatcattgagaccaaattcgagatgatcaaacttatagatattgcacggcagactgcacagggcatggattacttacacgccaagtcaatcatccacagagacctcaagagtaataatatttttcttcatgaagacctcacagtaaaaataggtgattttggtctagccacagtgaaatctcgatggagtgggtcccatcagtttgaacagttgtctggatccattttgtggatggcaccagaagtaatcagaatgcaagataaaaacccatatagctttcagtcagatgtatatgcatttgggattgttctgtatgaattgatgaccggacagttaccttattcaaatatcaacaacagggaccagtctgtgcaaggaaaagagacaaagccacggatcagaagcacatggccataactgaagattttgtgaactctcacaaggaaaaaatttgctctttgaacaataagaaggaactcactaaaatgtaactgagaactgttcaacaggttgaaagctgaaagatgccattggaactgacaaaatgtttcttaaacataaatgatgaaacagtgaaactacataatatctcctctggctgaaacattcaagaagtttaaaatgcttaagttaaaaataaaatcctagtaaacaatggacttactgtgcaacatagagaatatcttacgataacctgtaatggaaaagaatctgaaaaagaatgtatataactgaatcactttgctgtaaactagaatctgacacaacactgtaaatcactacacttttctgttgcatgccaaagattatttaataacgtcattaaaaaattattttaataatta

SEQ ID NO: 85 - protein, 679 aa, Bos taurus
MAALSGGGGGGGGGAEQGQALFNGDMEPEAGAAASSAADPAIPEEVWNIKQMIKLTQEHIEALLDKFGGEHNPPSIYLEAYEEYTSKLDALQQREQQLLESLGNGTDFSVSSSASTDTVTSSSSSSLSVLPSSLSVFQNPTDVSRSNPKSPQKPIVRVFLPNKQRTVVPARCGVTVRDSLKKALMMRGLIPECCAVYRIQDGEKKPIGWDTDISWLTGEELHVEVLENVPLTTHNFVRKTFFTLAFCDFCRKLLFQGFRCQTCGYKFHQRCSTEVPLMCVNYDQLDLLFVSKFFEHHPIPQEEASLAETTLPCGSSPSAPPSDSIGPPILTSPSPSKSIPIPQPFRPADEDHRNQFGQRDRSSSAPNVHINTIEPVNIDDLIRDQGFRSDGGSTTGLSATPPASLPGSLSNVKALQKSPGPQRERKSSSSSEDRNRMKTLGRRDSSDDWEIPDGQITVGQRIGSGSFGTVYKGKWHGDVAVKMLNVTAPTPQQLQAFKNEVGVLRKTRHVNILLFMGYSTKPQLAIVTQWCEGSSLYHHLHIIETKFEMIKLIDIARQTAQGMDYLHAKSIIHRDLKSNNIFLHEDLTVKIGDFGLATVKSRWSGSHQFEQLSGSILWMAPEVIRMQDKNPYSFQSDVYAFGIVLYELMTGQLPYSNINNRDQSVQGKETKPRIRSTWP

SEQ ID NO: 86 - DNA, 7434 bp, Bos taurus
acaccgttacatcttcttcctcttctagcctttcagtgctgccttcatctctttcagtttttcaaaatcccacagatgtgtcacggagcaaccccaagtcaccacaaaaacctatcgttagagtcttcctgcccaataaacagaggacagtggtacctgcacggtgtggagtcacagtccgggacagcctgaagaaggcactgatgatgagaggtctaatcccagagtgctgtgctgtttacagaattcaggatggggagaagaaaccaattggctgggacactgatatttcctggcttactggagaggagttgcatgtagaagtgttggagaatgttccacttacaacacacaactttgtacggaaaacttttttcaccttagcattttgtgacttctgtagaaagctgcttttccagggattccgctgtcaaacatgtggttataaatttcaccagcgttgtagtacagaggttccactgatgtgtgttaattatgaccaactagatttgctgtttgtctccaagttctttgaacaccacccaataccacaggaggaggcctccttagcagagactacccttccatgtggctcatccccttctgcacccccctccgattctattgggcccccaattctcaccagtccatctccttcaaaatccattccaattccacagcctttccgaccagcagatgaagatcatcgaaatcagtttggacaacgagaccggtcctcatcagctccaaatgtgcatataaacacaatagaacccgtcaatattgatgacttgattagagaccaagggtttcgtagtgatggaggatcaaccacaggtttatccgccacaccccctgcctcattacctggctcactctctaatgtgaaagcattgcagaaatctccaggacctcagcgagaaagaaagtcctcttcatcctcagaagacaggaatcgaatgaaaacgcttggtagacgggattcaagtgacgattgggagattcctgatggacagatcacagtgggacaaagaattggatcagggtcatttgggacagtctacaagggaaagtggcatggtgatgtggcagtgaaaatgttgaatgtgacagcacccacacctcagcagttacaggccttcaaaaatgaagtaggagtactcaggaaaacgcgacatgtgaatatcctcctcttcatgggttattcaacaaagccacaactggctattgttacccagtggtgtgagggctccagtttatatcatcatctccacatcattgagaccaaattcgagatgatcaaacttatagatattgcacggcagactgcacagggcatggattacttacacgccaagtcaatcatccacagagacctcaagagtaataatatttttcttcatgaagacctcacagtaaaaataggtgattttggtctagccacagtgaaatctcgatggagtgggtcccatcagtttgaacagttgtctggatccattttgtggatggcaccagaagtaatcagaatgcaagataaaaacccatatagctttcagtcagatgtatatgcatttgggattgttctgtatgaattgatgaccggacagttaccttattcaaatatcaacaacagggaccagataatttttatggtgggacgaggatatctgtctccagatctcagtaaggtacggagtaactgtccaaaagccatgaagagattaatggcagagtgcctaaaaaagaaaagagatgaaagaccactctttccccaagtaggaaagactctcctaagcaagagacaaaattcagaagttatcagggaaaaagataagcagattctcgcctctattgagctgctggcccgctcattgccaaaaattcaccgcagtgcatcagaaccctccttgaatcgggctggcttccaaacagaggattttagtctatatgcttgtgcttctccaaaaacacccattcaggcagggggatatggagaatttgcagccttcaagtagccacaccatcatgacagcatctactcttatttcttaagtcttgtgttcgtacaatttgttaacatcaaaacacagttctgttcctcaactctttttaaagttaaaatttttcagtgcataagctggtgtggaacagaaggaaatttcccatccaacaaaagagggaagaatgttttaggaaccagaattctctgctgccagtgtttcttcttcaacacaaatatcacaagtctgcccactcccaggaagaaagaggagagaccctgagttctgaccttttgatggtcaggcatgatggaaagaaactgctgctacagcttgggagatttgctctgggaagtctgccagtcaactttgcccttctaaccaccagatcaatatgtggctgatcatctgatggggcagttgcaatcaccaagccttgttctctttcctgttctgggattgtgttgtggaacccttttccctagccaccaccagttcatttctgagggatggaacaaaaatgcagcatgcccttcctgtgtggtgcatgttcagtccttgacaaatttttaccaaaatgaagctactttatttaaaaggagggtgagaggtgaggaggtcactttgggtgtggcggaaagggaatgctgcatctttttcctgggctgctggggctctggccttggcttgccagccggaagcgctggcacgcatcgccttcttttcccattgggtccagcaatgaagacgagtgtttggggttttttttttctccaccatgtagcaagttctcaggaaaatacaattgatatcttcctcctaagctcttccaatcagtcaccaagtacttatgtggttactttgtccagggcacaaaatgcctgtatctaattaaaagcctacaaaactgcttgataacagttttgaatgtgagacatttatgtaatttaaatgtaaggtacaagttttaatttctgagtttcttctattatatttttattaaaaaaagaaaataattttcagattgaattggagtaaaataatattacttcccactagaattatatatcctggaaaattgtatttttgttacataagcagcttttaaagaaagatcattacccttttctctacataaatatatggggagtcttagcctaatgacaaatatttataatttttaaattaatggtacttgctggatccatactaacatctttactaatacctcattgtttcttccaacttactcctacactacatcctacatcttcttcctagtcttttatctagaatatgcaacctcaaataaaaatggtggtgtcctcattcattctcctccttccttttttcccaagcctgatcttcaaaaggttggttaatttggcagctgagttcctccccaggcagagaatagaccaattttaggtgtattgggactgagggaggatgtgtaaagattaacatcagtaaagaaccgctgtggagtaattaagaactttgttctttataactggagaatataacctaaccctaacatccctcagcctttactaaagtgtggcgtaaatcacagtagtagcaaagaaagtgactctggatgtgttcctggccagtacctcccttatcatgaatgtagactctctcatcaagatttaggaatataaatcaaatcaaatgtgcccagccaagctatgtagtaagggacttgaacaatattaggcagaacctataaaataaatcagggaattagaaattatttaaagttttcaaattgtaaattgccccggtgtctttcagcctactgccattatttttgctacaatacctacatttcagaggagggcctactgaaaattccatgcaagtggaaaataatcctcaagttattaatgagtttgaaaagcaatgagttcttaagtctttgtgagtagagcaagatcctacaaaattcagaaatagtaaaaatggattcatgctgatttgaagagcatctgtgtgcataatataatgctgcatctcttttaaaagcagtctatttttctttttaaatttgtccccatagatgcttttgaacatgaacatgcttatgttaccttttccgaggttgggaagagccaggagctctcaggcagggccccctccctcagctgggcaggagctgctcaggaggagctagttatagaggaagcttagcgttggcattttcaaaattcaaggtgataacgctttcttcttcctttctgttttagaatagattgctgtctgatttgaaaaagggaaatagatttgatctcaaatgaatctgtgcccagaagccaggctcagggtattcagagatttgtatagtgccctcaaaaaataacaaaattttagctttccttttttcttcttttctccatcaaattcttttttctctagtttacaaatgacatggaaaaggaatttcccctgagttttgtatgcctttttttttttggcttagactatagataggcgtgttgagctcctaagaaaatacaaggaggaactctttgttgtgcagagcactttatgagtagtttgtgtggataatatgtgactgcttccctgacgagcttgtgaggctgtacttatgtctttcctgtaaggcagcttcagtgccttctgtagtgtatataaggaaagattacgccttctgaaaaatctcagagcaaccataagattattttaaaatatgtagtatgactgatggactttttcatcattaaattagtctagcatctaaacttttaccactgaaataatattgaccaaaaagcaatttataaaaggtatttgtgaatagaaaatacaatgtgatcatttgtacttatgtgcaccttaaaagaggaattctgtctagctgtcaaattctggttccttaacatccagtccttgattgtgattgagatctggtaggacgtgctggggcacgctagcagataaaatcccgtatactttaggatagatgttacatttatgtcagtgttggcaaagagcattgtgtagtaataaagaattcaagacttcagcaatgtcaacctgaaactttgtaaatatttcctagattgttatttgatgcagtcacagctctttatcacacaatgttgtctttccctcatcaggcaattttagaactgctgcacacccctcctcagatctcacctgcccctcctgtacattcacctctccagccttgtgcacacctcatttagctttagtttgaaacacattgcagggttcaggtgacctcttcaaaaactacctcctcagaatgaggtaatgaatagttatttattttaaaatatgaaaagtcaggagctctagaatatgaagatgatctaagattttaacttttatgtatacttgttgagcactctccttttgtcctaaagggcattatacatttaagcagtaatactgaaaaatgtagctcagagtaactgaatgttgttgaaagtggtgccagaatctgttttaggggtacgtatcagaatcttaatcttaaatcggttacatgaaattaaatagttaatggtaacacttgactaacagatataattttaattttcggtaggcttttagcaagacagtaagtacatcttcataatgagttagccacagcttcatcacatgcacagattttcctgttgagagactgcccagttaagagggtagaatgatgaaccatttttcaggattctcttctttgtccaaactggcattgtgagtgctagaatatcagcactttcaaactagtgattccaactattaggctattaaaaagcaaaacaaaccaaacaaaccatagccagacatgggaagtttactatgagtataaacagcaaatagcttacaggtcatacattgaaatggtgtaggtaaggcgttagaaaaataccttgacaatttgccaaatgatcttactgtgccttcatgatgcaataaaaaaaaaaaaaatttagcataaatcagtgatttgtgaagagagcagccaccctggtctaactcagctgtgttaatattttttagcgtgcaatttagactgcaaagataaatgcactaaagagtttatagccaaaatcacatttaaaaaatgagagaaaacacaggtaaattttcagtgaacaaaattatttttttaaagtacataatccctagtatagtcagatatatttatcacatagagcaaataggttgaaatcacaattcagtgacatttctagagaaactttttctactcccataggttcttcaaagcatggaacttttatataacagaaatgtgtgacggtcattttaaattgctgtagtttggggctgaagtactgtgtgctgggcagcaatcacatgtattaactagtgagaaaggagaaattaagatataggacagaatttgattttcttgttcccagattactgctgccaacctagacactgagtttccagaggctgaaacgtaaacttgcagctcagcaactgttttgcaaagttagtgggactgtcctgcttatgctgttcaaaaatgctctgagggccaggtggggcctccaggggctcctctctgaggggacatcagactagctaacgacctggcgggcggatgtgaaccggacacactccatggtgtgcttcttgtatcggtccctcgccaccctcaagaaaggcttcagcgggttctctagacgtctccactaaggtgtgttactaacagccatgggttgttgagcacccgaggagtgcaatagcatctctgcatgattgtatattggcccgaagagaatgaagtggccagtgtactcatgttccatgttgctagctctggtaaactgaaaatactggtaagatttttgttttatcagtacactagagagtaagctttgttttgttgtttttagataatgttttcacttccatttggaaagacatttaaattgagtttcagtcctaaattttgccagtcatggtaattagcagtttctatcaggtatttttaaggtagaagaggatagaaacataagttctaaaagcttaaggtaaccgtggtttattttaaaatgtttaggggtggttagtctctacctcaaaaaaagtgagtgaatcttttatttcagcattcacaagttcggctgttgtttttgtaatacattttttttttaaccttttgacccccctttacctaagtgtcaatgtagttttattaattactaagtcagtttcattaaaatgtttatttagcagttttgactaattgcaatgattaatatagccagttgtgcatgaggacacagccagtgagtatatctgggttttttttgtgatgctttttttcttaagacttctgtagatttatgaagtactcattgaaaacaactaaaatacgtttattcgtgttaatatggaaaaaaaaaaa

SEQ ID NO: 87 - protein, 603 aa, Bos taurus
MMRGLIPECCAVYRIQDGEKKPIGWDTDISWLTGEELHVEVLENVPLTTHNFVRKTFFTLAFCDFCRKLLFQGFRCQTCGYKFHQRCSTEVPLMCVNYDQLDLLFVSKFFEHHPIPQEEASLAETTLPCGSSPSAPPSDSIGPPILTSPSPSKSIPIPQPFRPADEDHRNQFGQRDRSSSAPNVHINTIEPVNIDDLIRDQGFRSDGGSTTGLSATPPASLPGSLSNVKALQKSPGPQRERKSSSSSEDRNRMKTLGRRDSSDDWEIPDGQITVGQRIGSGSFGTVYKGKWHGDVAVKMLNVTAPTPQQLQAFKNEVGVLRKTRHVNILLFMGYSTKPQLAIVTQWCEGSSLYHHLHIIETKFEMIKLIDIARQTAQGMDYLHAKSIIHRDLKSNNIFLHEDLTVKIGDFGLATVKSRWSGSHQFEQLSGSILWMAPEVIRMQDKNPYSFQSDVYAFGIVLYELMTGQLPYSNINNRDQIIFMVGRGYLSPDLSKVRSNCPKAMKRLMAECLKKKRDERPLFPQVGKTLLSKRQNSEVIREKDKQILASIELLARSLPKIHRSASEPSLNRAGFQTEDFSLYACASPKTPIQAGGYGEFAAFK

SEQ ID NO: 88 - DNA, 2295 bp, Equus caballus
  misc_feature (79)..(79): n is a, c, g, or t
atgaagacgctgagcggcggcggcggcggcgcggagcagggccaggctctgttcaacggggacatggaacccggaggcnccgcgccggcgcccgcggcctcgtcggccgcggaccctgccattcccgaggaggtatggaatatcaaacaaatgattaaattgacacaggaacatatagaggccctattggacaaatttggtggggagcataatccaccatcaatatatctggaggcctatgaagaatacaccagcaagctagatgccctccaacaaagagaacaacagttattggaatccctggggaatggaactgatttttctgtttctagttctgcatcaacggacaccgttacatcttcttcctcttctagcctttcagtgctaccttcatctctttcagtttttcaaaatcccacagatgtgtcacggagcaaccctaagtcaccacaaaaacctatcgttagagtcttcctgcccaacaaacagaggacagtggtacctgcaaggtgtggcgttacagtccgggacagtctaaagaaagcactgatgatgagaggtctaatcccagagtgctgtgctgtttacagaattcaggatggagagaagaaaccaattggctgggacactgatatttcctggctcactggagaggaattgcatgtagaagtgttggagaatgttccacttacaacacacaactttgtacggaaaacttttttcaccttagcattttgtgacttttgtcgaaagctgcttttccagggtttccgctgtcaaacatgtggttataaatttcaccagcgttgtagtacagaggttccactgatgtgtgttaattatgaccaacttgatttgctgtttgtctccaagttctttgaacaccacccagtatcacaggaggaggcctccttagcagagactgcccttacatctggatcatccccttctgcacccccctccgattccattgggccccaaattctcaccagtccatctccttcaaaatccattccaattccacagcctttccgaccagcagatgaagatcatcgaaatcagtttggacaacgagaccggtcctcatcagctccaaatgtacatataaacacaatagaacctgtcaatattgatgacttgattagagaccaagggtttcgtagtgatggaggatcaaccacaggtttatctgccaccccccctgcctcattacctggctcactcactaatgtgaaggcattacagaaatctccaggacctcaacgggaaaggaaatcatcttcatcctcagaagacaggaatcgaatgaaaactcttggtagacgggattcaagtgacgattgggagattcctgatgggcagatcacagtgggacaaagaattggatctgggtcatttgggacagtctacaagggaaagtggcatggtgatgtggcagtgaaaatgttgaatgtgacagcacccacacctcagcagttacaggccttcaaaaatgaagtaggagtactcaggaaaactcgacatgtgaatatcctactcttcatgggctattcaacaaagccacaactggctattgttacccagtggtgtgagggctccagcttatatcaccatctccacatcattgagaccaaatttgagatgatcaaacttatagatattgctcggcaaactgcacagggcatggattacttacacgccaagtcaatcatccacagagacctcaagagtaataatatttttcttcatgaagacctcacagtaaaaataggtgattttggtctagccacagtgaaatctcgatggagtgggtcccatcagtttgaacagttgtctggatccattttgtggatggcaccagaagtaatcagaatgcaagataaaaacccgtatagctttcaatcagatgtatatgcctttgggattgttctgtatgaattgatgactggacagttaccttattcaaacatcaacaacagggaccagataatttttatggtgggaagaggatatctatctccagatctcagtaaggtacggagtaactgtccaaaagccatgaagagattaatggcagagtgcctaaaaaagaaaagagacgagagaccactcttcccccaaattctcgcctctattgagctgctggcccgctcattgccaaaaattcaccgcagtgcatcagagccctccttgaatcgggctggcttccagacagaggattttagtctatatgcttgtgcttctccgaaaacacccatccaggcagggggatatggtgcgtttcctgtccactga

SEQ ID NO: 89 - protein, 764 aa, Equus caballus
  misc_feature (27)..(27): Xaa can be any naturally occurring amino acid
MKTLSGGGGGAEQGQALFNGDMEPGGXAPAPAASSAADPAIPEEVWNIKQMIKLTQEHIEALLDKFGGEHNPPSIYLEAYEEYTSKLDALQQREQQLLESLGNGTDFSVSSSASTDTVTSSSSSSLSVLPSSLSVFQNPTDVSRSNPKSPQKPIVRVFLPNKQRTVVPARCGVTVRDSLKKALMMRGLIPECCAVYRIQDGEKKPIGWDTDISWLTGEELHVEVLENVPLTTHNFVRKTFFTLAFCDFCRKLLFQGFRCQTCGYKFHQRCSTEVPLMCVNYDQLDLLFVSKFFEHHPVSQEEASLAETALTSGSSPSAPPSDSIGPQILTSPSPSKSIPIPQPFRPADEDHRNQFGQRDRSSSAPNVHINTIEPVNIDDLIRDQGFRSDGGSTTGLSATPPASLPGSLTNVKALQKSPGPQRERKSSSSSEDRNRMKTLGRRDSSDDWEIPDGQITVGQRIGSGSFGTVYKGKWHGDVAVKMLNVTAPTPQQLQAFKNEVGVLRKTRHVNILLFMGYSTKPQLAIVTQWCEGSSLYHHLHIIETKFEMIKLIDIARQTAQGMDYLHAKSIIHRDLKSNNIFLHEDLTVKIGDFGLATVKSRWSGSHQFEQLSGSILWMAPEVIRMQDKNPYSFQSDVYAFGIVLYELMTGQLPYSNINNRDQIIFMVGRGYLSPDLSKVRSNCPKAMKRLMAECLKKKRDERPLFPQILASIELLARSLPKIHRSASEPSLNRAGFQTEDFSLYACASPKTPIQAGGYGAFPVH

SEQ ID NO: 90 - DNA, 2678 bp, Gallus gallus
tccccctccctcgccccagcgcttcgatccaagatggcggcgctgagcagcggcagcagcgccgagggggcctcgctcttcaacggggacatggagcccgagccgccgccgcccgtgctgggcgcctgctacgccgggagcggcggcggcgacccggccatcccggaggaggtgtggaatatcaaacagatgattaaattaacacaagaacatatagaagcgctgttagacaagtttggaggagagcataacccaccatcaatatatttagaggcctatgaggagtacaccagcaaactagatgctctacagcagagagaacagcagttattggaatccatgggaaatggaactgatttctctgtttccagttcagcttcaacggacacagttgcatcatcttcctcctctagcctctctgtagcaccttcatccctttcagtttatcaaaatcctactgatatgtcgcggaataaccctaagtctccacagaagcctattgttagagtcttcctgcccaacaagcaaaggactgtggttccggcaagatgtggggtgacagtccgagacagcctgaagaaagctctgatgatgagaggtcttattccagaatgctgtgctgtttacagaatacaggatggagagaagaagccaattggctgggacactgacatttcctggctaaccggagaggagttacacgtggaggtcttggagaatgtgccactcacaacacacaattttgtacgaaaaacattcttcacgttagcgttctgcgacttctgtcgaaagctgcttttccagggattccgatgccagacatgtggctacaaatttcaccagcgctgtagcacagaagtgccactgatgtgtgttaactacgaccaactcgatttgctgtttgtctccaagttctttgaacatcaccccatatcgcaggaggagaccaccttaggagagaccaccccggcatcgggatcgtacccctcagtgcccccatcagattctgttggaccaccaattctccctagtccttctccttcaaaatccattccaatcccacagcccttccgaccagcagatgaagaccatcggaatcagtttgggcaacgcgaccgatcctcttcagctcccaatgttcacatcaatacaattgagccagtcaatattgatgacttgattagagaccagggtgtacgaggagagggagcccctttgaaccagctgatgcgctgtcttcggaaataccaatcccggactcccagtcccctccttcattctgtccccagtgaaatagtgtttgattttgagcctggcccagtgttcagaggttcaactgcaggtttgtctgcaacacctcctgcatctttgcctgggtcacttaccaatgtgaaagcattacagaaatcaccaggcccccaacgggaaaggaaatcatcctcatcctcagaagacagaaataggatgaaaacccttggtcgacgagattcaagtgatgattgggaaataccagatgggcagatcacagttggacaaaggataggatctggatcatttggaacagtctacaaaggaaagtggcatggtgacgtggcagtgaaaatgttgaatgttacagcacccacacctcaacagttacaggctttcaaaaatgaagtaggagtgctcaggaaaacacggcatgtgaatatcctactttttatgggttattcaacaaaacctcagttggctattgttacacagtggtgtgaggggtccagcttatatcaccatctgcacataattgagaccaagtttgaaatgatcaaactaattgatattgcacgacagactgcacaaggcatggattatttgcatgccaagtcaatcatccacagagacctcaagagtaataatatttttcttcatgaagacctcacagtaaaaataggtgacttcggtctggctacagtgaaatcacgatggagtggatctcatcaatttgaacagttatctggatcaattctatggatggcaccggaagtgatcaggatgcaagacaaaaacccatatagctttcagtcagatgtgtatgcattcgggattgtgctttatgaactgatgactggacagttaccatactcaaacatcaacaacagggaccagataatttttatggtgggacgaggatatctatctccagacctcagtaaagtaagaagtaactgtccaaaagctatgaagagactaatggcagaatgcttgaaaaagaaaagagatgagagacctctttttccacagattcttgcctccattgagcttctggcccggtcgttgccaaaaattcaccgcagtgcatctgagccgtcactaaaccgggctggcttccagaccgaggatttcagtctgtatgcttgtgcttctccaaaaacgcccatccaagcagggggatacggtgggtttccagtacactgaaaagaaatgtgaaagcgtgtgcctgtttgctcatgtgctggtgtgttcctgtgtgtgcaacgcatacgtacgttctcagttcctaccagcgactttttaaggtttactgagggaatgaagactcatttcctaacatggggcattgaacgtcctgagcacaagtcagtgctggtaaggaatgtcttgggaacagctggcaagaagaattagaaggtacttaaagg

SEQ ID NO: 91 - protein, 806 aa, Gallus gallus
MAALSSGSSAEGASLFNGDMEPEPPPPVLGACYAGSGGGDPAIPEEVWNIKQMIKLTQEHIEALLDKFGGEHNPPSIYLEAYEEYTSKLDALQQREQQLLESMGNGTDFSVSSSASTDTVASSSSSSLSVAPSSLSVYQNPTDMSRNNPKSPQKPIVRVFLPNKQRTVVPARCGVTVRDSLKKALMMRGLIPECCAVYRIQDGEKKPIGWDTDISWLTGEELHVEVLENVPLTTHNFVRKTFFTLAFCDFCRKLLFQGFRCQTCGYKFHQRCSTEVPLMCVNYDQLDLLFVSKFFEHHPISQEETTLGETTPASGSYPSVPPSDSVGPPILPSPSPSKSIPIPQPFRPADEDHRNQFGQRDRSSSAPNVHINTIEPVNIDDLIRDQGVRGEGAPLNQLMRCLRKYQSRTPSPLLHSVPSEIVFDFEPGPVFRGSTAGLSATPPASLPGSLTNVKALQKSPGPQRERKSSSSSEDRNRMKTLGRRDSSDDWEIPDGQITVGQRIGSGSFGTVYKGKWHGDVAVKMLNVTAPTPQQLQAFKNEVGVLRKTRHVNILLFMGYSTKPQLAIVTQWCEGSSLYHHLHIIETKFEMIKLIDIARQTAQGMDYLHAKSIIHRDLKSNNIFLHEDLTVKIGDFGLATVKSRWSGSHQFEQLSGSILWMAPEVIRMQDKNPYSFQSDVYAFGIVLYELMTGQLPYSNINNRDQIIFMVGRGYLSPDLSKVRSNCPKAMKRLMAECLKKKRDERPLFPQILASIELLARSLPKIHRSASEPSLNRAGFQTEDFSLYACASPKTPIQAGGYGGFPVH

SEQ ID NO: 92 - DNA, 21 bp, Artificial Sequence
  BRAF siRNA 313
tacaccagcaagctagatgca

SEQ ID NO: 93 - DNA, 21 bp, Artificial Sequence
  BRAF siRNA 523
cctatcgttagagtcttcctg